European Patent Application EP 4 810 604 A2, published September 23, 2026. Title: METHODS, MODELS, SYSTEMS, AND APPARATUS FOR IDENTIFYING TARGET SEQUENCES FOR CAS ENZYMES OR CRISPR-CAS SYSTEMS FOR TARGET SEQUENCES AND CONVEYING RESULTS THEREOF. Applicant: THE BROAD INSTITUTE, INC. Application US PCT/US2013/074812, filed December 12, 2013. The sequence listing filed with the application follows.

SEQUENCE LISTING (1076 sequences)

SEQ ID NO: 1 - RNA, 12 nt, synthetic construct
  misc_feature 1..12: note = source = /note="Description of Artificial Sequence: Synthetic oligonucleotide"
  source 1..12: mol_type = other RNA
gttttagagcta

SEQ ID NO: 2 - protein, 7 aa, Simian virus 40
PKKKRKV

SEQ ID NO: 3 - protein, 16 aa, unidentified
  REGION 1..16: note = source = /note="Description of Unknown: Nucleoplasmin bipartite NLS sequence"
KRPAATKKAGQAKKKK

SEQ ID NO: 4 - protein, 9 aa, unidentified
  REGION 1..9: note = source = /note="Description of Unknown: C-myc NLS sequence"
PAAKRVKLD

SEQ ID NO: 5 - protein, 11 aa, unidentified
  REGION 1..11: note = source = /note="Description of Unknown: C-myc NLS sequence"
RQRRNELKRSP

SEQ ID NO: 6 - protein, 38 aa, Homo sapiens
NQSSNFGPMKGGNFGGRSSGPYGGGGQYFAKPRNQGGY

SEQ ID NO: 7 - protein, 42 aa, unidentified
  REGION 1..42: note = source = /note="Description of Unknown: IBB domain from importin-alpha sequence"
RMRIZFKNKGKDTAELRRRRVEVSVELRKAKKDEQILKRRNV

SEQ ID NO: 8 - protein, 8 aa, unidentified
  REGION 1..8: note = source = /note="Description of Unknown: Myoma T protein sequence"
VSRKRPRP

SEQ ID NO: 9 - protein, 8 aa, unidentified
  REGION 1..8: note = source = /note="Description of Unknown: Myoma T protein sequence"
PPKKARED

SEQ ID NO: 10 - protein, 8 aa, Homo sapiens
PQPKKKPL

SEQ ID NO: 11 - protein, 12 aa, Mus musculus
SALIKKKKKMAP

SEQ ID NO: 12 - protein, 5 aa, Influenza virus
DRLRR

SEQ ID NO: 13 - protein, 7 aa, Influenza virus
PKQKKRK

SEQ ID NO: 14 - protein, 10 aa, Hepatitus delta virus
RKLKKKIKKL

SEQ ID NO: 15 - protein, 10 aa, Mus musculus
REKKKFLKRR

SEQ ID NO: 16 - protein, 20 aa, Homo sapiens
KRKGDEVDGVDEVAKKKSKK

SEQ ID NO: 17 - protein, 17 aa, Homo sapiens
RKCLQAGMNLEARKTKK

SEQ ID NO: 18-21 - skipped (4 entries)

SEQ ID NO: 22 - DNA, 137 bp, synthetic construct
  modified_base 1..20: mod_base = OTHER; note = a, c, t, g, unknown or other
  misc_feature 1..137: note = source = /note="Description of Artificial Sequence: Synthetic polynucleotide"
  source 1..137: mol_type = other DNA
nnnnnnnnnnnnnnnnnnnngtttttgtactctcaagatttagaaataaatcttgcagaagctacaaagataaggcttcatgccgaaatcaacaccctgtcattttatggcagggtgttttcgttatttaatttttt

SEQ ID NO: 23 - DNA, 123 bp, synthetic construct
  modified_base 1..20: mod_base = OTHER; note = a, c, t, g, unknown or other
  misc_feature 1..123: note = source = /note="Description of Artificial Sequence: Synthetic polynucleotide"
  source 1..123: mol_type = other DNA
nnnnnnnnnnnnnnnnnnnngtttttgtactctcagaaatgcagaagctacaaagataaggcttcatgccgaaatcaacaccctgtcattttatggcagggtgttttcgttatttaatttttt

SEQ ID NO: 24 - DNA, 110 bp, synthetic construct
  modified_base 1..20: mod_base = OTHER; note = a, c, t, g, unknown or other
  misc_feature 1..110: note = source = /note="Description of Artificial Sequence: Synthetic polynucleotide"
  source 1..110: mol_type = other DNA
nnnnnnnnnnnnnnnnnnnngtttttgtactctcagaaatgcagaagctacaaagataaggcttcatgccgaaatcaacaccctgtcattttatggcagggtgttttttt

SEQ ID NO: 25 - DNA, 102 bp, synthetic construct
  modified_base 1..20: mod_base = OTHER; note = a, c, t, g, unknown or other
  misc_feature 1..102: note = source = /note="Description of Artificial Sequence: Synthetic polynucleotide"
  source 1..102: mol_type = other DNA
nnnnnnnnnnnnnnnnnnnngttttagagctagaaatagcaagttaaaataaggctagtccgttatcaacttgaaaaagtggcaccgagtcggtgctttttt

SEQ ID NO: 26 - DNA, 88 bp, synthetic construct
  modified_base 1..20: mod_base = OTHER; note = a, c, t, g, unknown or other
  misc_feature 1..88: note = source = /note="Description of Artificial Sequence: Synthetic oligonucleotide"
  source 1..88: mol_type = other DNA
nnnnnnnnnnnnnnnnnnnngttttagagctagaaatagcaagttaaaataaggctagtccgttatcaacttgaaaaagtgttttttt

SEQ ID NO: 27 - DNA, 76 bp, synthetic construct
  modified_base 1..20: mod_base = OTHER; note = a, c, t, g, unknown or other
  misc_feature 1..76: note = source = /note="Description of Artificial Sequence: Synthetic oligonucleotide"
  source 1..76: mol_type = other DNA
nnnnnnnnnnnnnnnnnnnngttttagagctagaaatagcaagttaaaataaggctagtccgttatcatttttttt

SEQ ID NO: 28 - DNA, 22 bp, Homo sapiens
  modified_base 20: mod_base = OTHER; note = a, c, t, g, unknown or other
  source 1..22: mol_type = unassigned DNA
aggccccagtggctgctctnaa

SEQ ID NO: 29 - DNA, 22 bp, Homo sapiens
  modified_base 20: mod_base = OTHER; note = a, c, t, g, unknown or other
  source 1..22: mol_type = unassigned DNA
acatcaaccggtggcgcatnat

SEQ ID NO: 30 - DNA, 22 bp, Homo sapiens
  modified_base 20: mod_base = OTHER; note = a, c, t, g, unknown or other
  source 1..22: mol_type = unassigned DNA
aaggtgtggttccagaaccnac

SEQ ID NO: 31 - DNA, 22 bp, Homo sapiens
  modified_base 20: mod_base = OTHER; note = a, c, t, g, unknown or other
  source 1..22: mol_type = unassigned DNA
ccatcacatcaaccggtggnag

SEQ ID NO: 32 - DNA, 22 bp, Homo sapiens
  modified_base 20: mod_base = OTHER; note = a, c, t, g, unknown or other
  source 1..22: mol_type = unassigned DNA
aaacggcagaagctggaggnta

SEQ ID NO: 33 - DNA, 22 bp, Homo sapiens
  modified_base 20: mod_base = OTHER; note = a, c, t, g, unknown or other
  source 1..22: mol_type = unassigned DNA
ggcagaagctggaggaggantt

SEQ ID NO: 34 - DNA, 22 bp, Homo sapiens
  modified_base 20: mod_base = OTHER; note = a, c, t, g, unknown or other
  source 1..22: mol_type = unassigned DNA
ggtgtggttccagaaccggntc

SEQ ID NO: 35 - DNA, 22 bp, Homo sapiens
  modified_base 20: mod_base = OTHER; note = a, c, t, g, unknown or other
  source 1..22: mol_type = unassigned DNA
aaccggaggacaaagtacantg

SEQ ID NO: 36 - DNA, 22 bp, Homo sapiens
  modified_base 20: mod_base = OTHER; note = a, c, t, g, unknown or other
  source 1..22: mol_type = unassigned DNA
ttccagaaccggaggacaanca

SEQ ID NO: 37 - DNA, 22 bp, Homo sapiens
  modified_base 20: mod_base = OTHER; note = a, c, t, g, unknown or other
  source 1..22: mol_type = unassigned DNA
gtgtggttccagaaccgganct

SEQ ID NO: 38 - DNA, 22 bp, Homo sapiens
  modified_base 20: mod_base = OTHER; note = a, c, t, g, unknown or other
  source 1..22: mol_type = unassigned DNA
tccagaaccggaggacaaancc

SEQ ID NO: 39 - DNA, 22 bp, Homo sapiens
  modified_base 20: mod_base = OTHER; note = a, c, t, g, unknown or other
  source 1..22: mol_type = unassigned DNA
cagaagctggaggaggaagncg

SEQ ID NO: 40 - DNA, 22 bp, Homo sapiens
  modified_base 20: mod_base = OTHER; note = a, c, t, g, unknown or other
  source 1..22: mol_type = unassigned DNA
catcaaccggtggcgcattnga

SEQ ID NO: 41 - DNA, 22 bp, Homo sapiens
  modified_base 20: mod_base = OTHER; note = a, c, t, g, unknown or other
  source 1..22: mol_type = unassigned DNA
gcagaagctggaggaggaangt

SEQ ID NO: 42 - DNA, 22 bp, Homo sapiens
  modified_base 20: mod_base = OTHER; note = a, c, t, g, unknown or other
  source 1..22: mol_type = unassigned DNA
cctccctccctggcccaggngc

SEQ ID NO: 43 - DNA, 22 bp, Homo sapiens
  modified_base 20: mod_base = OTHER; note = a, c, t, g, unknown or other
  source 1..22: mol_type = unassigned DNA
tcatctgtgcccctccctcnaa

SEQ ID NO: 44 - DNA, 22 bp, Homo sapiens
  modified_base 20: mod_base = OTHER; note = a, c, t, g, unknown or other
  source 1..22: mol_type = unassigned DNA
gggaggacatcgatgtcacnat

SEQ ID NO: 45 - DNA, 22 bp, Homo sapiens
  modified_base 20: mod_base = OTHER; note = a, c, t, g, unknown or other
  source 1..22: mol_type = unassigned DNA
caaacggcagaagctggagnac

SEQ ID NO: 46 - DNA, 22 bp, Homo sapiens
  modified_base 20: mod_base = OTHER; note = a, c, t, g, unknown or other
  source 1..22: mol_type = unassigned DNA
gggtgggcaaccacaaaccnag

SEQ ID NO: 47 - DNA, 22 bp, Homo sapiens
  modified_base 20: mod_base = OTHER; note = a, c, t, g, unknown or other
  source 1..22: mol_type = unassigned DNA
ggtgggcaaccacaaacccnta

SEQ ID NO: 48 - DNA, 22 bp, Homo sapiens
  modified_base 20: mod_base = OTHER; note = a, c, t, g, unknown or other
  source 1..22: mol_type = unassigned DNA
ggctcccatcacatcaaccntt

SEQ ID NO: 49 - DNA, 22 bp, Homo sapiens
  modified_base 20: mod_base = OTHER; note = a, c, t, g, unknown or other
  source 1..22: mol_type = unassigned DNA
gaagggcctgagtccgagcntc

SEQ ID NO: 50 - DNA, 22 bp, Homo sapiens
  modified_base 20: mod_base = OTHER; note = a, c, t, g, unknown or other
  source 1..22: mol_type = unassigned DNA
caaccggtggcgcattgccntg

SEQ ID NO: 51 - DNA, 22 bp, Homo sapiens
  modified_base 20: mod_base = OTHER; note = a, c, t, g, unknown or other
  source 1..22: mol_type = unassigned DNA
aggaggaagggcctgagtcnca

SEQ ID NO: 52 - DNA, 22 bp, Homo sapiens
  modified_base 20: mod_base = OTHER; note = a, c, t, g, unknown or other
  source 1..22: mol_type = unassigned DNA
agctggaggaggaagggccnct

SEQ ID NO: 53 - DNA, 22 bp, Homo sapiens
  modified_base 20: mod_base = OTHER; note = a, c, t, g, unknown or other
  source 1..22: mol_type = unassigned DNA
gcattgccacgaagcaggcncc

SEQ ID NO: 54 - DNA, 22 bp, Homo sapiens
  modified_base 20: mod_base = OTHER; note = a, c, t, g, unknown or other
  source 1..22: mol_type = unassigned DNA
attgccacgaagcaggccancg

SEQ ID NO: 55 - DNA, 22 bp, Homo sapiens
  modified_base 20: mod_base = OTHER; note = a, c, t, g, unknown or other
  source 1..22: mol_type = unassigned DNA
agaaccggaggacaaagtanga

SEQ ID NO: 56 - DNA, 22 bp, Homo sapiens
  modified_base 20: mod_base = OTHER; note = a, c, t, g, unknown or other
  source 1..22: mol_type = unassigned DNA
tcaaccggtggcgcattgcngt

SEQ ID NO: 57 - DNA, 22 bp, Homo sapiens
  modified_base 20: mod_base = OTHER; note = a, c, t, g, unknown or other
  source 1..22: mol_type = unassigned DNA
gaagctggaggaggaagggngc

SEQ ID NO: 58 - DNA, 23 bp, synthetic construct
  misc_feature 1..23: note = source = /note="Description of Artificial Sequence: Synthetic oligonucleotide"
  source 1..23: mol_type = other DNA
gccaaattggacgaccctcgcgg

SEQ ID NO: 59 - DNA, 23 bp, synthetic construct
  misc_feature 1..23: note = source = /note="Description of Artificial Sequence: Synthetic oligonucleotide"
  source 1..23: mol_type = other DNA
cgaggagacccccgtttcggtgg

SEQ ID NO: 60 - DNA, 23 bp, synthetic construct
  misc_feature 1..23: note = source = /note="Description of Artificial Sequence: Synthetic oligonucleotide"
  source 1..23: mol_type = other DNA
cccgccgccgccgtggctcgagg

SEQ ID NO: 61 - DNA, 23 bp, synthetic construct
  misc_feature 1..23: note = source = /note="Description of Artificial Sequence: Synthetic oligonucleotide"
  source 1..23: mol_type = other DNA
tgagctctacgagatccacaagg

SEQ ID NO: 62 - DNA, 23 bp, synthetic construct
  misc_feature 1..23: note = source = /note="Description of Artificial Sequence: Synthetic oligonucleotide"
  source 1..23: mol_type = other DNA
ctcaaaattcataccggttgtgg

SEQ ID NO: 63 - DNA, 23 bp, synthetic construct
  misc_feature 1..23: note = source = /note="Description of Artificial Sequence: Synthetic oligonucleotide"
  source 1..23: mol_type = other DNA
cgttaaacaacaaccggacttgg

SEQ ID NO: 64 - DNA, 23 bp, synthetic construct
  misc_feature 1..23: note = source = /note="Description of Artificial Sequence: Synthetic oligonucleotide"
  source 1..23: mol_type = other DNA
ttcaccccgcggcgctgaatggg

SEQ ID NO: 65 - DNA, 23 bp, synthetic construct
  misc_feature 1..23: note = source = /note="Description of Artificial Sequence: Synthetic oligonucleotide"
  source 1..23: mol_type = other DNA
accactaccagtccgtccacagg

SEQ ID NO: 66 - DNA, 23 bp, synthetic construct
  misc_feature 1..23: note = source = /note="Description of Artificial Sequence: Synthetic oligonucleotide"
  source 1..23: mol_type = other DNA
cactgcttaagcctcgctcgagg

SEQ ID NO: 67 - DNA, 23 bp, synthetic construct
  misc_feature 1..23: note = source = /note="Description of Artificial Sequence: Synthetic oligonucleotide"
  source 1..23: mol_type = other DNA
tcaccagcaatattcgctcgagg

SEQ ID NO: 68 - DNA, 23 bp, synthetic construct
  misc_feature 1..23: note = source = /note="Description of Artificial Sequence: Synthetic oligonucleotide"
  source 1..23: mol_type = other DNA
caccagcaatattccgctcgagg

SEQ ID NO: 69 - DNA, 23 bp, synthetic construct
  misc_feature 1..23: note = source = /note="Description of Artificial Sequence: Synthetic oligonucleotide"
  source 1..23: mol_type = other DNA
tagcaacagacatacgctcgagg

SEQ ID NO: 70 - DNA, 23 bp, synthetic construct
  misc_feature 1..23: note = source = /note="Description of Artificial Sequence: Synthetic oligonucleotide"
  source 1..23: mol_type = other DNA
gggcagtagtaatacgctcgagg

SEQ ID NO: 71 - DNA, 23 bp, synthetic construct
  misc_feature 1..23: note = source = /note="Description of Artificial Sequence: Synthetic oligonucleotide"
  source 1..23: mol_type = other DNA
ccaattcccatacattattgtac

SEQ ID NO: 72 - DNA, 33 bp, Homo sapiens
  source 1..33: mol_type = unassigned DNA
ggacatcgatgtcacctccaatgactagggtgg

SEQ ID NO: 73 - DNA, 33 bp, Homo sapiens
  source 1..33: mol_type = unassigned DNA
cattggaggtgacatcgatgtcctccccattgg

SEQ ID NO: 74 - DNA, 33 bp, Homo sapiens
  source 1..33: mol_type = unassigned DNA
ggaagggcctgagtccgagcagaagaagaaggg

SEQ ID NO: 75 - DNA, 33 bp, Homo sapiens
  source 1..33: mol_type = unassigned DNA
ggtggcgagaggggccgagattgggtgttcagg

SEQ ID NO: 76 - DNA, 33 bp, Homo sapiens
  source 1..33: mol_type = unassigned DNA
atgcaggagggtggcgagaggggccgagattgg

SEQ ID NO: 77 - DNA, 23 bp, Homo sapiens
  source 1..23: mol_type = unassigned DNA
gtcacctccaatgactagggtgg

SEQ ID NO: 78 - DNA, 23 bp, Homo sapiens
  source 1..23: mol_type = unassigned DNA
gacatcgatgtcctccccattgg

SEQ ID NO: 79 - DNA, 23 bp, Homo sapiens
  source 1..23: mol_type = unassigned DNA
gagtccgagcagaagaagaaggg

SEQ ID NO: 80 - DNA, 23 bp, Homo sapiens
  source 1..23: mol_type = unassigned DNA
gcgccaccggttgatgtgatggg

SEQ ID NO: 81 - DNA, 23 bp, Homo sapiens
  source 1..23: mol_type = unassigned DNA
ggggcacagatgagaaactcagg

SEQ ID NO: 82 - DNA, 23 bp, Homo sapiens
  source 1..23: mol_type = unassigned DNA
gtacaaacggcagaagctggagg

SEQ ID NO: 83 - DNA, 23 bp, Homo sapiens
  source 1..23: mol_type = unassigned DNA
ggcagaagctggaggaggaaggg

SEQ ID NO: 84 - DNA, 23 bp, Homo sapiens
  source 1..23: mol_type = unassigned DNA
ggagcccttcttcttctgctcgg

SEQ ID NO: 85 - DNA, 23 bp, Homo sapiens
  source 1..23: mol_type = unassigned DNA
gggcaaccacaaacccacgaggg

SEQ ID NO: 86 - DNA, 23 bp, Homo sapiens
  source 1..23: mol_type = unassigned DNA
gctcccatcacatcaaccggtgg

SEQ ID NO: 87 - DNA, 23 bp, Homo sapiens
  source 1..23: mol_type = unassigned DNA
gtggcgcattgccacgaagcagg

SEQ ID NO: 88 - DNA, 23 bp, Homo sapiens
  source 1..23: mol_type = unassigned DNA
ggcagagtgctgcttgctgctgg

SEQ ID NO: 89 - DNA, 23 bp, Homo sapiens
  source 1..23: mol_type = unassigned DNA
gcccctgcgtgggcccaagctgg

SEQ ID NO: 90 - DNA, 23 bp, Homo sapiens
  source 1..23: mol_type = unassigned DNA
gagtggccagagtccagcttggg

SEQ ID NO: 91 - DNA, 23 bp, Homo sapiens
  source 1..23: mol_type = unassigned DNA
ggcctccccaaagcctggccagg

SEQ ID NO: 92 - DNA, 23 bp, Homo sapiens
  source 1..23: mol_type = unassigned DNA
ggggccgagattgggtgttcagg

SEQ ID NO: 93 - DNA, 23 bp, Homo sapiens
  source 1..23: mol_type = unassigned DNA
gtggcgagaggggccgagattgg

SEQ ID NO: 94 - DNA, 23 bp, Homo sapiens
  source 1..23: mol_type = unassigned DNA
gagtgccgccgaggcggggcggg

SEQ ID NO: 95 - DNA, 23 bp, Homo sapiens
  source 1..23: mol_type = unassigned DNA
ggagtgccgccgaggcggggcgg

SEQ ID NO: 96 - DNA, 23 bp, Homo sapiens
  source 1..23: mol_type = unassigned DNA
ggagaggagtgccgccgaggcgg

SEQ ID NO: 97 - DNA, 21 bp, synthetic construct
  misc_feature 1..21: note = source = /note="Description of Artificial Sequence: Synthetic primer"
  source 1..21: mol_type = other DNA
aaaaccacccttctctctggc

SEQ ID NO: 98 - DNA, 21 bp, synthetic construct
  misc_feature 1..21: note = source = /note="Description of Artificial Sequence: Synthetic primer"
  source 1..21: mol_type = other DNA
ggagattggagacacggagag

SEQ ID NO: 99 - DNA, 20 bp, synthetic construct
  misc_feature 1..20: note = source = /note="Description of Artificial Sequence: Synthetic primer"
  source 1..20: mol_type = other DNA
ccatccccttctgtgaatgt

SEQ ID NO: 100 - DNA, 20 bp, synthetic construct
  misc_feature 1..20: note = source = /note="Description of Artificial Sequence: Synthetic primer"
  source 1..20: mol_type = other DNA
ggagattggagacacggaga

SEQ ID NO: 101 - DNA, 20 bp, synthetic construct
  misc_feature 1..20: note = source = /note="Description of Artificial Sequence: Synthetic primer"
  source 1..20: mol_type = other DNA
ctggaaagccaatgcctgac

SEQ ID NO: 102 - DNA, 20 bp, synthetic construct
  misc_feature 1..20: note = source = /note="Description of Artificial Sequence: Synthetic primer"
  source 1..20: mol_type = other DNA
ggcagcaaactccttgtcct

SEQ ID NO: 103 - DNA, 20 bp, synthetic construct
  misc_feature 1..20: note = source = /note="Description of Artificial Sequence: Synthetic primer"
  source 1..20: mol_type = other DNA
aagcaccgactcggtgccac

SEQ ID NO: 104 - DNA, 20 bp, synthetic construct
  misc_feature 1..20: note = source = /note="Description of Artificial Sequence: Synthetic primer"
  source 1..20: mol_type = other DNA
tcacctccaatgactagggg

SEQ ID NO: 105 - DNA, 22 bp, synthetic construct
  misc_feature 1..22: note = source = /note="Description of Artificial Sequence: Synthetic primer"
  source 1..22: mol_type = other DNA
caagttgataacggactagcct

SEQ ID NO: 106 - DNA, 23 bp, synthetic construct
  misc_feature 1..23: note = source = /note="Description of Artificial Sequence: Synthetic primer"
  source 1..23: mol_type = other DNA
agtccgagcagaagaagaagttt

SEQ ID NO: 107 - DNA, 25 bp, synthetic construct
  misc_feature 1..25: note = source = /note="Description of Artificial Sequence: Synthetic primer"
  source 1..25: mol_type = other DNA
tttcaagttgataacggactagcct

SEQ ID NO: 108 - DNA, 20 bp, synthetic construct
  misc_feature 1..20: note = source = /note="Description of Artificial Sequence: Synthetic primer"
  source 1..20: mol_type = other DNA
aaacagcagattcgcctgga

SEQ ID NO: 109 - DNA, 20 bp, synthetic construct
  misc_feature 1..20: note = source = /note="Description of Artificial Sequence: Synthetic primer"
  source 1..20: mol_type = other DNA
tcatccgctcgatgaagctc

SEQ ID NO: 110 - DNA, 20 bp, synthetic construct
  misc_feature 1..20: note = source = /note="Description of Artificial Sequence: Synthetic primer"
  source 1..20: mol_type = other DNA
tccaaaatcaagtggggcga

SEQ ID NO: 111 - DNA, 20 bp, synthetic construct
  misc_feature 1..20: note = source = /note="Description of Artificial Sequence: Synthetic primer"
  source 1..20: mol_type = other DNA
tgatgacccttttggctccc

SEQ ID NO: 112 - DNA, 45 bp, synthetic construct
  misc_feature 1..45: note = source = /note="Description of Artificial Sequence: Synthetic primer"
  source 1..45: mol_type = other DNA
gaggaattctttttttgttygaatatgttggaggttttttggaag

SEQ ID NO: 113 - DNA, 42 bp, synthetic construct
  misc_feature 1..42: note = source = /note="Description of Artificial Sequence: Synthetic primer"
  source 1..42: mol_type = other DNA
gagaagcttaaataaaaaacracaatactcaacccaacaacc

SEQ ID NO: 114 - DNA, 17 bp, synthetic construct
  misc_feature 1..17: note = source = /note="Description of Artificial Sequence: Synthetic primer"
  source 1..17: mol_type = other DNA
caggaaacagctatgac

SEQ ID NO: 115 - DNA, 39 bp, synthetic construct
  misc_feature 1..39: note = source = /note="Description of Artificial Sequence: Synthetic primer"
  source 1..39: mol_type = other DNA
gcctctagaggtacctgagggcctatttcccatgattcc

SEQ ID NO: 116 - DNA, 133 bp, synthetic construct
  modified_base 92..111: mod_base = OTHER; note = a, c, t, g, unknown or other
  misc_feature 1..133: note = source = /note="Description of Artificial Sequence: Synthetic primer"
  source 1..133: mol_type = other DNA
acctctagaaaaaaagcaccgactcggtgccactttttcaagttgataacggactagccttattttaacttgctatttctagctctaaaacnnnnnnnnnnnnnnnnnnnnggtgtttcgtcctttccacaag

SEQ ID NO: 117 - DNA, 133 bp, synthetic construct
  modified_base 92..111: mod_base = OTHER; note = a, c, t, g, unknown or other
  misc_feature 1..133: note = source = /note="Description of Artificial Sequence: Synthetic primer"
  source 1..133: mol_type = other DNA
acctctagaaaaaaagcaccgactcggtgccactttttcaagttgataacggactagccttatattaacttgctatttctagctctaatacnnnnnnnnnnnnnnnnnnnnggtgtttcgtcctttccacaag

SEQ ID NO: 118 - DNA, 153 bp, synthetic construct
  modified_base 112..131: mod_base = OTHER; note = a, c, t, g, unknown or other
  misc_feature 1..153: note = source = /note="Description of Artificial Sequence: Synthetic primer"
  source 1..153: mol_type = other DNA
acctctagaaaaaaagcaccgactcggtgccactttttcaagttgataacggactagccttattttaacttgctatgctgttttgtttccaaaacagcatagctctaaaacnnnnnnnnnnnnnnnnnnnnggtgtttcgtcctttccacaag

SEQ ID NO: 119 - DNA, 153 bp, synthetic construct
  modified_base 112..131: mod_base = OTHER; note = a, c, t, g, unknown or other
  misc_feature 1..153: note = source = /note="Description of Artificial Sequence: Synthetic primer"
  source 1..153: mol_type = other DNA
acctctagaaaaaaagcaccgactcggtgccactttttcaagttgataacggactagccttatattaacttgctatgctgtattgtttccaatacagcatagctctaatacnnnnnnnnnnnnnnnnnnnnggtgtttcgtcctttccacaag

SEQ ID NO: 120 - DNA, 335 bp, synthetic construct
  misc_feature 1..335: note = source = /note="Description of Artificial Sequence: Synthetic polynucleotide"
  source 1..335: mol_type = other DNA
gagggcctatttcccatgattccttcatatttgcatatacgatacaaggctgttagagagataattggaattaatttgactgtaaacacaaagatattagtacaaaatacgtgacgtagaaagtaataatttcttgggtagtttgcagttttaaaattatgttttaaaatggactatcatatgcttaccgtaacttgaaagtatttcgatttcttggctttatatatcttgtggaaaggacgaaacaccggaaccattcaaaacagcatagcaagttaaaataaggctagtccgttatcaacttgaaaaagtggcaccgagtcggtgcttttttt

SEQ ID NO: 121 - DNA, 360 bp, synthetic construct
  modified_base 288..317: mod_base = OTHER; note = a, c, t, g, unknown or other
  misc_feature 1..360: note = source = /note="Description of Artificial Sequence: Synthetic polynucleotide"
  source 1..360: mol_type = other DNA
gagggcctatttcccatgattccttcatatttgcatatacgatacaaggctgttagagagataattggaattaatttgactgtaaacacaaagatattagtacaaaatacgtgacgtagaaagtaataatttcttgggtagtttgcagttttaaaattatgttttaaaatggactatcatatgcttaccgtaacttgaaagtatttcgatttcttggctttatatatcttgtggaaaggacgaaacaccgggttttagagctatgctgttttgaatggtcccaaaacnnnnnnnnnnnnnnnnnnnnnnnnnnnnnngttttagagctatgctgttttgaatggtcccaaaacttttttt

SEQ ID NO: 122 - DNA, 318 bp, synthetic construct
  modified_base 250..269: mod_base = OTHER; note = a, c, t, g, unknown or other
  misc_feature 1..318: note = source = /note="Description of Artificial Sequence: Synthetic polynucleotide"
  source 1..318: mol_type = other DNA
gagggcctatttcccatgattccttcatatttgcatatacgatacaaggctgttagagagataattggaattaatttgactgtaaacacaaagatattagtacaaaatacgtgacgtagaaagtaataatttcttgggtagtttgcagttttaaaattatgttttaaaatggactatcatatgcttaccgtaacttgaaagtatttcgatttcttggctttatatatcttgtggaaaggacgaaacaccnnnnnnnnnnnnnnnnnnnngttttagagctagaaatagcaagttaaaataaggctagtccgttttttt

SEQ ID NO: 123 - DNA, 325 bp, synthetic construct
  modified_base 250..269: mod_base = OTHER; note = a, c, t, g, unknown or other
  misc_feature 1..325: note = source = /note="Description of Artificial Sequence: Synthetic polynucleotide"
  source 1..325: mol_type = other DNA
gagggcctatttcccatgattccttcatatttgcatatacgatacaaggctgttagagagataattggaattaatttgactgtaaacacaaagatattagtacaaaatacgtgacgtagaaagtaataatttcttgggtagtttgcagttttaaaattatgttttaaaatggactatcatatgcttaccgtaacttgaaagtatttcgatttcttggctttatatatcttgtggaaaggacgaaacaccnnnnnnnnnnnnnnnnnnnngttttagagctagaaatagcaagttaaaataaggctagtccgttatcatttttttt

SEQ ID NO: 124 - DNA, 337 bp, synthetic construct
  modified_base 250..269: mod_base = OTHER; note = a, c, t, g, unknown or other
  misc_feature 1..337: note = source = /note="Description of Artificial Sequence: Synthetic polynucleotide"
  source 1..337: mol_type = other DNA
gagggcctatttcccatgattccttcatatttgcatatacgatacaaggctgttagagagataattggaattaatttgactgtaaacacaaagatattagtacaaaatacgtgacgtagaaagtaataatttcttgggtagtttgcagttttaaaattatgttttaaaatggactatcatatgcttaccgtaacttgaaagtatttcgatttcttggctttatatatcttgtggaaaggacgaaacaccnnnnnnnnnnnnnnnnnnnngttttagagctagaaatagcaagttaaaataaggctagtccgttatcaacttgaaaaagtgttttttt

SEQ ID NO: 125 - DNA, 352 bp, synthetic construct
  modified_base 250..269: mod_base = OTHER; note = a, c, t, g, unknown or other
  misc_feature 1..352: note = source = /note="Description of Artificial Sequence: Synthetic polynucleotide"
  source 1..352: mol_type = other DNA
gagggcctatttcccatgattccttcatatttgcatatacgatacaaggctgttagagagataattggaattaatttgactgtaaacacaaagatattagtacaaaatacgtgacgtagaaagtaataatttcttgggtagtttgcagttttaaaattatgttttaaaatggactatcatatgcttaccgtaacttgaaagtatttcgatttcttggctttatatatcttgtggaaaggacgaaacaccnnnnnnnnnnnnnnnnnnnngttttagagctagaaatagcaagttaaaataaggctagtccgttatcaacttgaaaaagtggcaccgagtcggtgcttttttt

SEQ ID NO: 126 - DNA, 5101 bp, synthetic construct
  misc_feature 1..5101: note = source = /note="Description of Artificial Sequence: Synthetic polynucleotide"
  source 1..5101: mol_type = other DNA
cgttacataacttacggtaaatggcccgcctggctgaccgcccaacgacccccgcccattgacgtcaataatgacgtatgttcccatagtaacgccaatagggactttccattgacgtcaatgggtggagtatttacggtaaactgcccacttggcagtacatcaagtgtatcatatgccaagtacgccccctattgacgtcaatgacggtaaatggcccgcctggcattatgcccagtacatgaccttatgggactttcctacttggcagtacatctacgtattagtcatcgctattaccatggtcgaggtgagccccacgttctgcttcactctccccatctcccccccctccccacccccaattttgtatttatttattttttaattattttgtgcagcgatgggggcggggggggggggggggcgcgcgccaggcggggcggggcggggcgaggggcggggcggggcgaggcggagaggtgcggcggcagccaatcagagcggcgcgctccgaaagtttccttttatggcgaggcggcggcggcggcggccctataaaaagcgaagcgcgcggcgggcgggagtcgctgcgacgctgccttcgccccgtgccccgctccgccgccgcctcgcgccgcccgccccggctctgactgaccgcgttactcccacaggtgagcgggcgggacggcccttctcctccgggctgtaattagctgagcaagaggtaagggtttaagggatggttggttggtggggtattaatgtttaattacctggagcacctgcctgaaatcactttttttcaggttggaccggtgccaccatggactataaggaccacgacggagactacaaggatcatgatattgattacaaagacgatgacgataagatggccccaaagaagaagcggaaggtcggtatccacggagtcccagcagccgacaagaagtacagcatcggcctggacatcggcaccaactctgtgggctgggccgtgatcaccgacgagtacaaggtgcccagcaagaaattcaaggtgctgggcaacaccgaccggcacagcatcaagaagaacctgatcggagccctgctgttcgacagcggcgaaacagccgaggccacccggctgaagagaaccgccagaagaagatacaccagacggaagaaccggatctgctatctgcaagagatcttcagcaacgagatggccaaggtggacgacagcttcttccacagactggaagagtccttcctggtggaagaggataagaagcacgagcggcaccccatcttcggcaacatcgtggacgaggtggcctaccacgagaagtaccccaccatctaccacctgagaaagaaactggtggacagcaccgacaaggccgacctgcggctgatctatctggccctggcccacatgatcaagttccggggccacttcctgatcgagggcgacctgaaccccgacaacagcgacgtggacaagctgttcatccagctggtgcagacctacaaccagctgttcgaggaaaaccccatcaacgccagcggcgtggacgccaaggccatcctgtctgccagactgagcaagagcagacggctggaaaatctgatcgcccagctgcccggcgagaagaagaatggcctgttcggcaacctgattgccctgagcctgggcctgacccccaacttcaagagcaacttcgacctggccgaggatgccaaactgcagctgagcaaggacacctacgacgacgacctggacaacctgctggcccagatcggcgaccagtacgccgacctgtttctggccgccaagaacctgtccgacgccatcctgctgagcgacatcctgagagtgaacaccgagatcaccaaggcccccctgagcgcctctatgatcaagagatacgacgagcaccaccaggacctgaccctgctgaaagctctcgtgcggcagcagctgcctgagaagtacaaagagattttcttcgaccagagcaagaacggctacgccggctacattgacggcggagccagccaggaagagttctacaagttcatcaagcccatcctggaaaagatggacggcaccgaggaactgctcgtgaagctgaacagagaggacctgctgcggaagcagcggaccttcgacaacggcagcatcccccaccagatccacctgggagagctgcacgccattctgcggcggcaggaagatttttacccattcctgaaggacaaccgggaaaagatcgagaagatcctgaccttccgcatcccctactacgtgggccctctggccaggggaaacagcagattcgcctggatgaccagaaagagcgaggaaaccatcaccccctggaacttcgaggaagtggtggacaagggcgcttccgcccagagcttcatcgagcggatgaccaacttcgataagaacctgcccaacgagaaggtgctgcccaagcacagcctgctgtacgagtacttcaccgtgtataacgagctgaccaaagtgaaatacgtgaccgagggaatgagaaagcccgccttcctgagcggcgagcagaaaaaggccatcgtggacctgctgttcaagaccaaccggaaagtgaccgtgaagcagctgaaagaggactacttcaagaaaatcgagtgcttcgactccgtggaaatctccggcgtggaagatcggttcaacgcctccctgggcacataccacgatctgctgaaaattatcaaggacaaggacttcctggacaatgaggaaaacgaggacattctggaagatatcgtgctgaccctgacactgtttgaggacagagagatgatcgaggaacggctgaaaacctatgcccacctgttcgacgacaaagtgatgaagcagctgaagcggcggagatacaccggctggggcaggctgagccggaagctgatcaacggcatccgggacaagcagtccggcaagacaatcctggatttcctgaagtccgacggcttcgccaacagaaacttcatgcagctgatccacgacgacagcctgacctttaaagaggacatccagaaagcccaggtgtccggccagggcgatagcctgcacgagcacattgccaatctggccggcagccccgccattaagaagggcatcctgcagacagtgaaggtggtggacgagctcgtgaaagtgatgggccggcacaagcccgagaacatcgtgatcgaaatggccagagagaaccagaccacccagaagggacagaagaacagccgcgagagaatgaagcggatcgaagagggcatcaaagagctgggcagccagatcctgaaagaacaccccgtggaaaacacccagctgcagaacgagaagctgtacctgtactacctgcagaatgggcgggatatgtacgtggaccaggaactggacatcaaccggctgtccgactacgatgtggaccatatcgtgcctcagagctttctgaaggacgactccatcgacaacaaggtgctgaccagaagcgacaagaaccggggcaagagcgacaacgtgccctccgaagaggtcgtgaagaagatgaagaactactggcggcagctgctgaacgccaagctgattacccagagaaagttcgacaatctgaccaaggccgagagaggcggcctgagcgaactggataaggccggcttcatcaagagacagctggtggaaacccggcagatcacaaagcacgtggcacagatcctggactcccggatgaacactaagtacgacgagaatgacaagctgatccgggaagtgaaagtgatcaccctgaagtccaagctggtgtccgatttccggaaggatttccagttttacaaagtgcgcgagatcaacaactaccaccacgcccacgacgcctacctgaacgccgtcgtgggaaccgccctgatcaaaaagtaccctaagctggaaagcgagttcgtgtacggcgactacaaggtgtacgacgtgcggaagatgatcgccaagagcgagcaggaaatcggcaaggctaccgccaagtacttcttctacagcaacatcatgaactttttcaagaccgagattaccctggccaacggcgagatccggaagcggcctctgatcgagacaaacggcgaaaccggggagatcgtgtgggataagggccgggattttgccaccgtgcggaaagtgctgagcatgccccaagtgaatatcgtgaaaaagaccgaggtgcagacaggcggcttcagcaaagagtctatcctgcccaagaggaacagcgataagctgatcgccagaaagaaggactgggaccctaagaagtacggcggcttcgacagccccaccgtggcctattctgtgctggtggtggccaaagtggaaaagggcaagtccaagaaactgaagagtgtgaaagagctgctggggatcaccatcatggaaagaagcagcttcgagaagaatcccatcgactttctggaagccaagggctacaaagaagtgaaaaaggacctgatcatcaagctgcctaagtactccctgttcgagctggaaaacggccggaagagaatgctggcctctgccggcgaactgcagaagggaaacgaactggccctgccctccaaatatgtgaacttcctgtacctggccagccactatgagaagctgaagggctcccccgaggataatgagcagaaacagctgtttgtggaacagcacaagcactacctggacgagatcatcgagcagatcagcgagttctccaagagagtgatcctggccgacgctaatctggacaaagtgctgtccgcctacaacaagcaccgggataagcccatcagagagcaggccgagaatatcatccacctgtttaccctgaccaatctgggagcccctgccgccttcaagtactttgacaccaccatcgaccggaagaggtacaccagcaccaaagaggtgctggacgccaccctgatccaccagagcatcaccggcctgtacgagacacggatcgacctgtctcagctgggaggcgactttctttttcttagcttgaccagctttcttagtagcagcaggacgctttaa

SEQ ID NO: 127 - DNA, 123 bp, synthetic construct
  misc_feature 1..123: note = source = /note="Description of Artificial Sequence: Synthetic polynucleotide"
  source 1..123: mol_type = other DNA
ccaatggggaggacatcgatgtcacctccaatgactagggtgggcaaccacaaacccacgagggcagagtgctgcttgctgctggccaggcccctgcgtgggcccaagctggactctggccac

SEQ ID NO: 128 - DNA, 121 bp, synthetic construct
  misc_feature 1..121: note = source = /note="Description of Artificial Sequence: Synthetic polynucleotide"
  source 1..121: mol_type = other DNA
cgagcagaagaagaagggctcccatcacatcaaccggtggcgcattgccacgaagcaggccaatggggaggacatcgatgtcacctccaatgactagggtgggcaaccacaaacccacgag

SEQ ID NO: 129 - DNA, 128 bp, synthetic construct
  misc_feature 1..128: note = source = /note="Description of Artificial Sequence: Synthetic polynucleotide"
  source 1..128: mol_type = other DNA
ggaggacaaagtacaaacggcagaagctggaggaggaagggcctgagtccgagcagaagaagaagggctcccatcacatcaaccggtggcgcattgccacgaagcaggccaatggggaggacatcgat

SEQ ID NO: 130 - DNA, 130 bp, synthetic construct
  misc_feature 1..130: note = source = /note="Description of Artificial Sequence: Synthetic polynucleotide"
  source 1..130: mol_type = other DNA
agaagctggaggaggaagggcctgagtccgagcagaagaagaagggctcccatcacatcaaccggtggcgcattgccacgaagcaggccaatggggaggacatcgatgtcacctccaatgactagggtgg

SEQ ID NO: 131 - DNA, 125 bp, synthetic construct
  misc_feature 1..125: note = source = /note="Description of Artificial Sequence: Synthetic polynucleotide"
  source 1..125: mol_type = other DNA
cctcagtcttcccatcaggctctcagctcagcctgagtgttgaggccccagtggctgctctgggggcctcctgagtttctcatctgtgcccctccctccctggcccaggtgaaggtgtggttcca

SEQ ID NO: 132 - DNA, 129 bp, synthetic construct
  misc_feature 1..129: note = source = /note="Description of Artificial Sequence: Synthetic polynucleotide"
  source 1..129: mol_type = other DNA
tcatctgtgcccctccctccctggcccaggtgaaggtgtggttccagaaccggaggacaaagtacaaacggcagaagctggaggaggaagggcctgagtccgagcagaagaagaagggctcccatcaca

SEQ ID NO: 133 - DNA, 129 bp, synthetic construct
  misc_feature 1..129: note = source = /note="Description of Artificial Sequence: Synthetic polynucleotide"
  source 1..129: mol_type = other DNA
ctccaatgactagggtgggcaaccacaaacccacgagggcagagtgctgcttgctgctggccaggcccctgcgtgggcccaagctggactctggccactccctggccaggctttggggaggcctggagt

SEQ ID NO: 134 - DNA, 127 bp, synthetic construct
  misc_feature 1..127: note = source = /note="Description of Artificial Sequence: Synthetic polynucleotide"
  source 1..127: mol_type = other DNA
ctgcttgctgctggccaggcccctgcgtgggcccaagctggactctggccactccctggccaggctttggggaggcctggagtcatggccccacagggcttgaagcccggggccgccattgacagag

SEQ ID NO: 135 - DNA, 25 bp, synthetic construct
  misc_feature 1..25: note = source = /note="Description of Artificial Sequence: Synthetic primer"
  source 1..25: mol_type = other DNA
gaaattaatacgactcactataggg

SEQ ID NO: 136 - DNA, 126 bp, synthetic construct
  misc_feature 1..126: note = source = /note="Description of Artificial Sequence: Synthetic polynucleotide"
  source 1..126: mol_type = other DNA
aaaaaagcaccgactcggtgccactttttcaagttgataacggactagccttattttaacttgctatttctagctctaaaacaacgacgagcgtgacaccaccctatagtgagtcgtattaatttc

SEQ ID NO: 137 - DNA, 126 bp, synthetic construct
  misc_feature 1..126: note = source = /note="Description of Artificial Sequence: Synthetic polynucleotide"
  source 1..126: mol_type = other DNA
aaaaaagcaccgactcggtgccactttttcaagttgataacggactagccttattttaacttgctatttctagctctaaaacgcaacaattaatagactggacctatagtgagtcgtattaatttc

SEQ ID NO: 138 - DNA, 102 bp, synthetic construct
  misc_feature 1..102: note = source = /note="Description of Artificial Sequence: Synthetic polynucleotide"
  source 1..102: mol_type = other DNA
gttttagagctatgctgttttgaatggtcccaaaacggaagggcctgagtccgagcagaagaagaagttttagagctatgctgttttgaatggtcccaaaac

SEQ ID NO: 139 - DNA, 100 bp, Homo sapiens
  source 1..100: mol_type = unassigned DNA
cggaggacaaagtacaaacggcagaagctggaggaggaagggcctgagtccgagcagaagaagaagggctcccatcacatcaaccggtggcgcattgcca

SEQ ID NO: 140 - DNA, 50 bp, Homo sapiens
  source 1..50: mol_type = unassigned DNA
agctggaggaggaagggcctgagtccgagcagaagaagaagggctcccac

SEQ ID NO: 141 - RNA, 30 nt, synthetic construct
  misc_feature 1..30: note = source = /note="Description of Artificial Sequence: Synthetic oligonucleotide"
  source 1..30: mol_type = other RNA
gagtccgagcagaagaagaagttttagagc

SEQ ID NO: 142 - DNA, 49 bp, Homo sapiens
  source 1..49: mol_type = unassigned DNA
agctggaggaggaagggcctgagtccgagcagaagagaagggctcccat

SEQ ID NO: 143 - DNA, 53 bp, Homo sapiens
  source 1..53: mol_type = unassigned DNA
ctggaggaggaagggcctgagtccgagcagaagaagaagggctcccatcacat

SEQ ID NO: 144 - DNA, 52 bp, Homo sapiens
  source 1..52: mol_type = unassigned DNA
ctggaggaggaagggcctgagtccgagcagaagagaagggctcccatcacat

SEQ ID NO: 145 - DNA, 54 bp, Homo sapiens
  source 1..54: mol_type = unassigned DNA
ctggaggaggaagggcctgagtccgagcagaagaaagaagggctcccatcacat

SEQ ID NO: 146 - DNA, 50 bp, Homo sapiens
  source 1..50: mol_type = unassigned DNA
ctggaggaggaagggcctgagtccgagcagaagaagggctcccatcacat

SEQ ID NO: 147 - DNA, 47 bp, Homo sapiens
  source 1..47: mol_type = unassigned DNA
ctggaggaggaagggcctgagcccgagcagaagggctcccatcacat

SEQ ID NO: 148 - DNA, 23 bp, Homo sapiens
  source 1..23: mol_type = unassigned DNA
gtcacctccaatgactagggtgg

SEQ ID NO: 149 - DNA, 23 bp, Homo sapiens
  source 1..23: mol_type = unassigned DNA
gcgccaccggttgatgtgatggg

SEQ ID NO: 150 - RNA, 99 nt, synthetic construct
  modified_base 1..20: mod_base = OTHER; note = a, c, u, g, unknown or other
  misc_feature 1..99: note = source = /note="Description of Artificial Sequence: Synthetic oligonucleotide"
  source 1..99: mol_type = other RNA
nnnnnnnnnnnnnnnnnnnngttttagagctagaaatagcaagttaaaataaggctagtccgttatcaacttgaaaaagtggcaccgagtcggtgcttt

SEQ ID NO: 151 - DNA, 64 bp, Homo sapiens
  source 1..64: mol_type = unassigned DNA
caagaggcttgagtaggagaggagtgccgccgaggcggggcggggcggggcgtggagctgggct

SEQ ID NO: 152 - RNA, 20 nt, synthetic construct
  misc_feature 1..20: note = source = /note="Description of Artificial Sequence: Synthetic oligonucleotide"
  source 1..20: mol_type = other RNA
gtcacctccaatgactaggg

SEQ ID NO: 153 - RNA, 20 nt, synthetic construct
  misc_feature 1..20: note = source = /note="Description of Artificial Sequence: Synthetic oligonucleotide"
  source 1..20: mol_type = other RNA
gtcacctccaatgactaaga

SEQ ID NO: 154 - RNA, 20 nt, synthetic construct
  misc_feature 1..20: note = source = /note="Description of Artificial Sequence: Synthetic oligonucleotide"
  source 1..20: mol_type = other RNA
gtcacctccaatgattagga

SEQ ID NO: 155 - RNA, 20 nt, synthetic construct
  misc_feature 1..20: note = source = /note="Description of Artificial Sequence: Synthetic oligonucleotide"
  source 1..20: mol_type = other RNA
gtcacctccagtgactagga

SEQ ID NO: 156 - RNA, 20 nt, synthetic construct
  misc_feature 1..20: note = source = /note="Description of Artificial Sequence: Synthetic oligonucleotide"
  source 1..20: mol_type = other RNA
gtcacttccaatgactagga

SEQ ID NO: 157 - RNA, 20 nt, synthetic construct
  misc_feature 1..20: note = source = /note="Description of Artificial Sequence: Synthetic oligonucleotide"
  source 1..20: mol_type = other RNA
atcacctccaatgactagga

SEQ ID NO: 158 - RNA, 20 nt, synthetic construct
  misc_feature 1..20: note = source = /note="Description of Artificial Sequence: Synthetic oligonucleotide"
  source 1..20: mol_type = other RNA
gtcacctccaatgaccaagg

SEQ ID NO: 159 - RNA, 20 nt, synthetic construct
  misc_feature 1..20: note = source = /note="Description of Artificial Sequence: Synthetic oligonucleotide"
  source 1..20: mol_type = other RNA
gtcacctccaataactaagg

SEQ ID NO: 160 - RNA, 20 nt, synthetic construct
  misc_feature 1..20: note = source = /note="Description of Artificial Sequence: Synthetic oligonucleotide"
  source 1..20: mol_type = other RNA
gtcacctctaatgactaagg

SEQ ID NO: 161 - RNA, 20 nt, synthetic construct
  misc_feature 1..20: note = source = /note="Description of Artificial Sequence: Synthetic oligonucleotide"
  source 1..20: mol_type = other RNA
gtcgcctccaatgactaagg

SEQ ID NO: 162 - RNA, 20 nt, synthetic construct
  misc_feature 1..20: note = source = /note="Description of Artificial Sequence: Synthetic oligonucleotide"
  source 1..20: mol_type = other RNA
gtcacctccaatggccaggg

SEQ ID NO: 163 - RNA, 20 nt, synthetic construct
  misc_feature 1..20: note = source = /note="Description of Artificial Sequence: Synthetic oligonucleotide"
  source 1..20: mol_type = other RNA
gtcacctccagtgaccaggg

SEQ ID NO: 164 - RNA, 20 nt, synthetic construct
  misc_feature 1..20: note = source = /note="Description of Artificial Sequence: Synthetic oligonucleotide"
  source 1..20: mol_type = other RNA
gtcacccccaatgaccaggg

SEQ ID NO: 165 - RNA, 20 nt, synthetic construct
  misc_feature 1..20: note = source = /note="Description of Artificial Sequence: Synthetic oligonucleotide"
  source 1..20: mol_type = other RNA
gccacctccaatgaccaggg

SEQ ID NO: 166 - RNA, 20 nt, synthetic construct
  misc_feature 1..20: note = source = /note="Description of Artificial Sequence: Synthetic oligonucleotide"
  source 1..20: mol_type = other RNA
gtcacctccaatgaccaaga

SEQ ID NO: 167 - RNA, 20 nt, synthetic construct
  misc_feature 1..20: note = source = /note="Description of Artificial Sequence: Synthetic oligonucleotide"
  source 1..20: mol_type = other RNA
gtcacctccaatggctggga

SEQ ID NO: 168 - RNA, 20 nt, synthetic construct
  misc_feature 1..20: note = source = /note="Description of Artificial Sequence: Synthetic oligonucleotide"
  source 1..20: mol_type = other RNA
gtcacctccaacgaccagga

SEQ ID NO: 169 - RNA, 20 nt, synthetic construct
  misc_feature 1..20: note = source = /note="Description of Artificial Sequence: Synthetic oligonucleotide"
  source 1..20: mol_type = other RNA
gtcacctccgatgattagga

SEQ ID NO: 170 - RNA, 20 nt, synthetic construct
  misc_feature 1..20: note = source = /note="Description of Artificial Sequence: Synthetic oligonucleotide"
  source 1..20: mol_type = other RNA
gtcacctccaatggccaagg

SEQ ID NO: 171 - RNA, 20 nt, synthetic construct
  misc_feature 1..20: note = source = /note="Description of Artificial Sequence: Synthetic oligonucleotide"
  source 1..20: mol_type = other RNA
gtcacctccaacgattaagg

SEQ ID NO: 172 - RNA, 20 nt, synthetic construct
  misc_feature 1..20: note = source = /note="Description of Artificial Sequence: Synthetic oligonucleotide"
  source 1..20: mol_type = other RNA
gtcacctccgatggctaagg

SEQ ID NO: 173 - RNA, 20 nt, synthetic construct
  misc_feature 1..20: note = source = /note="Description of Artificial Sequence: Synthetic oligonucleotide"
  source 1..20: mol_type = other RNA
gtcaccttcaataactaagg

SEQ ID NO: 174 - RNA, 20 nt, synthetic construct
  misc_feature 1..20: note = source = /note="Description of Artificial Sequence: Synthetic oligonucleotide"
  source 1..20: mol_type = other RNA
gtcacctccaatggccaaga

SEQ ID NO: 175 - RNA, 20 nt, synthetic construct
  misc_feature 1..20: note = source = /note="Description of Artificial Sequence: Synthetic oligonucleotide"
  source 1..20: mol_type = other RNA
gtcacctccagtggctggga

SEQ ID NO: 176 - RNA, 20 nt, synthetic construct
  misc_feature 1..20: note = source = /note="Description of Artificial Sequence: Synthetic oligonucleotide"
  source 1..20: mol_type = other RNA
gtcaccttcaacgaccagga

SEQ ID NO: 177 - RNA, 20 nt, synthetic construct
  misc_feature 1..20: note = source = /note="Description of Artificial Sequence: Synthetic oligonucleotide"
  source 1..20: mol_type = other RNA
gtcatctccgatgattagga

SEQ ID NO: 178 - RNA, 20 nt, synthetic construct
  misc_feature 1..20: note = source = /note="Description of Artificial Sequence: Synthetic oligonucleotide"
  source 1..20: mol_type = other RNA
gccaccttcaatggctagga

SEQ ID NO: 179 - RNA, 20 nt, synthetic construct
  misc_feature 1..20: note = source = /note="Description of Artificial Sequence: Synthetic oligonucleotide"
  source 1..20: mol_type = other RNA
gtcacctccaatgactagaa

SEQ ID NO: 180 - RNA, 20 nt, synthetic construct
  misc_feature 1..20: note = source = /note="Description of Artificial Sequence: Synthetic oligonucleotide"
  source 1..20: mol_type = other RNA
gtcacctccaatgactgagg

SEQ ID NO: 181 - RNA, 20 nt, synthetic construct
  misc_feature 1..20: note = source = /note="Description of Artificial Sequence: Synthetic oligonucleotide"
  source 1..20: mol_type = other RNA
gtcacctccaatgatcaggg

SEQ ID NO: 182 - RNA, 20 nt, synthetic construct
  misc_feature 1..20: note = source = /note="Description of Artificial Sequence: Synthetic oligonucleotide"
  source 1..20: mol_type = other RNA
gtcacctccaatagctaggg

SEQ ID NO: 183 - RNA, 20 nt, synthetic construct
  misc_feature 1..20: note = source = /note="Description of Artificial Sequence: Synthetic oligonucleotide"
  source 1..20: mol_type = other RNA
gtcacctccagcgactaggg

SEQ ID NO: 184 - RNA, 20 nt, synthetic construct
  misc_feature 1..20: note = source = /note="Description of Artificial Sequence: Synthetic oligonucleotide"
  source 1..20: mol_type = other RNA
gtcacctctgatgactaggg

SEQ ID NO: 185 - RNA, 20 nt, synthetic construct
  misc_feature 1..20: note = source = /note="Description of Artificial Sequence: Synthetic oligonucleotide"
  source 1..20: mol_type = other RNA
gtcaccctcaatgactaggg

SEQ ID NO: 186 - RNA, 20 nt, synthetic construct
  misc_feature 1..20: note = source = /note="Description of Artificial Sequence: Synthetic oligonucleotide"
  source 1..20: mol_type = other RNA
gtcatttccaatgactaggg

SEQ ID NO: 187 - RNA, 20 nt, synthetic construct
  misc_feature 1..20: note = source = /note="Description of Artificial Sequence: Synthetic oligonucleotide"
  source 1..20: mol_type = other RNA
gttgcctccaatgactaggg

SEQ ID NO: 188 - RNA, 20 nt, synthetic construct
  misc_feature 1..20: note = source = /note="Description of Artificial Sequence: Synthetic oligonucleotide"
  source 1..20: mol_type = other RNA
accacctccaatgactaggg

SEQ ID NO: 189 - RNA, 20 nt, synthetic construct
  misc_feature 1..20: note = source = /note="Description of Artificial Sequence: Synthetic oligonucleotide"
  source 1..20: mol_type = other RNA
gtcacctccaatgactgaag

SEQ ID NO: 190 - RNA, 20 nt, synthetic construct
  misc_feature 1..20: note = source = /note="Description of Artificial Sequence: Synthetic oligonucleotide"
  source 1..20: mol_type = other RNA
gtcacctccaatggtcaggg

SEQ ID NO: 191 - RNA, 20 nt, synthetic construct
  misc_feature 1..20: note = source = /note="Description of Artificial Sequence: Synthetic oligonucleotide"
  source 1..20: mol_type = other RNA
gtcacctccagcaactaggg

SEQ ID NO: 192 - RNA, 20 nt, synthetic construct
  misc_feature 1..20: note = source = /note="Description of Artificial Sequence: Synthetic oligonucleotide"
  source 1..20: mol_type = other RNA
gtcacctttgatgactaggg

SEQ ID NO: 193 - RNA, 20 nt, synthetic construct
  misc_feature 1..20: note = source = /note="Description of Artificial Sequence: Synthetic oligonucleotide"
  source 1..20: mol_type = other RNA
gtcattcccaatgactaggg

SEQ ID NO: 194 - RNA, 20 nt, synthetic construct
  misc_feature 1..20: note = source = /note="Description of Artificial Sequence: Synthetic oligonucleotide"
  source 1..20: mol_type = other RNA
gctgcctccaatgactaggg

SEQ ID NO: 195 - RNA, 20 nt, synthetic construct
  misc_feature 1..20: note = source = /note="Description of Artificial Sequence: Synthetic oligonucleotide"
  source 1..20: mol_type = other RNA
gtcacctccaatgaccgaaa

SEQ ID NO: 196 - RNA, 20 nt, synthetic construct
  misc_feature 1..20: note = source = /note="Description of Artificial Sequence: Synthetic oligonucleotide"
  source 1..20: mol_type = other RNA
gtcacctccaatagtcgggg

SEQ ID NO: 197 - RNA, 20 nt, synthetic construct
  misc_feature 1..20: note = source = /note="Description of Artificial Sequence: Synthetic oligonucleotide"
  source 1..20: mol_type = other RNA
gtcacctccggcagctaggg

SEQ ID NO: 198 - RNA, 20 nt, synthetic construct
  misc_feature 1..20: note = source = /note="Description of Artificial Sequence: Synthetic oligonucleotide"
  source 1..20: mol_type = other RNA
gtcacccttggtgactaggg

SEQ ID NO: 199 - RNA, 20 nt, synthetic construct
  misc_feature 1..20: note = source = /note="Description of Artificial Sequence: Synthetic oligonucleotide"
  source 1..20: mol_type = other RNA
gtcgttctcaatgactaggg

SEQ ID NO: 200 - RNA, 20 nt, synthetic construct
  misc_feature 1..20: note = source = /note="Description of Artificial Sequence: Synthetic oligonucleotide"
  source 1..20: mol_type = other RNA
actgtctccaatgactaggg

SEQ ID NO: 201 - RNA, 20 nt, synthetic construct
  misc_feature 1..20: note = source = /note="Description of Artificial Sequence: Synthetic oligonucleotide"
  source 1..20: mol_type = other RNA
gcgccaccggttgatgtgat

SEQ ID NO: 202 - RNA, 20 nt, synthetic construct
  misc_feature 1..20: note = source = /note="Description of Artificial Sequence: Synthetic oligonucleotide"
  source 1..20: mol_type = other RNA
gcgccaccggttgatgtaac

SEQ ID NO: 203 - RNA, 20 nt, synthetic construct
  misc_feature 1..20: note = source = /note="Description of Artificial Sequence: Synthetic oligonucleotide"
  source 1..20: mol_type = other RNA
gcgccaccggttgacgtgac

SEQ ID NO: 204 - RNA, 20 nt, synthetic construct
  misc_feature 1..20: note = source = /note="Description of Artificial Sequence: Synthetic oligonucleotide"
  source 1..20: mol_type = other RNA
gcgccaccggctgatgtgac

SEQ ID NO: 205 - RNA, 20 nt, synthetic construct
  misc_feature 1..20: note = source = /note="Description of Artificial Sequence: Synthetic oligonucleotide"
  source 1..20: mol_type = other RNA
gcgccgccggttgatgtgac

SEQ ID NO: 206 - RNA, 20 nt, synthetic construct
  misc_feature 1..20: note = source = /note="Description of Artificial Sequence: Synthetic oligonucleotide"
  source 1..20: mol_type = other RNA
acgccaccggttgatgtgac

SEQ ID NO: 207 - RNA, 20 nt, synthetic construct
  misc_feature 1..20: note = source = /note="Description of Artificial Sequence: Synthetic oligonucleotide"
  source 1..20: mol_type = other RNA
gcgccaccggttgatataat

SEQ ID NO: 208 - RNA, 20 nt, synthetic construct
  misc_feature 1..20: note = source = /note="Description of Artificial Sequence: Synthetic oligonucleotide"
  source 1..20: mol_type = other RNA
gcgccaccggttaatgtaat

SEQ ID NO: 209 - RNA, 20 nt, synthetic construct
  misc_feature 1..20: note = source = /note="Description of Artificial Sequence: Synthetic oligonucleotide"
  source 1..20: mol_type = other RNA
gcgccaccagttgatgtaat

SEQ ID NO: 210 - RNA, 20 nt, synthetic construct
  misc_feature 1..20: note = source = /note="Description of Artificial Sequence: Synthetic oligonucleotide"
  source 1..20: mol_type = other RNA
gcgtcaccggttgatgtaat

SEQ ID NO: 211 - RNA, 20 nt, synthetic construct
  misc_feature 1..20: note = source = /note="Description of Artificial Sequence: Synthetic oligonucleotide"
  source 1..20: mol_type = other RNA
gcgccaccggttggtatgat

SEQ ID NO: 212 - RNA, 20 nt, synthetic construct
  misc_feature 1..20: note = source = /note="Description of Artificial Sequence: Synthetic oligonucleotide"
  source 1..20: mol_type = other RNA
gcgccaccggctgatatgat

SEQ ID NO: 213 - RNA, 20 nt, synthetic construct
  misc_feature 1..20: note = source = /note="Description of Artificial Sequence: Synthetic oligonucleotide"
  source 1..20: mol_type = other RNA
gcgccatcggttgatatgat

SEQ ID NO: 214 - RNA, 20 nt, synthetic construct
  misc_feature 1..20: note = source = /note="Description of Artificial Sequence: Synthetic oligonucleotide"
  source 1..20: mol_type = other RNA
gtgccaccggttgatatgat

SEQ ID NO: 215 - RNA, 20 nt, synthetic construct
  misc_feature 1..20: note = source = /note="Description of Artificial Sequence: Synthetic oligonucleotide"
  source 1..20: mol_type = other RNA
gcgccaccggttgatataac

SEQ ID NO: 216 - RNA, 20 nt, synthetic construct
  misc_feature 1..20: note = source = /note="Description of Artificial Sequence: Synthetic oligonucleotide"
  source 1..20: mol_type = other RNA
gcgccaccggttggtgcgac

SEQ ID NO: 217 - RNA, 20 nt, synthetic construct
  misc_feature 1..20: note = source = /note="Description of Artificial Sequence: Synthetic oligonucleotide"
  source 1..20: mol_type = other RNA
gcgccaccggtcgatatgac

SEQ ID NO: 218 - RNA, 20 nt, synthetic construct
  misc_feature 1..20: note = source = /note="Description of Artificial Sequence: Synthetic oligonucleotide"
  source 1..20: mol_type = other RNA
gcgccaccgattgacgtgac

SEQ ID NO: 219 - RNA, 20 nt, synthetic construct
  misc_feature 1..20: note = source = /note="Description of Artificial Sequence: Synthetic oligonucleotide"
  source 1..20: mol_type = other RNA
gcgccaccggttggtataat

SEQ ID NO: 220 - RNA, 20 nt, synthetic construct
  misc_feature 1..20: note = source = /note="Description of Artificial Sequence: Synthetic oligonucleotide"
  source 1..20: mol_type = other RNA
gcgccaccggtcgacgtaat

SEQ ID NO: 221 - RNA, 20 nt, synthetic construct
  misc_feature 1..20: note = source = /note="Description of Artificial Sequence: Synthetic oligonucleotide"
  source 1..20: mol_type = other RNA
gcgccaccgattggtgtaat

SEQ ID NO: 222 - RNA, 20 nt, synthetic construct
  misc_feature 1..20: note = source = /note="Description of Artificial Sequence: Synthetic oligonucleotide"
  source 1..20: mol_type = other RNA
gcgccactggttaatgtaat

SEQ ID NO: 223 - RNA, 20 nt, synthetic construct
  misc_feature 1..20: note = source = /note="Description of Artificial Sequence: Synthetic oligonucleotide"
  source 1..20: mol_type = other RNA
gcgccaccggttggtataac

SEQ ID NO: 224 - RNA, 20 nt, synthetic construct
  misc_feature 1..20: note = source = /note="Description of Artificial Sequence: Synthetic oligonucleotide"
  source 1..20: mol_type = other RNA
gcgccaccggctggtgcgac

SEQ ID NO: 225 - RNA, 20 nt, synthetic construct
  misc_feature 1..20: note = source = /note="Description of Artificial Sequence: Synthetic oligonucleotide"
  source 1..20: mol_type = other RNA
gcgccactggtcgatatgac

SEQ ID NO: 226 - RNA, 20 nt, synthetic construct
  misc_feature 1..20: note = source = /note="Description of Artificial Sequence: Synthetic oligonucleotide"
  source 1..20: mol_type = other RNA
gcgctaccgattgacgtgac

SEQ ID NO: 227 - RNA, 20 nt, synthetic construct
  misc_feature 1..20: note = source = /note="Description of Artificial Sequence: Synthetic oligonucleotide"
  source 1..20: mol_type = other RNA
gtgccactggttggtgtgac

SEQ ID NO: 228 - RNA, 20 nt, synthetic construct
  misc_feature 1..20: note = source = /note="Description of Artificial Sequence: Synthetic oligonucleotide"
  source 1..20: mol_type = other RNA
gcgccaccggttgatgtggc

SEQ ID NO: 229 - RNA, 20 nt, synthetic construct
  misc_feature 1..20: note = source = /note="Description of Artificial Sequence: Synthetic oligonucleotide"
  source 1..20: mol_type = other RNA
gcgccaccggttgatgcaat

SEQ ID NO: 230 - RNA, 20 nt, synthetic construct
  misc_feature 1..20: note = source = /note="Description of Artificial Sequence: Synthetic oligonucleotide"
  source 1..20: mol_type = other RNA
gcgccaccggttgacatgat

SEQ ID NO: 231 - RNA, 20 nt, synthetic construct
  misc_feature 1..20: note = source = /note="Description of Artificial Sequence: Synthetic oligonucleotide"
  source 1..20: mol_type = other RNA
gcgccaccggttagtgtgat

SEQ ID NO: 232 - RNA, 20 nt, synthetic construct
  misc_feature 1..20: note = source = /note="Description of Artificial Sequence: Synthetic oligonucleotide"
  source 1..20: mol_type = other RNA
gcgccaccggccgatgtgat

SEQ ID NO: 233 - RNA, 20 nt, synthetic construct
  misc_feature 1..20: note = source = /note="Description of Artificial Sequence: Synthetic oligonucleotide"
  source 1..20: mol_type = other RNA
gcgccaccaattgatgtgat

SEQ ID NO: 234 - RNA, 20 nt, synthetic construct
  misc_feature 1..20: note = source = /note="Description of Artificial Sequence: Synthetic oligonucleotide"
  source 1..20: mol_type = other RNA
gcgccattggttgatgtgat

SEQ ID NO: 235 - RNA, 20 nt, synthetic construct
  misc_feature 1..20: note = source = /note="Description of Artificial Sequence: Synthetic oligonucleotide"
  source 1..20: mol_type = other RNA
gcgctgccggttgatgtgat

SEQ ID NO: 236 - RNA, 20 nt, synthetic construct
  misc_feature 1..20: note = source = /note="Description of Artificial Sequence: Synthetic oligonucleotide"
  source 1..20: mol_type = other RNA
gcatcaccggttgatgtgat

SEQ ID NO: 237 - RNA, 20 nt, synthetic construct
  misc_feature 1..20: note = source = /note="Description of Artificial Sequence: Synthetic oligonucleotide"
  source 1..20: mol_type = other RNA
atgccaccggttgatgtgat

SEQ ID NO: 238 - RNA, 20 nt, synthetic construct
  misc_feature 1..20: note = source = /note="Description of Artificial Sequence: Synthetic oligonucleotide"
  source 1..20: mol_type = other RNA
gcgccaccggttgatgcagt

SEQ ID NO: 239 - RNA, 20 nt, synthetic construct
  misc_feature 1..20: note = source = /note="Description of Artificial Sequence: Synthetic oligonucleotide"
  source 1..20: mol_type = other RNA
gcgccaccggttggcatgat

SEQ ID NO: 240 - RNA, 20 nt, synthetic construct
  misc_feature 1..20: note = source = /note="Description of Artificial Sequence: Synthetic oligonucleotide"
  source 1..20: mol_type = other RNA
gcgccaccggccaatgtgat

SEQ ID NO: 241 - RNA, 20 nt, synthetic construct
  misc_feature 1..20: note = source = /note="Description of Artificial Sequence: Synthetic oligonucleotide"
  source 1..20: mol_type = other RNA
gcgccactaattgatgtgat

SEQ ID NO: 242 - RNA, 20 nt, synthetic construct
  misc_feature 1..20: note = source = /note="Description of Artificial Sequence: Synthetic oligonucleotide"
  source 1..20: mol_type = other RNA
gcgctgtcggttgatgtgat

SEQ ID NO: 243 - RNA, 20 nt, synthetic construct
  misc_feature 1..20: note = source = /note="Description of Artificial Sequence: Synthetic oligonucleotide"
  source 1..20: mol_type = other RNA
gtatcaccggttgatgtgat

SEQ ID NO: 244 - RNA, 20 nt, synthetic construct
  misc_feature 1..20: note = source = /note="Description of Artificial Sequence: Synthetic oligonucleotide"
  source 1..20: mol_type = other RNA
gcgccaccggttgatacagc

SEQ ID NO: 245 - RNA, 20 nt, synthetic construct
  misc_feature 1..20: note = source = /note="Description of Artificial Sequence: Synthetic oligonucleotide"
  source 1..20: mol_type = other RNA
gcgccaccggttagcacgat

SEQ ID NO: 246 - RNA, 20 nt, synthetic construct
  misc_feature 1..20: note = source = /note="Description of Artificial Sequence: Synthetic oligonucleotide"
  source 1..20: mol_type = other RNA
gcgccaccgaccagtgtgat

SEQ ID NO: 247 - RNA, 20 nt, synthetic construct
  misc_feature 1..20: note = source = /note="Description of Artificial Sequence: Synthetic oligonucleotide"
  source 1..20: mol_type = other RNA
gcgccattaactgatgtgat

SEQ ID NO: 248 - RNA, 20 nt, synthetic construct
  misc_feature 1..20: note = source = /note="Description of Artificial Sequence: Synthetic oligonucleotide"
  source 1..20: mol_type = other RNA
gcgttgttggttgatgtgat

SEQ ID NO: 249 - RNA, 20 nt, synthetic construct
  misc_feature 1..20: note = source = /note="Description of Artificial Sequence: Synthetic oligonucleotide"
  source 1..20: mol_type = other RNA
atattaccggttgatgtgat

SEQ ID NO: 250 - RNA, 20 nt, synthetic construct
  misc_feature 1..20: note = source = /note="Description of Artificial Sequence: Synthetic oligonucleotide"
  source 1..20: mol_type = other RNA
gtcacctccaatgactaggg

SEQ ID NO: 251 - RNA, 20 nt, synthetic construct
  misc_feature 1..20: note = source = /note="Description of Artificial Sequence: Synthetic oligonucleotide"
  source 1..20: mol_type = other RNA
gtcacctggaatgactaggg

SEQ ID NO: 252 - RNA, 20 nt, synthetic construct
  misc_feature 1..20: note = source = /note="Description of Artificial Sequence: Synthetic oligonucleotide"
  source 1..20: mol_type = other RNA
gtcacgaccaatgactaggg

SEQ ID NO: 253 - RNA, 20 nt, synthetic construct
  misc_feature 1..20: note = source = /note="Description of Artificial Sequence: Synthetic oligonucleotide"
  source 1..20: mol_type = other RNA
gtctgctccaatgactaggg

SEQ ID NO: 254 - RNA, 20 nt, synthetic construct
  misc_feature 1..20: note = source = /note="Description of Artificial Sequence: Synthetic oligonucleotide"
  source 1..20: mol_type = other RNA
gagacctccaatgactaggg

SEQ ID NO: 255 - RNA, 20 nt, synthetic construct
  misc_feature 1..20: note = source = /note="Description of Artificial Sequence: Synthetic oligonucleotide"
  source 1..20: mol_type = other RNA
gtcaccaggaatgactaggg

SEQ ID NO: 256 - RNA, 20 nt, synthetic construct
  misc_feature 1..20: note = source = /note="Description of Artificial Sequence: Synthetic oligonucleotide"
  source 1..20: mol_type = other RNA
gtctggtccaatgactaggg

SEQ ID NO: 257 - RNA, 20 nt, synthetic construct
  misc_feature 1..20: note = source = /note="Description of Artificial Sequence: Synthetic oligonucleotide"
  source 1..20: mol_type = other RNA
gagtcctccaatgactaggg

SEQ ID NO: 258 - RNA, 20 nt, synthetic construct
  misc_feature 1..20: note = source = /note="Description of Artificial Sequence: Synthetic oligonucleotide"
  source 1..20: mol_type = other RNA
gtcacgaggaatgactaggg

SEQ ID NO: 259 - RNA, 20 nt, synthetic construct
  misc_feature 1..20: note = source = /note="Description of Artificial Sequence: Synthetic oligonucleotide"
  source 1..20: mol_type = other RNA
gtctggaccaatgactaggg

SEQ ID NO: 260 - RNA, 20 nt, synthetic construct
  misc_feature 1..20: note = source = /note="Description of Artificial Sequence: Synthetic oligonucleotide"
  source 1..20: mol_type = other RNA
gagtgctccaatgactaggg

SEQ ID NO: 261 - RNA, 20 nt, synthetic construct
  misc_feature 1..20: note = source = /note="Description of Artificial Sequence: Synthetic oligonucleotide"
  source 1..20: mol_type = other RNA
gtctgctggaatgactaggg

SEQ ID NO: 262 - RNA, 20 nt, synthetic construct
  misc_feature 1..20: note = source = /note="Description of Artificial Sequence: Synthetic oligonucleotide"
  source 1..20: mol_type = other RNA
gagacgaccaatgactaggg

SEQ ID NO: 263 - RNA, 20 nt, synthetic construct
  misc_feature 1..20: note = source = /note="Description of Artificial Sequence: Synthetic oligonucleotide"
  source 1..20: mol_type = other RNA
gagacctggaatgactaggg

SEQ ID NO: 264 - DNA, 40 bp, Homo sapiens
  source 1..40: mol_type = unassigned DNA
ggacatcgatgtcacctccaatgactagggtgggcaacca

SEQ ID NO: 265 - RNA, 20 nt, synthetic construct
  misc_feature 1..20: note = source = /note="Description of Artificial Sequence: Synthetic oligonucleotide"
  source 1..20: mol_type = other RNA
gtcacctccaatgactaggg

SEQ ID NO: 266 - RNA, 20 nt, synthetic construct
  modified_base 20: mod_base = OTHER; note = a, c, u, g, unknown or other
  misc_feature 1..20: note = source = /note="Description of Artificial Sequence: Synthetic oligonucleotide"
  source 1..20: mol_type = other RNA
gtcacctccaatgactaggn

SEQ ID NO: 267 - RNA, 20 nt, synthetic construct
  modified_base 19: mod_base = OTHER; note = a, c, u, g, unknown or other
  misc_feature 1..20: note = source = /note="Description of Artificial Sequence: Synthetic oligonucleotide"
  source 1..20: mol_type = other RNA
gtcacctccaatgactagng

SEQ ID NO: 268 - RNA, 20 nt, synthetic construct
  modified_base 18: mod_base = OTHER; note = a, c, u, g, unknown or other
  misc_feature 1..20: note = source = /note="Description of Artificial Sequence: Synthetic oligonucleotide"
  source 1..20: mol_type = other RNA
gtcacctccaatgactangg

SEQ ID NO: 269 - RNA, 20 nt, synthetic construct
  modified_base 17: mod_base = OTHER; note = a, c, u, g, unknown or other
  misc_feature 1..20: note = source = /note="Description of Artificial Sequence: Synthetic oligonucleotide"
  source 1..20: mol_type = other RNA
gtcacctccaatgactnggg

SEQ ID NO: 270 - RNA, 20 nt, synthetic construct
  modified_base 16: mod_base = OTHER; note = a, c, u, g, unknown or other
  misc_feature 1..20: note = source = /note="Description of Artificial Sequence: Synthetic oligonucleotide"
  source 1..20: mol_type = other RNA
gtcacctccaatgacnaggg

SEQ ID NO: 271 - RNA, 20 nt, synthetic construct
  modified_base 15: mod_base = OTHER; note = a, c, u, g, unknown or other
  misc_feature 1..20: note = source = /note="Description of Artificial Sequence: Synthetic oligonucleotide"
  source 1..20: mol_type = other RNA
gtcacctccaatgantaggg

SEQ ID NO: 272 - RNA, 20 nt, synthetic construct
  modified_base 14: mod_base = OTHER; note = a, c, u, g, unknown or other
  misc_feature 1..20: note = source = /note="Description of Artificial Sequence: Synthetic oligonucleotide"
  source 1..20: mol_type = other RNA
gtcacctccaatgnctaggg

SEQ ID NO: 273 - RNA, 20 nt, synthetic construct
  modified_base 13: mod_base = OTHER; note = a, c, u, g, unknown or other
  misc_feature 1..20: note = source = /note="Description of Artificial Sequence: Synthetic oligonucleotide"
  source 1..20: mol_type = other RNA
gtcacctccaatnactaggg

SEQ ID NO: 274 - RNA, 20 nt, synthetic construct
  modified_base 12: mod_base = OTHER; note = a, c, u, g, unknown or other
  misc_feature 1..20: note = source = /note="Description of Artificial Sequence: Synthetic oligonucleotide"
  source 1..20: mol_type = other RNA
gtcacctccaangactaggg

SEQ ID NO: 275 - RNA, 20 nt, synthetic construct
  modified_base 11: mod_base = OTHER; note = a, c, u, g, unknown or other
  misc_feature 1..20: note = source = /note="Description of Artificial Sequence: Synthetic oligonucleotide"
  source 1..20: mol_type = other RNA
gtcacctccantgactaggg

SEQ ID NO: 276 - RNA, 20 nt, synthetic construct
  modified_base 10: mod_base = OTHER; note = a, c, u, g, unknown or other
  misc_feature 1..20: note = source = /note="Description of Artificial Sequence: Synthetic oligonucleotide"
  source 1..20: mol_type = other RNA
gtcacctccnatgactaggg

SEQ ID NO: 277 - RNA, 20 nt, synthetic construct
  modified_base 9: mod_base = OTHER; note = a, c, u, g, unknown or other
  misc_feature 1..20: note = source = /note="Description of Artificial Sequence: Synthetic oligonucleotide"
  source 1..20: mol_type = other RNA
gtcacctcnaatgactaggg

SEQ ID NO: 278 - RNA, 20 nt, synthetic construct
  modified_base 8: mod_base = OTHER; note = a, c, u, g, unknown or other
  misc_feature 1..20: note = source = /note="Description of Artificial Sequence: Synthetic oligonucleotide"
  source 1..20: mol_type = other RNA
gtcacctncaatgactaggg

SEQ ID NO: 279 - RNA, 20 nt, synthetic construct
  modified_base 7: mod_base = OTHER; note = a, c, u, g, unknown or other
  misc_feature 1..20: note = source = /note="Description of Artificial Sequence: Synthetic oligonucleotide"
  source 1..20: mol_type = other RNA
gtcaccnccaatgactaggg

SEQ ID NO: 280 - RNA, 20 nt, synthetic construct
  modified_base 6: mod_base = OTHER; note = a, c, u, g, unknown or other
  misc_feature 1..20: note = source = /note="Description of Artificial Sequence: Synthetic oligonucleotide"
  source 1..20: mol_type = other RNA
gtcacntccaatgactaggg

SEQ ID NO: 281 - RNA, 20 nt, synthetic construct
  modified_base 5: mod_base = OTHER; note = a, c, u, g, unknown or other
  misc_feature 1..20: note = source = /note="Description of Artificial Sequence: Synthetic oligonucleotide"
  source 1..20: mol_type = other RNA
gtcanctccaatgactaggg

SEQ ID NO: 282 - RNA, 20 nt, synthetic construct
  modified_base 4: mod_base = OTHER; note = a, c, u, g, unknown or other
  misc_feature 1..20: note = source = /note="Description of Artificial Sequence: Synthetic oligonucleotide"
  source 1..20: mol_type = other RNA
gtcncctccaatgactaggg

SEQ ID NO: 283 - RNA, 20 nt, synthetic construct
  modified_base 3: mod_base = OTHER; note = a, c, u, g, unknown or other
  misc_feature 1..20: note = source = /note="Description of Artificial Sequence: Synthetic oligonucleotide"
  source 1..20: mol_type = other RNA
gtnacctccaatgactaggg

SEQ ID NO: 284 - RNA, 20 nt, synthetic construct
  modified_base 2: mod_base = OTHER; note = a, c, u, g, unknown or other
  misc_feature 1..20: note = source = /note="Description of Artificial Sequence: Synthetic oligonucleotide"
  source 1..20: mol_type = other RNA
gncacctccaatgactaggg

SEQ ID NO: 285 - RNA, 20 nt, synthetic construct
  misc_feature 1..20: note = source = /note="Description of Artificial Sequence: Synthetic oligonucleotide"
  source 1..20: mol_type = other RNA
gtcacctccaatgactaggg

SEQ ID NO: 286 - RNA, 20 nt, synthetic construct
  misc_feature 1..20: note = source = /note="Description of Artificial Sequence: Synthetic oligonucleotide"
  source 1..20: mol_type = other RNA
gacatcgatgtcctccccat

SEQ ID NO: 287 - RNA, 20 nt, synthetic construct
  misc_feature 1..20: note = source = /note="Description of Artificial Sequence: Synthetic oligonucleotide"
  source 1..20: mol_type = other RNA
gcgccaccggttgatgtgat

SEQ ID NO: 288 - RNA, 20 nt, synthetic construct
  misc_feature 1..20: note = source = /note="Description of Artificial Sequence: Synthetic oligonucleotide"
  source 1..20: mol_type = other RNA
gtcacctccaatgactaggg

SEQ ID NO: 289 - RNA, 20 nt, synthetic construct
  misc_feature 1..20: note = source = /note="Description of Artificial Sequence: Synthetic oligonucleotide"
  source 1..20: mol_type = other RNA
gtcacctccaatgactagaa

SEQ ID NO: 290 - RNA, 20 nt, synthetic construct
  misc_feature 1..20: note = source = /note="Description of Artificial Sequence: Synthetic oligonucleotide"
  source 1..20: mol_type = other RNA
gtcacctccaatgactgagg

SEQ ID NO: 291 - RNA, 20 nt, synthetic construct
  misc_feature 1..20: note = source = /note="Description of Artificial Sequence: Synthetic oligonucleotide"
  source 1..20: mol_type = other RNA
gtcacctccaatgatcaggg

SEQ ID NO: 292 - RNA, 20 nt, synthetic construct
  misc_feature 1..20: note = source = /note="Description of Artificial Sequence: Synthetic oligonucleotide"
  source 1..20: mol_type = other RNA
gtcacctccaatagctaggg

SEQ ID NO: 293 - RNA, 20 nt, synthetic construct
  misc_feature 1..20: note = source = /note="Description of Artificial Sequence: Synthetic oligonucleotide"
  source 1..20: mol_type = other RNA
gtcacctccagcgactaggg

SEQ ID NO: 294 - RNA, 20 nt, synthetic construct
  misc_feature 1..20: note = source = /note="Description of Artificial Sequence: Synthetic oligonucleotide"
  source 1..20: mol_type = other RNA
gtcacctctgatgactaggg

SEQ ID NO: 295 - RNA, 20 nt, synthetic construct
  misc_feature 1..20: note = source = /note="Description of Artificial Sequence: Synthetic oligonucleotide"
  source 1..20: mol_type = other RNA
gtcaccctcaatgactaggg

SEQ ID NO: 296 - RNA, 20 nt, synthetic construct
  misc_feature 1..20: note = source = /note="Description of Artificial Sequence: Synthetic oligonucleotide"
  source 1..20: mol_type = other RNA
gtcatttccaatgactaggg

SEQ ID NO: 297 - RNA, 20 nt, synthetic construct
  misc_feature 1..20: note = source = /note="Description of Artificial Sequence: Synthetic oligonucleotide"
  source 1..20: mol_type = other RNA
gttgcctccaatgactaggg

SEQ ID NO: 298 - RNA, 20 nt, synthetic construct
  misc_feature 1..20: note = source = /note="Description of Artificial Sequence: Synthetic oligonucleotide"
  source 1..20: mol_type = other RNA
accacctccaatgactaggg

SEQ ID NO: 299 - RNA, 20 nt, synthetic construct
  misc_feature 1..20: note = source = /note="Description of Artificial Sequence: Synthetic oligonucleotide"
  source 1..20: mol_type = other RNA
gtcacctccaatgactgaag

SEQ ID NO: 300 - RNA, 20 nt, synthetic construct
  misc_feature 1..20: note = source = /note="Description of Artificial Sequence: Synthetic oligonucleotide"
  source 1..20: mol_type = other RNA
gtcacctccaatggtcaggg

SEQ ID NO: 301 - RNA, 20 nt, synthetic construct
  misc_feature 1..20: note = source = /note="Description of Artificial Sequence: Synthetic oligonucleotide"
  source 1..20: mol_type = other RNA
gtcacctccagcaactaggg

SEQ ID NO: 302 - RNA, 20 nt, synthetic construct
  misc_feature 1..20: note = source = /note="Description of Artificial Sequence: Synthetic oligonucleotide"
  source 1..20: mol_type = other RNA
gtcacctttgatgactaggg

SEQ ID NO: 303 - RNA, 20 nt, synthetic construct
  misc_feature 1..20: note = source = /note="Description of Artificial Sequence: Synthetic oligonucleotide"
  source 1..20: mol_type = other RNA
gtcattcccaatgactaggg

SEQ ID NO: 304 - RNA, 20 nt, synthetic construct
  misc_feature 1..20: note = source = /note="Description of Artificial Sequence: Synthetic oligonucleotide"
  source 1..20: mol_type = other RNA
gctgcctccaatgactaggg

SEQ ID NO: 305 - RNA, 20 nt, synthetic construct
  misc_feature 1..20: note = source = /note="Description of Artificial Sequence: Synthetic oligonucleotide"
  source 1..20: mol_type = other RNA
gtcacctccaatgaccgaaa

SEQ ID NO: 306 - RNA, 20 nt, synthetic construct
  misc_feature 1..20: note = source = /note="Description of Artificial Sequence: Synthetic oligonucleotide"
  source 1..20: mol_type = other RNA
gtcacctccaatagtcgggg

SEQ ID NO: 307 - RNA, 20 nt, synthetic construct
  misc_feature 1..20: note = source = /note="Description of Artificial Sequence: Synthetic oligonucleotide"
  source 1..20: mol_type = other RNA
gtcacctccggcagctaggg

SEQ ID NO: 308 - RNA, 20 nt, synthetic construct
  misc_feature 1..20: note = source = /note="Description of Artificial Sequence: Synthetic oligonucleotide"
  source 1..20: mol_type = other RNA
gtcacccttggtgactaggg

SEQ ID NO: 309 - RNA, 20 nt, synthetic construct
  misc_feature 1..20: note = source = /note="Description of Artificial Sequence: Synthetic oligonucleotide"
  source 1..20: mol_type = other RNA
gtcgttctcaatgactaggg

SEQ ID NO: 310 - RNA, 20 nt, synthetic construct
  misc_feature 1..20: note = source = /note="Description of Artificial Sequence: Synthetic oligonucleotide"
  source 1..20: mol_type = other RNA
actgtctccaatgactaggg

SEQ ID NO: 311 - RNA, 20 nt, synthetic construct
  misc_feature 1..20: note = source = /note="Description of Artificial Sequence: Synthetic oligonucleotide"
  source 1..20: mol_type = other RNA
gcgccaccggttgatgtgat

SEQ ID NO: 312 - RNA, 20 nt, synthetic construct
  misc_feature 1..20: note = source = /note="Description of Artificial Sequence: Synthetic oligonucleotide"
  source 1..20: mol_type = other RNA
gcgccaccggttgatgtggc

SEQ ID NO: 313 - RNA, 20 nt, synthetic construct
  misc_feature 1..20: note = source = /note="Description of Artificial Sequence: Synthetic oligonucleotide"
  source 1..20: mol_type = other RNA
gcgccaccggttgatgcaat

SEQ ID NO: 314 - RNA, 20 nt, synthetic construct
  misc_feature 1..20: note = source = /note="Description of Artificial Sequence: Synthetic oligonucleotide"
  source 1..20: mol_type = other RNA
gcgccaccggttgacatgat

SEQ ID NO: 315 - RNA, 20 nt, synthetic construct
  misc_feature 1..20: note = source = /note="Description of Artificial Sequence: Synthetic oligonucleotide"
  source 1..20: mol_type = other RNA
gcgccaccggttagtgtgat

SEQ ID NO: 316 - RNA, 20 nt, synthetic construct
  misc_feature 1..20: note = source = /note="Description of Artificial Sequence: Synthetic oligonucleotide"
  source 1..20: mol_type = other RNA
gcgccaccggccgatgtgat

SEQ ID NO: 317 - RNA, 20 nt, synthetic construct
  misc_feature 1..20: note = source = /note="Description of Artificial Sequence: Synthetic oligonucleotide"
  source 1..20: mol_type = other RNA
gcgccaccaattgatgtgat

SEQ ID NO: 318 - RNA, 20 nt, synthetic construct
  misc_feature 1..20: note = source = /note="Description of Artificial Sequence: Synthetic oligonucleotide"
  source 1..20: mol_type = other RNA
gcgccattggttgatgtgat

SEQ ID NO: 319 - RNA, 20 nt, synthetic construct
  misc_feature 1..20: note = source = /note="Description of Artificial Sequence: Synthetic oligonucleotide"
  source 1..20: mol_type = other RNA
gcgctgccggttgatgtgat

SEQ ID NO: 320 - RNA, 20 nt, synthetic construct
  misc_feature 1..20: note = source = /note="Description of Artificial Sequence: Synthetic oligonucleotide"
  source 1..20: mol_type = other RNA
gcatcaccggttgatgtgat

SEQ ID NO: 321 - RNA, 20 nt, synthetic construct
  misc_feature 1..20: note = source = /note="Description of Artificial Sequence: Synthetic oligonucleotide"
  source 1..20: mol_type = other RNA
atgccaccggttgatgtgat

SEQ ID NO: 322 - RNA, 20 nt, synthetic construct
  misc_feature 1..20: note = source = /note="Description of Artificial Sequence: Synthetic oligonucleotide"
  source 1..20: mol_type = other RNA
gcgccaccggttgatgcagt

SEQ ID NO: 323 - RNA, 20 nt, synthetic construct
  misc_feature 1..20: note = source = /note="Description of Artificial Sequence: Synthetic oligonucleotide"
  source 1..20: mol_type = other RNA
gcgccaccggttggcatgat

SEQ ID NO: 324 - RNA, 20 nt, synthetic construct
  misc_feature 1..20: note = source = /note="Description of Artificial Sequence: Synthetic oligonucleotide"
  source 1..20: mol_type = other RNA
gcgccaccggccaatgtgat

SEQ ID NO: 325 - RNA, 20 nt, synthetic construct
  misc_feature 1..20: note = source = /note="Description of Artificial Sequence: Synthetic oligonucleotide"
  source 1..20: mol_type = other RNA
gcgccactaattgatgtgat

SEQ ID NO: 326 - RNA, 20 nt, synthetic construct
  misc_feature 1..20: note = source = /note="Description of Artificial Sequence: Synthetic oligonucleotide"
  source 1..20: mol_type = other RNA
gcgctgtcggttgatgtgat

SEQ ID NO: 327 - RNA, 20 nt, synthetic construct
  misc_feature 1..20: note = source = /note="Description of Artificial Sequence: Synthetic oligonucleotide"
  source 1..20: mol_type = other RNA
gtatcaccggttgatgtgat

SEQ ID NO: 328 - RNA, 20 nt, synthetic construct
  misc_feature 1..20: note = source = /note="Description of Artificial Sequence: Synthetic oligonucleotide"
  source 1..20: mol_type = other RNA
gcgccaccggttgatacagc

SEQ ID NO: 329 - RNA, 20 nt, synthetic construct
  misc_feature 1..20: note = source = /note="Description of Artificial Sequence: Synthetic oligonucleotide"
  source 1..20: mol_type = other RNA
gcgccaccggttagcacgat

SEQ ID NO: 330 - RNA, 20 nt, synthetic construct
  misc_feature 1..20: note = source = /note="Description of Artificial Sequence: Synthetic oligonucleotide"
  source 1..20: mol_type = other RNA
gcgccaccgaggagtgtgat

SEQ ID NO: 331 - RNA, 20 nt, synthetic construct
  misc_feature 1..20: note = source = /note="Description of Artificial Sequence: Synthetic oligonucleotide"
  source 1..20: mol_type = other RNA
gcgccattaagtgatgtgat

SEQ ID NO: 332 - RNA, 20 nt, synthetic construct
  misc_feature 1..20: note = source = /note="Description of Artificial Sequence: Synthetic oligonucleotide"
  source 1..20: mol_type = other RNA
gcgttgttggttgatgtgat

SEQ ID NO: 333 - RNA, 20 nt, synthetic construct
  misc_feature 1..20: note = source = /note="Description of Artificial Sequence: Synthetic oligonucleotide"
  source 1..20: mol_type = other RNA
atattaccggttgatgtgat

SEQ ID NO: 334 - RNA, 20 nt, synthetic construct
  misc_feature 1..20: note = source = /note="Description of Artificial Sequence: Synthetic oligonucleotide"
  source 1..20: mol_type = other RNA
gtcacctccaatgactaggg

SEQ ID NO: 335 - RNA, 20 nt, synthetic construct
  misc_feature 1..20: note = source = /note="Description of Artificial Sequence: Synthetic oligonucleotide"
  source 1..20: mol_type = other RNA
gtcacctccaatgactaaga

SEQ ID NO: 336 - RNA, 20 nt, synthetic construct
  misc_feature 1..20: note = source = /note="Description of Artificial Sequence: Synthetic oligonucleotide"
  source 1..20: mol_type = other RNA
gtcacctccaatgattagga

SEQ ID NO: 337 - RNA, 20 nt, synthetic construct
  misc_feature 1..20: note = source = /note="Description of Artificial Sequence: Synthetic oligonucleotide"
  source 1..20: mol_type = other RNA
gtcacctccagtgactagga

SEQ ID NO: 338 - RNA, 20 nt, synthetic construct
  misc_feature 1..20: note = source = /note="Description of Artificial Sequence: Synthetic oligonucleotide"
  source 1..20: mol_type = other RNA
gtcacttccaatgactagga

SEQ ID NO: 339 - RNA, 20 nt, synthetic construct
  misc_feature 1..20: note = source = /note="Description of Artificial Sequence: Synthetic oligonucleotide"
  source 1..20: mol_type = other RNA
atcacctccaatgactagga

SEQ ID NO: 340 - RNA, 20 nt, synthetic construct
  misc_feature 1..20: note = source = /note="Description of Artificial Sequence: Synthetic oligonucleotide"
  source 1..20: mol_type = other RNA
gtcacctccaatgactaggg

SEQ ID NO: 341 - RNA, 20 nt, synthetic construct
  misc_feature 1..20: note = source = /note="Description of Artificial Sequence: Synthetic oligonucleotide"
  source 1..20: mol_type = other RNA
gtcacctccaatgaccaaga

SEQ ID NO: 342 - RNA, 20 nt, synthetic construct
  misc_feature 1..20: note = source = /note="Description of Artificial Sequence: Synthetic oligonucleotide"
  source 1..20: mol_type = other RNA
gtcacctccaatggctggga

SEQ ID NO: 343 - RNA, 20 nt, synthetic construct
  misc_feature 1..20: note = source = /note="Description of Artificial Sequence: Synthetic oligonucleotide"
  source 1..20: mol_type = other RNA
gtcacctccaacgaccagga

SEQ ID NO: 344 - RNA, 20 nt, synthetic construct
  misc_feature 1..20: note = source = /note="Description of Artificial Sequence: Synthetic oligonucleotide"
  source 1..20: mol_type = other RNA
gtcacctccgatgattagga

SEQ ID NO: 345 - RNA, 20 nt, synthetic construct
  misc_feature 1..20: note = source = /note="Description of Artificial Sequence: Synthetic oligonucleotide"
  source 1..20: mol_type = other RNA
gtcacctccaatggccaagg

SEQ ID NO: 346 - RNA, 20 nt, synthetic construct
  misc_feature 1..20: note = source = /note="Description of Artificial Sequence: Synthetic oligonucleotide"
  source 1..20: mol_type = other RNA
gtcacctccaacgattaagg

SEQ ID NO: 347 - RNA, 20 nt, synthetic construct
  misc_feature 1..20: note = source = /note="Description of Artificial Sequence: Synthetic oligonucleotide"
  source 1..20: mol_type = other RNA
gtcacctccgatggctaagg

SEQ ID NO: 348 - RNA, 20 nt, synthetic construct
  misc_feature 1..20: note = source = /note="Description of Artificial Sequence: Synthetic oligonucleotide"
  source 1..20: mol_type = other RNA
gtcaccttcaataactaagg

SEQ ID NO: 349 - RNA, 20 nt, synthetic construct
  misc_feature 1..20: note = source = /note="Description of Artificial Sequence: Synthetic oligonucleotide"
  source 1..20: mol_type = other RNA
gtcacctccaatggccaaga

SEQ ID NO: 350 - RNA, 20 nt, synthetic construct
  misc_feature 1..20: note = source = /note="Description of Artificial Sequence: Synthetic oligonucleotide"
  source 1..20: mol_type = other RNA
gtcacctccagtggctggga

SEQ ID NO: 351 - RNA, 20 nt, synthetic construct
  misc_feature 1..20: note = source = /note="Description of Artificial Sequence: Synthetic oligonucleotide"
  source 1..20: mol_type = other RNA
gtcaccttcaacgaccagga

SEQ ID NO: 352 - RNA, 20 nt, synthetic construct
  misc_feature 1..20: note = source = /note="Description of Artificial Sequence: Synthetic oligonucleotide"
  source 1..20: mol_type = other RNA
gtcatctccgatgattagga

SEQ ID NO: 353 - RNA, 20 nt, synthetic construct
  misc_feature 1..20: note = source = /note="Description of Artificial Sequence: Synthetic oligonucleotide"
  source 1..20: mol_type = other RNA
gccaccttcaatggctagga

SEQ ID NO: 354 - RNA, 20 nt, synthetic construct
  misc_feature 1..20: note = source = /note="Description of Artificial Sequence: Synthetic oligonucleotide"
  source 1..20: mol_type = other RNA
gcgccaccggttgatgtgat

SEQ ID NO: 355 - RNA, 20 nt, synthetic construct
  misc_feature 1..20: note = source = /note="Description of Artificial Sequence: Synthetic oligonucleotide"
  source 1..20: mol_type = other RNA
gcgccaccggttgatgtaac

SEQ ID NO: 356 - RNA, 20 nt, synthetic construct
  misc_feature 1..20: note = source = /note="Description of Artificial Sequence: Synthetic oligonucleotide"
  source 1..20: mol_type = other RNA
gcgccaccggttgacgtgac

SEQ ID NO: 357 - RNA, 20 nt, synthetic construct
  misc_feature 1..20: note = source = /note="Description of Artificial Sequence: Synthetic oligonucleotide"
  source 1..20: mol_type = other RNA
gcgccaccggctgatgtgac

SEQ ID NO: 358 - RNA, 20 nt, synthetic construct
  misc_feature 1..20: note = source = /note="Description of Artificial Sequence: Synthetic oligonucleotide"
  source 1..20: mol_type = other RNA
gcgccgccggttgatgtgac

SEQ ID NO: 359 - RNA, 20 nt, synthetic construct
  misc_feature 1..20: note = source = /note="Description of Artificial Sequence: Synthetic oligonucleotide"
  source 1..20: mol_type = other RNA
acgccaccggttgatgtgac

SEQ ID NO: 360 - RNA, 20 nt, synthetic construct
  misc_feature 1..20: note = source = /note="Description of Artificial Sequence: Synthetic oligonucleotide"
  source 1..20: mol_type = other RNA
gcgccaccggttgatgtgat

SEQ ID NO: 361 - RNA, 20 nt, synthetic construct
  misc_feature 1..20: note = source = /note="Description of Artificial Sequence: Synthetic oligonucleotide"
  source 1..20: mol_type = other RNA
gcgccaccggttgatataac

SEQ ID NO: 362 - RNA, 20 nt, synthetic construct
  misc_feature 1..20: note = source = /note="Description of Artificial Sequence: Synthetic oligonucleotide"
  source 1..20: mol_type = other RNA
gcgccaccggttggtgcgac

SEQ ID NO: 363 - RNA, 20 nt, synthetic construct
  misc_feature 1..20: note = source = /note="Description of Artificial Sequence: Synthetic oligonucleotide"
  source 1..20: mol_type = other RNA
gcgccaccggtcgatatgac

SEQ ID NO: 364 - RNA, 20 nt, synthetic construct
  misc_feature 1..20: note = source = /note="Description of Artificial Sequence: Synthetic oligonucleotide"
  source 1..20: mol_type = other RNA
gcgccaccgattgacgtgac

SEQ ID NO: 365 - RNA, 20 nt, synthetic construct
  misc_feature 1..20: note = source = /note="Description of Artificial Sequence: Synthetic oligonucleotide"
  source 1..20: mol_type = other RNA
gcgccaccggttggtataat

SEQ ID NO: 366 - RNA, 20 nt, synthetic construct
  misc_feature 1..20: note = source = /note="Description of Artificial Sequence: Synthetic oligonucleotide"
  source 1..20: mol_type = other RNA
gcgccaccggtcgacgtaat

SEQ ID NO: 367 - RNA, 20 nt, synthetic construct
  misc_feature 1..20: note = source = /note="Description of Artificial Sequence: Synthetic oligonucleotide"
  source 1..20: mol_type = other RNA
gcgccaccgattggtgtaat

SEQ ID NO: 368 - RNA, 20 nt, synthetic construct
  misc_feature 1..20: note = source = /note="Description of Artificial Sequence: Synthetic oligonucleotide"
  source 1..20: mol_type = other RNA
gcgccactggttaatgtaat

SEQ ID NO: 369 - RNA, 20 nt, synthetic construct
  misc_feature 1..20: note = source = /note="Description of Artificial Sequence: Synthetic oligonucleotide"
  source 1..20: mol_type = other RNA
gcgccaccggttggtataac

SEQ ID NO: 370 - RNA, 20 nt, synthetic construct
  misc_feature 1..20: note = source = /note="Description of Artificial Sequence: Synthetic oligonucleotide"
  source 1..20: mol_type = other RNA
gcgccaccggctggtgcgac

SEQ ID NO: 371 - RNA, 20 nt, synthetic construct
  misc_feature 1..20: note = source = /note="Description of Artificial Sequence: Synthetic oligonucleotide"
  source 1..20: mol_type = other RNA
gcgccactggtcgatatgac

SEQ ID NO: 372 - RNA, 20 nt, synthetic construct
  misc_feature 1..20: note = source = /note="Description of Artificial Sequence: Synthetic oligonucleotide"
  source 1..20: mol_type = other RNA
gcgctaccgattgacgtgac

SEQ ID NO: 373 - RNA, 20 nt, synthetic construct
  misc_feature 1..20: note = source = /note="Description of Artificial Sequence: Synthetic oligonucleotide"
  source 1..20: mol_type = other RNA
gtgccactggttggtgtgac

SEQ ID NO: 374 - RNA, 23 nt, synthetic construct
  misc_feature 1..23: note = source = /note="Description of Artificial Sequence: Synthetic oligonucleotide"
  source 1..23: mol_type = other RNA
gagtccgagcagaagaagaaggg

SEQ ID NO: 375 - DNA, 23 bp, synthetic construct
  misc_feature 1..23: note = source = /note="Description of Artificial Sequence: Synthetic oligonucleotide"
  misc_feature 1..23: note = source = /note="Description of Combined DNA/RNA Molecule: Synthetic oligonucleotide"
  source 1..23: mol_type = other DNA
  modified_base 3..4: mod_base = OTHER; note = uracil
  modified_base 7: mod_base = OTHER; note = uracil
gattcctaccagaagaagaatgg

SEQ ID NO: 376 - RNA, 23 nt, synthetic construct
  misc_feature 1..23: note = source = /note="Description of Artificial Sequence: Synthetic oligonucleotide"
  source 1..23: mol_type = other RNA
aagtccgaggagaggaagaaagg

SEQ ID NO: 377 - RNA, 23 nt, synthetic construct
  misc_feature 1..23: note = source = /note="Description of Artificial Sequence: Synthetic oligonucleotide"
  source 1..23: mol_type = other RNA
aagtccgagaagaagcagaaaag

SEQ ID NO: 378 - RNA, 23 nt, synthetic construct
  misc_feature 1..23: note = source = /note="Description of Artificial Sequence: Synthetic oligonucleotide"
  source 1..23: mol_type = other RNA
gagttccagaagaagaagaagag

SEQ ID NO: 379 - RNA, 23 nt, synthetic construct
  misc_feature 1..23: note = source = /note="Description of Artificial Sequence: Synthetic oligonucleotide"
  source 1..23: mol_type = other RNA
gagtctgaacggaagaagaaaag

SEQ ID NO: 380 - RNA, 23 nt, synthetic construct
  misc_feature 1..23: note = source = /note="Description of Artificial Sequence: Synthetic oligonucleotide"
  source 1..23: mol_type = other RNA
gagtttgagtagaagaagaagag

SEQ ID NO: 381 - RNA, 23 nt, synthetic construct
  misc_feature 1..23: note = source = /note="Description of Artificial Sequence: Synthetic oligonucleotide"
  source 1..23: mol_type = other RNA
gagtcccagaagaagaaaaaaag

SEQ ID NO: 382 - DNA, 23 bp, synthetic construct
  misc_feature 1..23: note = source = /note="Description of Artificial Sequence: Synthetic oligonucleotide"
  misc_feature 1..23: note = source = /note="Description of Combined DNA/RNA Molecule: Synthetic oligonucleotide"
  source 1..23: mol_type = other DNA
  modified_base 4: mod_base = OTHER; note = uracil
gactccgagcagcagaaggatgg

SEQ ID NO: 383 - RNA, 23 nt, synthetic construct
  misc_feature 1..23: note = source = /note="Description of Artificial Sequence: Synthetic oligonucleotide"
  source 1..23: mol_type = other RNA
gagtcagagcagaactagaaggg

SEQ ID NO: 384 - RNA, 23 nt, synthetic construct
  misc_feature 1..23: note = source = /note="Description of Artificial Sequence: Synthetic oligonucleotide"
  source 1..23: mol_type = other RNA
gaggccgagcagaagaaagacgg

SEQ ID NO: 385 - RNA, 23 nt, synthetic construct
  misc_feature 1..23: note = source = /note="Description of Artificial Sequence: Synthetic oligonucleotide"
  source 1..23: mol_type = other RNA
gagtcagaccaggagaagaagag

SEQ ID NO: 386 - DNA, 23 bp, synthetic construct
  misc_feature 1..23: note = source = /note="Description of Artificial Sequence: Synthetic oligonucleotide"
  misc_feature 1..23: note = source = /note="Description of Combined DNA/RNA Molecule: Synthetic oligonucleotide"
  source 1..23: mol_type = other DNA
  modified_base 4: mod_base = OTHER; note = uracil
  modified_base 15: mod_base = OTHER; note = uracil
gagtccaagaagaataagaatag

SEQ ID NO: 387 - RNA, 23 nt, synthetic construct
  misc_feature 1..23: note = source = /note="Description of Artificial Sequence: Synthetic oligonucleotide"
  source 1..23: mol_type = other RNA
gagtaagagaagaagaagaaggg

SEQ ID NO: 388 - RNA, 23 nt, synthetic construct
  misc_feature 1..23: note = source = /note="Description of Artificial Sequence: Synthetic oligonucleotide"
  source 1..23: mol_type = other RNA
gagtaggaggagaagaagaaagg

SEQ ID NO: 389 - DNA, 23 bp, synthetic construct
  misc_feature 1..23: note = source = /note="Description of Artificial Sequence: Synthetic oligonucleotide"
  misc_feature 1..23: note = source = /note="Description of Combined DNA/RNA Molecule: Synthetic oligonucleotide"
  source 1..23: mol_type = other DNA
  modified_base 4: mod_base = OTHER; note = uracil
  modified_base 6: mod_base = OTHER; note = uracil
aagtctgagcacaagaagaatgg

SEQ ID NO: 390 - RNA, 23 nt, synthetic construct
  misc_feature 1..23: note = source = /note="Description of Artificial Sequence: Synthetic oligonucleotide"
  source 1..23: mol_type = other RNA
gagcccgagcagaaggaggaggg

SEQ ID NO: 391 - RNA, 23 nt, synthetic construct
  misc_feature 1..23: note = source = /note="Description of Artificial Sequence: Synthetic oligonucleotide"
  source 1..23: mol_type = other RNA
gagttagagcagaagaagaaagg

SEQ ID NO: 392 - RNA, 23 nt, synthetic construct
  misc_feature 1..23: note = source = /note="Description of Artificial Sequence: Synthetic oligonucleotide"
  source 1..23: mol_type = other RNA
gagtcagaacagaagaacaacag

SEQ ID NO: 393 - DNA, 23 bp, synthetic construct
  misc_feature 1..23: note = source = /note="Description of Artificial Sequence: Synthetic oligonucleotide"
  misc_feature 1..23: note = source = /note="Description of Combined DNA/RNA Molecule: Synthetic oligonucleotide"
  source 1..23: mol_type = other DNA
  modified_base 4: mod_base = OTHER; note = uracil
  modified_base 6: mod_base = OTHER; note = uracil
acgtctgagcagaagaagaatgg

SEQ ID NO: 394 - RNA, 23 nt, synthetic construct
  misc_feature 1..23: note = source = /note="Description of Artificial Sequence: Synthetic oligonucleotide"
  source 1..23: mol_type = other RNA
gagtactagaagaagaagaaaag

SEQ ID NO: 395 - RNA, 23 nt, synthetic construct
  misc_feature 1..23: note = source = /note="Description of Artificial Sequence: Synthetic oligonucleotide"
  source 1..23: mol_type = other RNA
aagtctgagcagaagaagcacag

SEQ ID NO: 396 - RNA, 23 nt, synthetic construct
  misc_feature 1..23: note = source = /note="Description of Artificial Sequence: Synthetic oligonucleotide"
  source 1..23: mol_type = other RNA
gagtcccagcagaggaagcagag

SEQ ID NO: 397 - RNA, 23 nt, synthetic construct
  misc_feature 1..23: note = source = /note="Description of Artificial Sequence: Synthetic oligonucleotide"
  source 1..23: mol_type = other RNA
gagtctgggcaggagaagaagag

SEQ ID NO: 398 - RNA, 23 nt, synthetic construct
  misc_feature 1..23: note = source = /note="Description of Artificial Sequence: Synthetic oligonucleotide"
  source 1..23: mol_type = other RNA
gagtcctagcaggagaagaagag

SEQ ID NO: 399 - RNA, 23 nt, synthetic construct
  misc_feature 1..23: note = source = /note="Description of Artificial Sequence: Synthetic oligonucleotide"
  source 1..23: mol_type = other RNA
gaggaggagcagaagaagaaaag

SEQ ID NO: 400 - RNA, 23 nt, synthetic construct
  misc_feature 1..23: note = source = /note="Description of Artificial Sequence: Synthetic oligonucleotide"
  source 1..23: mol_type = other RNA
gagtccgagaaaatgaagaagag

SEQ ID NO: 401 - RNA, 23 nt, synthetic construct
  misc_feature 1..23: note = source = /note="Description of Artificial Sequence: Synthetic oligonucleotide"
  source 1..23: mol_type = other RNA
gaggcccagcagaggaagaagag

SEQ ID NO: 402 - RNA, 23 nt, synthetic construct
  misc_feature 1..23: note = source = /note="Description of Artificial Sequence: Synthetic oligonucleotide"
  source 1..23: mol_type = other RNA
gaatccaagcagaagaagagaag

SEQ ID NO: 403 - DNA, 23 bp, synthetic construct
  misc_feature 1..23: note = source = /note="Description of Artificial Sequence: Synthetic oligonucleotide"
  misc_feature 1..23: note = source = /note="Description of Combined DNA/RNA Molecule: Synthetic oligonucleotide"
  source 1..23: mol_type = other DNA
  modified_base 4: mod_base = OTHER; note = uracil
  modified_base 7: mod_base = OTHER; note = uracil
gactcctagcaaaagaagaatgg

SEQ ID NO: 404 - RNA, 23 nt, synthetic construct
  misc_feature 1..23: note = source = /note="Description of Artificial Sequence: Synthetic oligonucleotide"
  source 1..23: mol_type = other RNA
gagtcccagcaaaagaagaaaag

SEQ ID NO: 405 - RNA, 23 nt, synthetic construct
  misc_feature 1..23: note = source = /note="Description of Artificial Sequence: Synthetic oligonucleotide"
  source 1..23: mol_type = other RNA
gagtctaagcagaagaagaagag

SEQ ID NO: 406 - RNA, 23 nt, synthetic construct
  misc_feature 1..23: note = source = /note="Description of Artificial Sequence: Synthetic oligonucleotide"
  source 1..23: mol_type = other RNA
aagtcagaggagaagaagaaggg

SEQ ID NO: 407 - DNA, 23 bp, synthetic construct
  misc_feature 1..23: note = source = /note="Description of Artificial Sequence: Synthetic oligonucleotide"
  misc_feature 1..23: note = source = /note="Description of Combined DNA/RNA Molecule: Synthetic oligonucleotide"
  source 1..23: mol_type = other DNA
  modified_base 4: mod_base = OTHER; note = uracil
gagtccaagcagaagaaggatag

SEQ ID NO: 408 - RNA, 23 nt, synthetic construct
  misc_feature 1..23: note = source = /note="Description of Artificial Sequence: Synthetic oligonucleotide"
  source 1..23: mol_type = other RNA
gagactgagaagaagaagaaagg

SEQ ID NO: 409 - RNA, 23 nt, synthetic construct
  misc_feature 1..23: note = source = /note="Description of Artificial Sequence: Synthetic oligonucleotide"
  source 1..23: mol_type = other RNA
gagtcccaggagaagaagagagg

SEQ ID NO: 410 - RNA, 23 nt, synthetic construct
  misc_feature 1..23: note = source = /note="Description of Artificial Sequence: Synthetic oligonucleotide"
  source 1..23: mol_type = other RNA
gagtcccaggagaagaaaaacag

SEQ ID NO: 411 - RNA, 23 nt, synthetic construct
  misc_feature 1..23: note = source = /note="Description of Artificial Sequence: Synthetic oligonucleotide"
  source 1..23: mol_type = other RNA
gagagcaagcagaagaagaaaag

SEQ ID NO: 412 - RNA, 23 nt, synthetic construct
  misc_feature 1..23: note = source = /note="Description of Artificial Sequence: Synthetic oligonucleotide"
  source 1..23: mol_type = other RNA
gagtccaagcataagaaaaacag

SEQ ID NO: 413 - RNA, 23 nt, synthetic construct
  misc_feature 1..23: note = source = /note="Description of Artificial Sequence: Synthetic oligonucleotide"
  source 1..23: mol_type = other RNA
gagtccaagcagtagaggaaggg

SEQ ID NO: 414 - RNA, 23 nt, synthetic construct
  misc_feature 1..23: note = source = /note="Description of Artificial Sequence: Synthetic oligonucleotide"
  source 1..23: mol_type = other RNA
gagtccgggaaggagaagaaagg

SEQ ID NO: 415 - RNA, 20 nt, synthetic construct
  misc_feature 1..20: note = source = /note="Description of Artificial Sequence: Synthetic oligonucleotide"
  source 1..20: mol_type = other RNA
gcgccaccggttgatgtgat

SEQ ID NO: 416 - RNA, 23 nt, synthetic construct
  misc_feature 1..23: note = source = /note="Description of Artificial Sequence: Synthetic oligonucleotide"
  source 1..23: mol_type = other RNA
gggccatgggttgatgtgatgag

SEQ ID NO: 417 - DNA, 23 bp, synthetic construct
  misc_feature 1..23: note = source = /note="Description of Artificial Sequence: Synthetic oligonucleotide"
  misc_feature 1..23: note = source = /note="Description of Combined DNA/RNA Molecule: Synthetic oligonucleotide"
  source 1..23: mol_type = other DNA
gtcacctccaatgactagggtgg

SEQ ID NO: 418 - DNA, 23 bp, synthetic construct
  misc_feature 1..23: note = source = /note="Description of Artificial Sequence: Synthetic oligonucleotide"
  misc_feature 1..23: note = source = /note="Description of Combined DNA/RNA Molecule: Synthetic oligonucleotide"
  source 1..23: mol_type = other DNA
  modified_base 3: mod_base = OTHER; note = uracil
gctacctccagtgactagggagg

SEQ ID NO: 419 - DNA, 23 bp, synthetic construct
  misc_feature 1..23: note = source = /note="Description of Artificial Sequence: Synthetic oligonucleotide"
  misc_feature 1..23: note = source = /note="Description of Combined DNA/RNA Molecule: Synthetic oligonucleotide"
  source 1..23: mol_type = other DNA
gtgacctccaatgcctagagggg

SEQ ID NO: 420 - DNA, 23 bp, synthetic construct
  misc_feature 1..23: note = source = /note="Description of Artificial Sequence: Synthetic oligonucleotide"
  misc_feature 1..23: note = source = /note="Description of Combined DNA/RNA Molecule: Synthetic oligonucleotide"
  source 1..23: mol_type = other DNA
  modified_base 13: mod_base = OTHER; note = uracil
gtcacctccacttcctagggcag

SEQ ID NO: 421 - DNA, 23 bp, synthetic construct
  misc_feature 1..23: note = source = /note="Description of Artificial Sequence: Synthetic oligonucleotide"
  misc_feature 1..23: note = source = /note="Description of Combined DNA/RNA Molecule: Synthetic oligonucleotide"
  source 1..23: mol_type = other DNA
  modified_base 1: mod_base = OTHER; note = uracil
ttcacctccaaaaactagggaag

SEQ ID NO: 422 - DNA, 23 bp, synthetic construct
  misc_feature 1..23: note = source = /note="Description of Artificial Sequence: Synthetic oligonucleotide"
  misc_feature 1..23: note = source = /note="Description of Combined DNA/RNA Molecule: Synthetic oligonucleotide"
  source 1..23: mol_type = other DNA
  modified_base 17: mod_base = OTHER; note = uracil
gtcaactccaatggcttgggagg

SEQ ID NO: 423 - DNA, 23 bp, synthetic construct
  misc_feature 1..23: note = source = /note="Description of Artificial Sequence: Synthetic oligonucleotide"
  misc_feature 1..23: note = source = /note="Description of Combined DNA/RNA Molecule: Synthetic oligonucleotide"
  source 1..23: mol_type = other DNA
  modified_base 8: mod_base = OTHER; note = uracil
  modified_base 17: mod_base = OTHER; note = uracil
gtcaccttaaatgacttgggaag

SEQ ID NO: 424 - DNA, 23 bp, synthetic construct
  misc_feature 1..23: note = source = /note="Description of Artificial Sequence: Synthetic oligonucleotide"
  misc_feature 1..23: note = source = /note="Description of Combined DNA/RNA Molecule: Synthetic oligonucleotide"
  source 1..23: mol_type = other DNA
  modified_base 6: mod_base = OTHER; note = uracil
gtcacttccaaggactagagaag

SEQ ID NO: 425 - DNA, 23 bp, synthetic construct
  misc_feature 1..23: note = source = /note="Description of Artificial Sequence: Synthetic oligonucleotide"
  misc_feature 1..23: note = source = /note="Description of Combined DNA/RNA Molecule: Synthetic oligonucleotide"
  source 1..23: mol_type = other DNA
  modified_base 14: mod_base = OTHER; note = uracil
gtcacctccagggtctagggcag

SEQ ID NO: 426 - DNA, 23 bp, synthetic construct
  misc_feature 1..23: note = source = /note="Description of Artificial Sequence: Synthetic oligonucleotide"
  misc_feature 1..23: note = source = /note="Description of Combined DNA/RNA Molecule: Synthetic oligonucleotide"
  source 1..23: mol_type = other DNA
  modified_base 14: mod_base = OTHER; note = uracil
gtcacctccactgtatagggagg

SEQ ID NO: 427 - DNA, 23 bp, synthetic construct
  misc_feature 1..23: note = source = /note="Description of Artificial Sequence: Synthetic oligonucleotide"
  misc_feature 1..23: note = source = /note="Description of Combined DNA/RNA Molecule: Synthetic oligonucleotide"
  source 1..23: mol_type = other DNA
  modified_base 15: mod_base = OTHER; note = uracil
gtcaactccaatgattaggacag

SEQ ID NO: 428 - DNA, 23 bp, synthetic construct
  misc_feature 1..23: note = source = /note="Description of Artificial Sequence: Synthetic oligonucleotide"
  source 1..23: mol_type = other DNA
gtggtgtcacgctcgtcgtttgg

SEQ ID NO: 429 - DNA, 23 bp, synthetic construct
  misc_feature 1..23: note = source = /note="Description of Artificial Sequence: Synthetic oligonucleotide"
  source 1..23: mol_type = other DNA
tccagtctattaattgttgccgg

SEQ ID NO: 430 - DNA, 12 bp, Homo sapiens
  source 1..12: mol_type = unassigned DNA
tagcgggtaagc

SEQ ID NO: 431 - DNA, 12 bp, Homo sapiens
  source 1..12: mol_type = unassigned DNA
tcggtcacatgt

SEQ ID NO: 432 - DNA, 12 bp, Homo sapiens
  source 1..12: mol_type = unassigned DNA
actccccgtagg

SEQ ID NO: 433 - DNA, 12 bp, Homo sapiens
  source 1..12: mol_type = unassigned DNA
actgcgtgttaa

SEQ ID NO: 434 - DNA, 12 bp, Homo sapiens
  source 1..12: mol_type = unassigned DNA
acgtcgcctgat

SEQ ID NO: 435 - DNA, 12 bp, Homo sapiens
  source 1..12: mol_type = unassigned DNA
taggtcgaccag

SEQ ID NO: 436 - DNA, 12 bp, Homo sapiens
  source 1..12: mol_type = unassigned DNA
ggcgttaatgat

SEQ ID NO: 437 - DNA, 12 bp, Homo sapiens
  source 1..12: mol_type = unassigned DNA
tgtcgcatgtta

SEQ ID NO: 438 - DNA, 12 bp, Homo sapiens
  source 1..12: mol_type = unassigned DNA
atggaaacgcat

SEQ ID NO: 439 - DNA, 12 bp, Homo sapiens
  source 1..12: mol_type = unassigned DNA
gccgaattcctc

SEQ ID NO: 440 - DNA, 12 bp, Homo sapiens
  source 1..12: mol_type = unassigned DNA
gcatggtacgga

SEQ ID NO: 441 - DNA, 12 bp, Homo sapiens
  source 1..12: mol_type = unassigned DNA
cggtactcttac

SEQ ID NO: 442 - DNA, 12 bp, Homo sapiens
  source 1..12: mol_type = unassigned DNA
gcctgtgccgta

SEQ ID NO: 443 - DNA, 12 bp, Homo sapiens
  source 1..12: mol_type = unassigned DNA
tacggtaagtcg

SEQ ID NO: 444 - DNA, 12 bp, Homo sapiens
  source 1..12: mol_type = unassigned DNA
cacgaaattacc

SEQ ID NO: 445 - DNA, 12 bp, Homo sapiens
  source 1..12: mol_type = unassigned DNA
aaccaagatacg

SEQ ID NO: 446 - DNA, 12 bp, Homo sapiens
  source 1..12: mol_type = unassigned DNA
gagtcgatacgc

SEQ ID NO: 447 - DNA, 12 bp, Homo sapiens
  source 1..12: mol_type = unassigned DNA
gtctcacgatcg

SEQ ID NO: 448 - DNA, 12 bp, Homo sapiens
  source 1..12: mol_type = unassigned DNA
tcgtcgggtgca

SEQ ID NO: 449 - DNA, 12 bp, Homo sapiens
  source 1..12: mol_type = unassigned DNA
actccgtagtga

SEQ ID NO: 450 - DNA, 12 bp, Homo sapiens
  source 1..12: mol_type = unassigned DNA
caggacgtccgt

SEQ ID NO: 451 - DNA, 12 bp, Homo sapiens
  source 1..12: mol_type = unassigned DNA
tcgtatccctac

SEQ ID NO: 452 - DNA, 12 bp, Homo sapiens
  source 1..12: mol_type = unassigned DNA
tttcaaggccgg

SEQ ID NO: 453 - DNA, 12 bp, Homo sapiens
  source 1..12: mol_type = unassigned DNA
cgccggtggaat

SEQ ID NO: 454 - DNA, 12 bp, Homo sapiens
  source 1..12: mol_type = unassigned DNA
gaacccgtccta

SEQ ID NO: 455 - DNA, 12 bp, Homo sapiens
  source 1..12: mol_type = unassigned DNA
gattcatcagcg

SEQ ID NO: 456 - DNA, 12 bp, Homo sapiens
  source 1..12: mol_type = unassigned DNA
acaccggtcttc

SEQ ID NO: 457 - DNA, 12 bp, Homo sapiens
  source 1..12: mol_type = unassigned DNA
atcgtgccctaa

SEQ ID NO: 458 - DNA, 12 bp, Homo sapiens
  source 1..12: mol_type = unassigned DNA
gcgtcaatgttc

SEQ ID NO: 459 - DNA, 12 bp, Homo sapiens
  source 1..12: mol_type = unassigned DNA
ctccgtatctcg

SEQ ID NO: 460 - DNA, 12 bp, Homo sapiens
  source 1..12: mol_type = unassigned DNA
ccgattccttcg

SEQ ID NO: 461 - DNA, 12 bp, Homo sapiens
  source 1..12: mol_type = unassigned DNA
tgcgcctccagt

SEQ ID NO: 462 - DNA, 12 bp, Homo sapiens
  source 1..12: mol_type = unassigned DNA
taacgtcggagc

SEQ ID NO: 463 - DNA, 12 bp, Homo sapiens
  source 1..12: mol_type = unassigned DNA
aaggtcgcccat

SEQ ID NO: 464 - DNA, 12 bp, Homo sapiens
  source 1..12: mol_type = unassigned DNA
ctcggggactat

SEQ ID NO: 465 - DNA, 12 bp, Homo sapiens
  source 1..12: mol_type = unassigned DNA
ttcgagcgattt

SEQ ID NO: 466 - DNA, 12 bp, Homo sapiens
  source 1..12: mol_type = unassigned DNA
tgagtcgtcgag

SEQ ID NO: 467 - DNA, 12 bp, Homo sapiens
  source 1..12: mol_type = unassigned DNA
tttacgcagagg

SEQ ID NO: 468 - DNA, 12 bp, Homo sapiens
  source 1..12: mol_type = unassigned DNA
aggaagtatcgc

SEQ ID NO: 469 - DNA, 12 bp, Homo sapiens
  source 1..12: mol_type = unassigned DNA
actcgataccat

SEQ ID NO: 470 - DNA, 12 bp, Homo sapiens
  source 1..12: mol_type = unassigned DNA
cgctacatagca

SEQ ID NO: 471 - DNA, 12 bp, Homo sapiens
  source 1..12: mol_type = unassigned DNA
ttcataaccggc

SEQ ID NO: 472 - DNA, 12 bp, Homo sapiens
  source 1..12: mol_type = unassigned DNA
ccaaacggttaa

SEQ ID NO: 473 - DNA, 12 bp, Homo sapiens
  source 1..12: mol_type = unassigned DNA
cgattccttcgt

SEQ ID NO: 474 - DNA, 12 bp, Homo sapiens
  source 1..12: mol_type = unassigned DNA
cgtcatgaataa

SEQ ID NO: 475 - DNA, 12 bp, Homo sapiens
  source 1..12: mol_type = unassigned DNA
agtggcgatgac

SEQ ID NO: 476 - DNA, 12 bp, Homo sapiens
  source 1..12: mol_type = unassigned DNA
cccctacggcac

SEQ ID NO: 477 - DNA, 12 bp, Homo sapiens
  source 1..12: mol_type = unassigned DNA
gccaacccgcac

SEQ ID NO: 478 - DNA, 12 bp, Homo sapiens
  source 1..12: mol_type = unassigned DNA
tgggacaccggt

SEQ ID NO: 479 - DNA, 12 bp, Homo sapiens
  source 1..12: mol_type = unassigned DNA
ttgactgcggcg

SEQ ID NO: 480 - DNA, 12 bp, Homo sapiens
  source 1..12: mol_type = unassigned DNA
actatgcgtagg

SEQ ID NO: 481 - DNA, 12 bp, Homo sapiens
  source 1..12: mol_type = unassigned DNA
tcacccaaagcg

SEQ ID NO: 482 - DNA, 12 bp, Homo sapiens
  source 1..12: mol_type = unassigned DNA
gcaggacgtccg

SEQ ID NO: 483 - DNA, 12 bp, Homo sapiens
  source 1..12: mol_type = unassigned DNA
acaccgaaaacg

SEQ ID NO: 484 - DNA, 12 bp, Homo sapiens
  source 1..12: mol_type = unassigned DNA
cggtgtattgag

SEQ ID NO: 485 - DNA, 12 bp, Homo sapiens
  source 1..12: mol_type = unassigned DNA
cacgaggtatgc

SEQ ID NO: 486 - DNA, 12 bp, Homo sapiens
  source 1..12: mol_type = unassigned DNA
taaagcgacccg

SEQ ID NO: 487 - DNA, 12 bp, Homo sapiens
  source 1..12: mol_type = unassigned DNA
cttagtcggcca

SEQ ID NO: 488 - DNA, 12 bp, Homo sapiens
  source 1..12: mol_type = unassigned DNA
cgaaaacgtggc

SEQ ID NO: 489 - DNA, 12 bp, Homo sapiens
  source 1..12: mol_type = unassigned DNA
cgtgccctgaac

SEQ ID NO: 490 - DNA, 12 bp, Homo sapiens
  source 1..12: mol_type = unassigned DNA
tttaccatcgaa

SEQ ID NO: 491 - DNA, 12 bp, Homo sapiens
  source 1..12: mol_type = unassigned DNA
cgtagccatgtt

SEQ ID NO: 492 - DNA, 12 bp, Homo sapiens
  source 1..12: mol_type = unassigned DNA
cccaaacggtta

SEQ ID NO: 493 - DNA, 12 bp, Homo sapiens
  source 1..12: mol_type = unassigned DNA
gcgttatcagaa

SEQ ID NO: 494 - DNA, 12 bp, Homo sapiens
  source 1..12: mol_type = unassigned DNA
tcgatggtaaac

SEQ ID NO: 495 - DNA, 12 bp, Homo sapiens
  source 1..12: mol_type = unassigned DNA
cgactttttgca

SEQ ID NO: 496 - DNA, 12 bp, Homo sapiens
  source 1..12: mol_type = unassigned DNA
tcgacgactcac

SEQ ID NO: 497 - DNA, 12 bp, Homo sapiens
  source 1..12: mol_type = unassigned DNA
acgcgtcagata

SEQ ID NO: 498 - DNA, 12 bp, Homo sapiens
  source 1..12: mol_type = unassigned DNA
cgtacggcacag

SEQ ID NO: 499 - DNA, 12 bp, Homo sapiens
  source 1..12: mol_type = unassigned DNA
ctatgccgtgca

SEQ ID NO: 500 - DNA, 12 bp, Homo sapiens
  source 1..12: mol_type = unassigned DNA
cgcgtcagatat

SEQ ID NO: 501 - DNA, 12 bp, Homo sapiens
  source 1..12: mol_type = unassigned DNA
aagatcggtagc

SEQ ID NO: 502 - DNA, 12 bp, Homo sapiens
  source 1..12: mol_type = unassigned DNA
cttcgcaaggag

SEQ ID NO: 503 - DNA, 12 bp, Homo sapiens
  source 1..12: mol_type = unassigned DNA
gtcgtggactac

SEQ ID NO: 504 - DNA, 12 bp, Homo sapiens
  source 1..12: mol_type = unassigned DNA
ggtcgtcatcaa

SEQ ID NO: 505 - DNA, 12 bp, Homo sapiens
  source 1..12: mol_type = unassigned DNA
gttaacagcgtg

SEQ ID NO: 506 - DNA, 12 bp, Homo sapiens
  source 1..12: mol_type = unassigned DNA
tagctaaccgtt

SEQ ID NO: 507 - DNA, 12 bp, Homo sapiens
  source 1..12: mol_type = unassigned DNA
agtaaaggcgct

SEQ ID NO: 508 - DNA, 12 bp, Homo sapiens
  source 1..12: mol_type = unassigned DNA
ggtaatttcgtg

SEQ ID NO: 509 - DNA, 20 bp, Mus musculus
  source 1..20: mol_type = unassigned DNA
gactgattcagctagaccgg

SEQ ID NO: 510 - DNA, 20 bp, Mus musculus
  source 1..20: mol_type = unassigned DNA
ggcacaaacgcgttcaatac

SEQ ID NO: 511 - DNA, 20 bp, Mus musculus
  source 1..20: mol_type = unassigned DNA
aacgcgttcaataccggtct

SEQ ID NO: 512 - DNA, 20 bp, Rattus norvegicus
  source 1..20: mol_type = unassigned DNA
gctaggaggatctcgggcgg

SEQ ID NO: 513 - DNA, 20 bp, Rattus norvegicus
  source 1..20: mol_type = unassigned DNA
gttccagcccgcgactaagc

SEQ ID NO: 514 - DNA, 20 bp, Rattus norvegicus
  source 1..20: mol_type = unassigned DNA
gtgagggggttgcaacgagg

SEQ ID NO: 515 - DNA, 20 bp, Rattus norvegicus
  source 1..20: mol_type = unassigned DNA
accgcaactcttggcgcgtc

SEQ ID NO: 516 - DNA, 20 bp, Rattus norvegicus
  source 1..20: mol_type = unassigned DNA
accagatgcggttgcagtcg

SEQ ID NO: 517 - DNA, 20 bp, Rattus norvegicus
  source 1..20: mol_type = unassigned DNA
tacttcggcgcgtattttta

SEQ ID NO: 518 - DNA, 20 bp, Rattus norvegicus
  source 1..20: mol_type = unassigned DNA
aaatgtgagattccggacta

SEQ ID NO: 519 - DNA, 20 bp, Rattus norvegicus
  source 1..20: mol_type = unassigned DNA
tgtgaccgcgcttgcgaact

SEQ ID NO: 520 - DNA, 20 bp, Rattus norvegicus
  source 1..20: mol_type = unassigned DNA
tctcgggcaccgcgagccgg

SEQ ID NO: 521 - DNA, 20 bp, Rattus norvegicus
  source 1..20: mol_type = unassigned DNA
cgctcctggctggtccgcaa

SEQ ID NO: 522 - DNA, 20 bp, Rattus norvegicus
  source 1..20: mol_type = unassigned DNA
tgagggtagttgagcgccgt

SEQ ID NO: 523 - DNA, 20 bp, Rattus norvegicus
  source 1..20: mol_type = unassigned DNA
tgagattgggaccgccacgc

SEQ ID NO: 524 - DNA, 20 bp, Rattus norvegicus
  source 1..20: mol_type = unassigned DNA
ttgatatagactttacgtgc

SEQ ID NO: 525 - DNA, 20 bp, Rattus norvegicus
  source 1..20: mol_type = unassigned DNA
agctaactacccccccgggt

SEQ ID NO: 526 - DNA, 20 bp, Rattus norvegicus
  source 1..20: mol_type = unassigned DNA
cacctccagcatcgggcgag

SEQ ID NO: 527 - DNA, 20 bp, Rattus norvegicus
  source 1..20: mol_type = unassigned DNA
aggcggcgtcgtcgggatgt

SEQ ID NO: 528 - DNA, 20 bp, Rattus norvegicus
  source 1..20: mol_type = unassigned DNA
ccgtttggcccccagttcgg

SEQ ID NO: 529 - DNA, 20 bp, Rattus norvegicus
  source 1..20: mol_type = unassigned DNA
ttccagcccgcgactaagcg

SEQ ID NO: 530 - DNA, 20 bp, Rattus norvegicus
  source 1..20: mol_type = unassigned DNA
agagtgagggggttgcaacg

SEQ ID NO: 531 - DNA, 20 bp, Rattus norvegicus
  source 1..20: mol_type = unassigned DNA
ccgcaactcttggcgcgtcg

SEQ ID NO: 532 - DNA, 20 bp, Rattus norvegicus
  source 1..20: mol_type = unassigned DNA
tgatcccgctcgcccgatgc

SEQ ID NO: 533 - DNA, 20 bp, Rattus norvegicus
  source 1..20: mol_type = unassigned DNA
ctggaagaggcggcgtcgtc

SEQ ID NO: 534 - DNA, 20 bp, Rattus norvegicus
  source 1..20: mol_type = unassigned DNA
aaccccgcttagtcgcgggc

SEQ ID NO: 535 - DNA, 20 bp, Rattus norvegicus
  source 1..20: mol_type = unassigned DNA
attgggaccgccacgccggt

SEQ ID NO: 536 - DNA, 20 bp, Rattus norvegicus
  source 1..20: mol_type = unassigned DNA
tccagaaccgcgtctcgacg

SEQ ID NO: 537 - DNA, 20 bp, Rattus norvegicus
  source 1..20: mol_type = unassigned DNA
cgcgcacagaacgcgtacgc

SEQ ID NO: 538 - DNA, 20 bp, Rattus norvegicus
  source 1..20: mol_type = unassigned DNA
gtgaaaccccgcttagtcgc

SEQ ID NO: 539 - DNA, 20 bp, Rattus norvegicus
  source 1..20: mol_type = unassigned DNA
ccccgacgcgccaagagttg

SEQ ID NO: 540 - DNA, 20 bp, Rattus norvegicus
  source 1..20: mol_type = unassigned DNA
accgcgtctcgacgcggaga

SEQ ID NO: 541 - DNA, 20 bp, Rattus norvegicus
  source 1..20: mol_type = unassigned DNA
ccgcgcacagaacgcgtacg

SEQ ID NO: 542 - DNA, 20 bp, Rattus norvegicus
  source 1..20: mol_type = unassigned DNA
ggtgaaaccccgcttagtcg

SEQ ID NO: 543 - DNA, 20 bp, Rattus norvegicus
  source 1..20: mol_type = unassigned DNA
actcttggcgcgtcggggca

SEQ ID NO: 544 - DNA, 20 bp, Rattus norvegicus
  source 1..20: mol_type = unassigned DNA
tccttctccgcgtcgagacg

SEQ ID NO: 545 - DNA, 20 bp, Rattus norvegicus
  source 1..20: mol_type = unassigned DNA
acggtccggacctccgaact

SEQ ID NO: 546 - DNA, 20 bp, Rattus norvegicus
  source 1..20: mol_type = unassigned DNA
ggcgccagccgctcgctcta

SEQ ID NO: 547 - DNA, 20 bp, Rattus norvegicus
  source 1..20: mol_type = unassigned DNA
gacttccgagttcgcaagcg

SEQ ID NO: 548 - DNA, 20 bp, Rattus norvegicus
  source 1..20: mol_type = unassigned DNA
tgcgaactcggaagtccaat

SEQ ID NO: 549 - DNA, 20 bp, Rattus norvegicus
  source 1..20: mol_type = unassigned DNA
tctggaagaggcggcgtcgt

SEQ ID NO: 550 - DNA, 20 bp, Rattus norvegicus
  source 1..20: mol_type = unassigned DNA
tcttagccccgagacccggt

SEQ ID NO: 551 - DNA, 20 bp, Rattus norvegicus
  source 1..20: mol_type = unassigned DNA
ccctccggcgccgtgttttc

SEQ ID NO: 552 - DNA, 20 bp, Rattus norvegicus
  source 1..20: mol_type = unassigned DNA
ccagaaaacacggcgccgga

SEQ ID NO: 553 - DNA, 17 bp, Danio rerio
  source 1..17: mol_type = unassigned DNA
atcaatatctcgcccag

SEQ ID NO: 554 - DNA, 17 bp, Danio rerio
  source 1..17: mol_type = unassigned DNA
attaaacgtgttccact

SEQ ID NO: 555 - DNA, 17 bp, Danio rerio
  source 1..17: mol_type = unassigned DNA
acgtttaatcgctttct

SEQ ID NO: 556 - DNA, 17 bp, Danio rerio
  source 1..17: mol_type = unassigned DNA
caagatgcgtacggtca

SEQ ID NO: 557 - DNA, 17 bp, Danio rerio
  source 1..17: mol_type = unassigned DNA
tctgtgtactcgaatat

SEQ ID NO: 558 - DNA, 17 bp, Danio rerio
  source 1..17: mol_type = unassigned DNA
tcctgacttctgggcac

SEQ ID NO: 559 - DNA, 17 bp, Danio rerio
  source 1..17: mol_type = unassigned DNA
cccggtgcccagaagtc

SEQ ID NO: 560 - DNA, 17 bp, Danio rerio
  source 1..17: mol_type = unassigned DNA
ccggagatccattcatg

SEQ ID NO: 561 - DNA, 17 bp, Danio rerio
  source 1..17: mol_type = unassigned DNA
tgatgacccagaatcaa

SEQ ID NO: 562 - DNA, 17 bp, Danio rerio
  source 1..17: mol_type = unassigned DNA
tgaatgaccggtcctcc

SEQ ID NO: 563 - DNA, 17 bp, Danio rerio
  source 1..17: mol_type = unassigned DNA
tccaaaggggcttcgga

SEQ ID NO: 564 - DNA, 17 bp, Danio rerio
  source 1..17: mol_type = unassigned DNA
cttcagttcgctgtgca

SEQ ID NO: 565 - DNA, 17 bp, Danio rerio
  source 1..17: mol_type = unassigned DNA
gatacacgccggcataa

SEQ ID NO: 566 - DNA, 17 bp, Danio rerio
  source 1..17: mol_type = unassigned DNA
cacacgaggatacacgc

SEQ ID NO: 567 - DNA, 17 bp, Danio rerio
  source 1..17: mol_type = unassigned DNA
tcgctgtcctcttcact

SEQ ID NO: 568 - DNA, 17 bp, Danio rerio
  source 1..17: mol_type = unassigned DNA
ttaaagtgattcccagt

SEQ ID NO: 569 - DNA, 17 bp, Danio rerio
  source 1..17: mol_type = unassigned DNA
cagctgatcctccaact

SEQ ID NO: 570 - DNA, 17 bp, Danio rerio
  source 1..17: mol_type = unassigned DNA
atatttagagtaagaat

SEQ ID NO: 571 - DNA, 17 bp, Drosophila melanogaster
  source 1..17: mol_type = unassigned DNA
aatttttatcattcagt

SEQ ID NO: 572 - DNA, 20 bp, Drosophila melanogaster
  source 1..20: mol_type = unassigned DNA
gattcttccatgatcggcca

SEQ ID NO: 573 - DNA, 20 bp, Drosophila melanogaster
  source 1..20: mol_type = unassigned DNA
cgattgaaaatccacataaa

SEQ ID NO: 574 - DNA, 20 bp, Drosophila melanogaster
  source 1..20: mol_type = unassigned DNA
gctgatttcggacaaaagtc

SEQ ID NO: 575 - DNA, 20 bp, Drosophila melanogaster
  source 1..20: mol_type = unassigned DNA
aaacggatgacgtgcaacgt

SEQ ID NO: 576 - DNA, 20 bp, Drosophila melanogaster
  source 1..20: mol_type = unassigned DNA
cgttttgtgtgcgtgcgcac

SEQ ID NO: 577 - DNA, 20 bp, Drosophila melanogaster
  source 1..20: mol_type = unassigned DNA
ggaataatcttcgtctatcc

SEQ ID NO: 578 - DNA, 20 bp, Drosophila melanogaster
  source 1..20: mol_type = unassigned DNA
ttcgctcacgaacaccaaca

SEQ ID NO: 579 - DNA, 20 bp, Drosophila melanogaster
  source 1..20: mol_type = unassigned DNA
acaaagtacatagggtgttt

SEQ ID NO: 580 - DNA, 20 bp, Drosophila melanogaster
  source 1..20: mol_type = unassigned DNA
ccatcccccgtaaagagggt

SEQ ID NO: 581 - DNA, 20 bp, Drosophila melanogaster
  source 1..20: mol_type = unassigned DNA
tatttttagttggtaaatta

SEQ ID NO: 582 - DNA, 17 bp, Drosophila melanogaster
  source 1..17: mol_type = unassigned DNA
attcactctgggttatg

SEQ ID NO: 583 - DNA, 20 bp, Drosophila melanogaster
  source 1..20: mol_type = unassigned DNA
ctgctttccttggccgatca

SEQ ID NO: 584 - DNA, 20 bp, Drosophila melanogaster
  source 1..20: mol_type = unassigned DNA
gattatttgctccatttatg

SEQ ID NO: 585 - DNA, 20 bp, Drosophila melanogaster
  source 1..20: mol_type = unassigned DNA
ctctgtacagaatattttct

SEQ ID NO: 586 - DNA, 20 bp, Drosophila melanogaster
  source 1..20: mol_type = unassigned DNA
gcagcggcagtgagagacgt

SEQ ID NO: 587 - DNA, 20 bp, Drosophila melanogaster
  source 1..20: mol_type = unassigned DNA
tgtgcgcacgcacacaaaac

SEQ ID NO: 588 - DNA, 20 bp, Drosophila melanogaster
  source 1..20: mol_type = unassigned DNA
aattcgctaattgggcagcc

SEQ ID NO: 589 - DNA, 20 bp, Drosophila melanogaster
  source 1..20: mol_type = unassigned DNA
caaggaaattgacagatgta

SEQ ID NO: 590 - DNA, 20 bp, Drosophila melanogaster
  source 1..20: mol_type = unassigned DNA
gctctagcaaccacgtcaga

SEQ ID NO: 591 - DNA, 20 bp, Drosophila melanogaster
  source 1..20: mol_type = unassigned DNA
acaatacgaatgcgagaagg

SEQ ID NO: 592 - DNA, 20 bp, Drosophila melanogaster
  source 1..20: mol_type = unassigned DNA
aaataaaaattagtgtccgc

SEQ ID NO: 593 - DNA, 17 bp, Drosophila melanogaster
  source 1..17: mol_type = unassigned DNA
agagtgaataaattaca

SEQ ID NO: 594 - DNA, 20 bp, Drosophila melanogaster
  source 1..20: mol_type = unassigned DNA
ttattcaagacttacaccat

SEQ ID NO: 595 - DNA, 20 bp, Drosophila melanogaster
  source 1..20: mol_type = unassigned DNA
attatgacgttttttggtac

SEQ ID NO: 596 - DNA, 20 bp, Drosophila melanogaster
  source 1..20: mol_type = unassigned DNA
ttcgggcggtctaaagcagt

SEQ ID NO: 597 - DNA, 20 bp, Drosophila melanogaster
  source 1..20: mol_type = unassigned DNA
tgttactttttcgaacgttg

SEQ ID NO: 598 - DNA, 20 bp, Drosophila melanogaster
  source 1..20: mol_type = unassigned DNA
gttttgtgtgcgtgcgcaca

SEQ ID NO: 599 - DNA, 20 bp, Drosophila melanogaster
  source 1..20: mol_type = unassigned DNA
tgcccaattagcgaattagg

SEQ ID NO: 600 - DNA, 20 bp, Drosophila melanogaster
  source 1..20: mol_type = unassigned DNA
cgccccaaaagaaaatacgt

SEQ ID NO: 601 - DNA, 20 bp, Drosophila melanogaster
  source 1..20: mol_type = unassigned DNA
gctgcggctttcgtgaaatg

SEQ ID NO: 602 - DNA, 20 bp, Drosophila melanogaster
  source 1..20: mol_type = unassigned DNA
aaaaggaggagaacatatct

SEQ ID NO: 603 - DNA, 17 bp, Drosophila melanogaster
  source 1..17: mol_type = unassigned DNA
atgtaatttattcactc

SEQ ID NO: 604 - DNA, 20 bp, Drosophila melanogaster
  source 1..20: mol_type = unassigned DNA
agaactaagcacgtattttt

SEQ ID NO: 605 - DNA, 20 bp, Drosophila melanogaster
  source 1..20: mol_type = unassigned DNA
acaaacaatccaaataaaag

SEQ ID NO: 606 - DNA, 20 bp, Drosophila melanogaster
  source 1..20: mol_type = unassigned DNA
caacaaaaaagtgagctctg

SEQ ID NO: 607 - DNA, 20 bp, Drosophila melanogaster
  source 1..20: mol_type = unassigned DNA
cgttgttcgtttttgtagtt

SEQ ID NO: 608 - DNA, 20 bp, Drosophila melanogaster
  source 1..20: mol_type = unassigned DNA
ctctttctggtaaatgctgt

SEQ ID NO: 609 - DNA, 20 bp, Drosophila melanogaster
  source 1..20: mol_type = unassigned DNA
ttaggtgggattttcgtgta

SEQ ID NO: 610 - DNA, 20 bp, Drosophila melanogaster
  source 1..20: mol_type = unassigned DNA
ctacaaaactacacgaatta

SEQ ID NO: 611 - DNA, 20 bp, Drosophila melanogaster
  source 1..20: mol_type = unassigned DNA
gctctcgctctgcctcgctg

SEQ ID NO: 612 - DNA, 20 bp, Drosophila melanogaster
  source 1..20: mol_type = unassigned DNA
aaaggaggagaacatatctt

SEQ ID NO: 613 - DNA, 17 bp, Drosophila melanogaster
  source 1..17: mol_type = unassigned DNA
aatcaaatcggtacatt

SEQ ID NO: 614 - DNA, 20 bp, Drosophila melanogaster
  source 1..20: mol_type = unassigned DNA
atttcagctctcaacgcaaa

SEQ ID NO: 615 - DNA, 20 bp, Drosophila melanogaster
  source 1..20: mol_type = unassigned DNA
attctgaaaccacttttatt

SEQ ID NO: 616 - DNA, 20 bp, Drosophila melanogaster
  source 1..20: mol_type = unassigned DNA
gagctctgcggtagtgacgc

SEQ ID NO: 617 - DNA, 20 bp, Drosophila melanogaster
  source 1..20: mol_type = unassigned DNA
ctacaaaaacgaacaacgca

SEQ ID NO: 618 - DNA, 20 bp, Drosophila melanogaster
  source 1..20: mol_type = unassigned DNA
tactaaacacatactaaaac

SEQ ID NO: 619 - DNA, 20 bp, Drosophila melanogaster
  source 1..20: mol_type = unassigned DNA
gtcgatttgtagaactggtg

SEQ ID NO: 620 - DNA, 20 bp, Drosophila melanogaster
  source 1..20: mol_type = unassigned DNA
tggtacttttctctcgtaca

SEQ ID NO: 621 - DNA, 20 bp, Drosophila melanogaster
  source 1..20: mol_type = unassigned DNA
ttccatgcttctttagtgca

SEQ ID NO: 622 - DNA, 20 bp, Drosophila melanogaster
  source 1..20: mol_type = unassigned DNA
attaaaagcgtatttttagt

SEQ ID NO: 623 - DNA, 17 bp, Drosophila melanogaster
  source 1..17: mol_type = unassigned DNA
ggttcgacacgcagaaa

SEQ ID NO: 624 - DNA, 20 bp, Drosophila melanogaster
  source 1..20: mol_type = unassigned DNA
tggagcaaataatccattca

SEQ ID NO: 625 - DNA, 20 bp, Drosophila melanogaster
  source 1..20: mol_type = unassigned DNA
gctctgtacagaatattttc

SEQ ID NO: 626 - DNA, 20 bp, Drosophila melanogaster
  source 1..20: mol_type = unassigned DNA
atgttactttttcgaacgtt

SEQ ID NO: 627 - DNA, 20 bp, Drosophila melanogaster
  source 1..20: mol_type = unassigned DNA
atcccgttagtgtgtgagat

SEQ ID NO: 628 - DNA, 20 bp, Drosophila melanogaster
  source 1..20: mol_type = unassigned DNA
taggtgggattttcgtgtag

SEQ ID NO: 629 - DNA, 20 bp, Drosophila melanogaster
  source 1..20: mol_type = unassigned DNA
tctttatgtacacgagtata

SEQ ID NO: 630 - DNA, 20 bp, Drosophila melanogaster
  source 1..20: mol_type = unassigned DNA
ttccatgcactaaagaagca

SEQ ID NO: 631 - DNA, 20 bp, Drosophila melanogaster
  source 1..20: mol_type = unassigned DNA
ggtcgcgtcgataccatttt

SEQ ID NO: 632 - DNA, 20 bp, Drosophila melanogaster
  source 1..20: mol_type = unassigned DNA
ctttcttcctcttcttcggg

SEQ ID NO: 633 - DNA, 20 bp, Drosophila melanogaster
  source 1..20: mol_type = unassigned DNA
catgttactttttcgaacgt

SEQ ID NO: 634 - DNA, 20 bp, Drosophila melanogaster
  source 1..20: mol_type = unassigned DNA
tccccaatctcacacactaa

SEQ ID NO: 635 - DNA, 20 bp, Drosophila melanogaster
  source 1..20: mol_type = unassigned DNA
tgtaggggtccctatagtag

SEQ ID NO: 636 - DNA, 20 bp, Drosophila melanogaster
  source 1..20: mol_type = unassigned DNA
cacaaagtacatagggtgtt

SEQ ID NO: 637 - DNA, 20 bp, Drosophila melanogaster
  source 1..20: mol_type = unassigned DNA
tcccccatcccccgtaaaga

SEQ ID NO: 638 - DNA, 20 bp, Drosophila melanogaster
  source 1..20: mol_type = unassigned DNA
ctttagaccgcccgaagaag

SEQ ID NO: 639 - DNA, 20 bp, Drosophila melanogaster
  source 1..20: mol_type = unassigned DNA
tacaaaaacgaacaacgcaa

SEQ ID NO: 640 - DNA, 20 bp, Drosophila melanogaster
  source 1..20: mol_type = unassigned DNA
gttgaatcgcctgtctttaa

SEQ ID NO: 641 - DNA, 20 bp, Drosophila melanogaster
  source 1..20: mol_type = unassigned DNA
ccgcgctgctcatccaaact

SEQ ID NO: 642 - DNA, 20 bp, Drosophila melanogaster
  source 1..20: mol_type = unassigned DNA
cttcagcgcacaaagtacat

SEQ ID NO: 643 - DNA, 20 bp, Drosophila melanogaster
  source 1..20: mol_type = unassigned DNA
gcaacaatacgaatgcgaga

SEQ ID NO: 644 - DNA, 20 bp, Drosophila melanogaster
  source 1..20: mol_type = unassigned DNA
gccggcagaggcagtgaccg

SEQ ID NO: 645 - DNA, 20 bp, Drosophila melanogaster
  source 1..20: mol_type = unassigned DNA
cgcaagggagcaatgggtac

SEQ ID NO: 646 - DNA, 20 bp, Drosophila melanogaster
  source 1..20: mol_type = unassigned DNA
ttgaatcgcctgtctttaat

SEQ ID NO: 647 - DNA, 20 bp, Drosophila melanogaster
  source 1..20: mol_type = unassigned DNA
agaaactttcacggcaccgt

SEQ ID NO: 648 - DNA, 20 bp, Drosophila melanogaster
  source 1..20: mol_type = unassigned DNA
gcaagcgaaatggcgcttcg

SEQ ID NO: 649 - DNA, 20 bp, Drosophila melanogaster
  source 1..20: mol_type = unassigned DNA
agaggcagtgaccgaggcag

SEQ ID NO: 650 - DNA, 20 bp, Drosophila melanogaster
  source 1..20: mol_type = unassigned DNA
ggaaaaaacccattaaagac

SEQ ID NO: 651 - DNA, 20 bp, Drosophila melanogaster
  source 1..20: mol_type = unassigned DNA
atgcacggaataagctccaa

SEQ ID NO: 652 - DNA, 20 bp, Drosophila melanogaster
  source 1..20: mol_type = unassigned DNA
tgtaccaccaaccctcttta

SEQ ID NO: 653 - DNA, 20 bp, Drosophila melanogaster
  source 1..20: mol_type = unassigned DNA
gaaatcttcattccctccaa

SEQ ID NO: 654 - DNA, 20 bp, Drosophila melanogaster
  source 1..20: mol_type = unassigned DNA
aaggaaattgacagatgtat

SEQ ID NO: 655 - DNA, 20 bp, Drosophila melanogaster
  source 1..20: mol_type = unassigned DNA
gtaccaccaaccctctttac

SEQ ID NO: 656 - DNA, 20 bp, Drosophila melanogaster
  source 1..20: mol_type = unassigned DNA
cgcaaaaagcctctactata

SEQ ID NO: 657 - DNA, 20 bp, Drosophila melanogaster
  source 1..20: mol_type = unassigned DNA
taccaccaaccctctttacg

SEQ ID NO: 658 - DNA, 20 bp, Drosophila melanogaster
  source 1..20: mol_type = unassigned DNA
tcgcaaaaagcctctactat

SEQ ID NO: 659 - DNA, 20 bp, Drosophila melanogaster
  source 1..20: mol_type = unassigned DNA
accaccaaccctctttacgg

SEQ ID NO: 660 - DNA, 20 bp, Drosophila melanogaster
  source 1..20: mol_type = unassigned DNA
ccaaccctctttacggggga

SEQ ID NO: 661 - DNA, 20 bp, Drosophila melanogaster
  source 1..20: mol_type = unassigned DNA
caaccctctttacgggggat

SEQ ID NO: 662 - DNA, 20 bp, Drosophila melanogaster
  source 1..20: mol_type = unassigned DNA
atcccccatcccccgtaaag

SEQ ID NO: 663 - DNA, 17 bp, Caenorhabditis elegans
  source 1..17: mol_type = unassigned DNA
aagagagtcagattgga

SEQ ID NO: 664 - DNA, 17 bp, Caenorhabditis elegans
  source 1..17: mol_type = unassigned DNA
tctgactctcttgtgtt

SEQ ID NO: 665 - DNA, 17 bp, Caenorhabditis elegans
  source 1..17: mol_type = unassigned DNA
acacaagagagtcagat

SEQ ID NO: 666 - DNA, 17 bp, Caenorhabditis elegans
  source 1..17: mol_type = unassigned DNA
attttcaggtaaaagtt

SEQ ID NO: 667 - DNA, 17 bp, Caenorhabditis elegans
  source 1..17: mol_type = unassigned DNA
gaagacgctcgaattct

SEQ ID NO: 668 - DNA, 17 bp, Caenorhabditis elegans
  source 1..17: mol_type = unassigned DNA
tatgtgacgtcttatct

SEQ ID NO: 669 - DNA, 17 bp, Caenorhabditis elegans
  source 1..17: mol_type = unassigned DNA
tgttcctcttgatcatc

SEQ ID NO: 670 - DNA, 17 bp, Caenorhabditis elegans
  source 1..17: mol_type = unassigned DNA
aagaggaacataatcta

SEQ ID NO: 671 - DNA, 17 bp, Caenorhabditis elegans
  source 1..17: mol_type = unassigned DNA
tctaggccacgtcttgc

SEQ ID NO: 672 - DNA, 17 bp, Caenorhabditis elegans
  source 1..17: mol_type = unassigned DNA
agtattctatattcagt

SEQ ID NO: 673 - DNA, 17 bp, Caenorhabditis elegans
  source 1..17: mol_type = unassigned DNA
tgcatggtttgaatctt

SEQ ID NO: 674 - DNA, 17 bp, Caenorhabditis elegans
  source 1..17: mol_type = unassigned DNA
gcaactgatgtgtttct

SEQ ID NO: 675 - DNA, 17 bp, Caenorhabditis elegans
  source 1..17: mol_type = unassigned DNA
gatgtgtttctaggctc

SEQ ID NO: 676 - DNA, 17 bp, Caenorhabditis elegans
  source 1..17: mol_type = unassigned DNA
aagttctagatcacgag

SEQ ID NO: 677 - DNA, 17 bp, Caenorhabditis elegans
  source 1..17: mol_type = unassigned DNA
tcccaaatcatccttga

SEQ ID NO: 678 - DNA, 17 bp, Caenorhabditis elegans
  source 1..17: mol_type = unassigned DNA
tgggttttaaaccatca

SEQ ID NO: 679 - DNA, 17 bp, Caenorhabditis elegans
  source 1..17: mol_type = unassigned DNA
gacgggttggaggcaga

SEQ ID NO: 680 - DNA, 17 bp, Caenorhabditis elegans
  source 1..17: mol_type = unassigned DNA
cctccaacccgtccaat

SEQ ID NO: 681 - DNA, 17 bp, Caenorhabditis elegans
  source 1..17: mol_type = unassigned DNA
aaaccgattggacgggt

SEQ ID NO: 682 - DNA, 17 bp, Caenorhabditis elegans
  source 1..17: mol_type = unassigned DNA
ttggaaaccgattggac

SEQ ID NO: 683 - DNA, 17 bp, Caenorhabditis elegans
  source 1..17: mol_type = unassigned DNA
tgtctattgtacaagct

SEQ ID NO: 684 - DNA, 17 bp, Caenorhabditis elegans
  source 1..17: mol_type = unassigned DNA
gtctattgtacaagctt

SEQ ID NO: 685 - DNA, 17 bp, Caenorhabditis elegans
  source 1..17: mol_type = unassigned DNA
tctattgtacaagcttg

SEQ ID NO: 686 - DNA, 17 bp, Caenorhabditis elegans
  source 1..17: mol_type = unassigned DNA
tagcactcgacccgaaa

SEQ ID NO: 687 - DNA, 17 bp, Caenorhabditis elegans
  source 1..17: mol_type = unassigned DNA
cactcgacccgaaacgg

SEQ ID NO: 688 - DNA, 17 bp, Caenorhabditis elegans
  source 1..17: mol_type = unassigned DNA
actcgacccgaaacggt

SEQ ID NO: 689 - DNA, 16 bp, Caenorhabditis elegans
  source 1..16: mol_type = unassigned DNA
acccgaaacggtggga

SEQ ID NO: 690 - DNA, 17 bp, Caenorhabditis elegans
  source 1..17: mol_type = unassigned DNA
cccgaaacggtgggaag

SEQ ID NO: 691 - DNA, 17 bp, Caenorhabditis elegans
  source 1..17: mol_type = unassigned DNA
ccgaaacggtgggaagg

SEQ ID NO: 692 - DNA, 17 bp, Caenorhabditis elegans
  source 1..17: mol_type = unassigned DNA
aacggtgggaagggggg

SEQ ID NO: 693 - DNA, 17 bp, Caenorhabditis elegans
  source 1..17: mol_type = unassigned DNA
ccccttcccaccgtttc

SEQ ID NO: 694 - DNA, 17 bp, Caenorhabditis elegans
  source 1..17: mol_type = unassigned DNA
cccccttcccaccgttt

SEQ ID NO: 695 - DNA, 17 bp, Caenorhabditis elegans
  source 1..17: mol_type = unassigned DNA
ggggggaggacatccgc

SEQ ID NO: 696 - DNA, 17 bp, Caenorhabditis elegans
  source 1..17: mol_type = unassigned DNA
taggtgactgactccgg

SEQ ID NO: 697 - DNA, 17 bp, Caenorhabditis elegans
  source 1..17: mol_type = unassigned DNA
ttgtaggtgactgactc

SEQ ID NO: 698 - DNA, 17 bp, Caenorhabditis elegans
  source 1..17: mol_type = unassigned DNA
ggattagctgctccaat

SEQ ID NO: 699 - DNA, 17 bp, Caenorhabditis elegans
  source 1..17: mol_type = unassigned DNA
attagctgctccaattg

SEQ ID NO: 700 - DNA, 17 bp, Caenorhabditis elegans
  source 1..17: mol_type = unassigned DNA
acttagcacaccccaat

SEQ ID NO: 701 - DNA, 17 bp, Caenorhabditis elegans
  source 1..17: mol_type = unassigned DNA
aattgtctatgtttaat

SEQ ID NO: 702 - DNA, 17 bp, Caenorhabditis elegans
  source 1..17: mol_type = unassigned DNA
taatgggtgtatcgtat

SEQ ID NO: 703 - DNA, 17 bp, Caenorhabditis elegans
  source 1..17: mol_type = unassigned DNA
agcactttttgagtggt

SEQ ID NO: 704 - DNA, 17 bp, Caenorhabditis elegans
  source 1..17: mol_type = unassigned DNA
aggaagtgagagtcact

SEQ ID NO: 705 - DNA, 17 bp, Caenorhabditis elegans
  source 1..17: mol_type = unassigned DNA
ggaagtgagagtcacta

SEQ ID NO: 706 - DNA, 17 bp, Caenorhabditis elegans
  source 1..17: mol_type = unassigned DNA
gaatggataaagccacg

SEQ ID NO: 707 - DNA, 17 bp, Caenorhabditis elegans
  source 1..17: mol_type = unassigned DNA
ccacgtggcaatcatat

SEQ ID NO: 708 - DNA, 17 bp, Caenorhabditis elegans
  source 1..17: mol_type = unassigned DNA
gtttatagtaggatttt

SEQ ID NO: 709 - DNA, 20 bp, Sus scrofa
  source 1..20: mol_type = unassigned DNA
aggatacctcaacgactacg

SEQ ID NO: 710 - DNA, 20 bp, Sus scrofa
  source 1..20: mol_type = unassigned DNA
gcgctgcccgacgtgtggca

SEQ ID NO: 711 - DNA, 20 bp, Sus scrofa
  source 1..20: mol_type = unassigned DNA
cttcaagcaatagggtcccg

SEQ ID NO: 712 - DNA, 20 bp, Sus scrofa
  source 1..20: mol_type = unassigned DNA
atgacgcatatcaaatcgca

SEQ ID NO: 713 - DNA, 20 bp, Sus scrofa
  source 1..20: mol_type = unassigned DNA
tattgctctatagtcggctt

SEQ ID NO: 714 - DNA, 20 bp, Sus scrofa
  source 1..20: mol_type = unassigned DNA
ataaccgacttagcgaattc

SEQ ID NO: 715 - DNA, 20 bp, Sus scrofa
  source 1..20: mol_type = unassigned DNA
aggctgctgaccgtattgcc

SEQ ID NO: 716 - DNA, 20 bp, Sus scrofa
  source 1..20: mol_type = unassigned DNA
ggatacctcaacgactacgc

SEQ ID NO: 717 - DNA, 20 bp, Sus scrofa
  source 1..20: mol_type = unassigned DNA
ctcagccccgtgcaggccta

SEQ ID NO: 718 - DNA, 20 bp, Sus scrofa
  source 1..20: mol_type = unassigned DNA
taggaaagcggctcggattg

SEQ ID NO: 719 - DNA, 20 bp, Sus scrofa
  source 1..20: mol_type = unassigned DNA
ggcatagacgggcgttaagt

SEQ ID NO: 720 - DNA, 20 bp, Sus scrofa
  source 1..20: mol_type = unassigned DNA
gcggtccctagacccaaccg

SEQ ID NO: 721 - DNA, 20 bp, Sus scrofa
  source 1..20: mol_type = unassigned DNA
agcccgggagtctttcgcta

SEQ ID NO: 722 - DNA, 20 bp, Sus scrofa
  source 1..20: mol_type = unassigned DNA
ctgctagtggcggccgttta

SEQ ID NO: 723 - DNA, 20 bp, Sus scrofa
  source 1..20: mol_type = unassigned DNA
gatacctcaacgactacgcg

SEQ ID NO: 724 - DNA, 20 bp, Sus scrofa
  source 1..20: mol_type = unassigned DNA
ttttcccagcaatagggtcg

SEQ ID NO: 725 - DNA, 20 bp, Sus scrofa
  source 1..20: mol_type = unassigned DNA
cgaatgcccgggtacgaggg

SEQ ID NO: 726 - DNA, 20 bp, Sus scrofa
  source 1..20: mol_type = unassigned DNA
ggaaagaaagtctgcgcgtc

SEQ ID NO: 727 - DNA, 20 bp, Sus scrofa
  source 1..20: mol_type = unassigned DNA
cgggccccgcgtagtcgttg

SEQ ID NO: 728 - DNA, 20 bp, Sus scrofa
  source 1..20: mol_type = unassigned DNA
ggtctcctcgaccctattgc

SEQ ID NO: 729 - DNA, 20 bp, Sus scrofa
  source 1..20: mol_type = unassigned DNA
tttatgaacggattgcactc

SEQ ID NO: 730 - DNA, 20 bp, Sus scrofa
  source 1..20: mol_type = unassigned DNA
gcagaggccggcgggtgtaa

SEQ ID NO: 731 - DNA, 20 bp, Sus scrofa
  source 1..20: mol_type = unassigned DNA
ggcgtcgccatcgtagacgg

SEQ ID NO: 732 - DNA, 20 bp, Sus scrofa
  source 1..20: mol_type = unassigned DNA
gtctctgcgacgcgatccag

SEQ ID NO: 733 - DNA, 20 bp, Sus scrofa
  source 1..20: mol_type = unassigned DNA
tcacccaccaaccgttcatt

SEQ ID NO: 734 - DNA, 20 bp, Sus scrofa
  source 1..20: mol_type = unassigned DNA
cgtctacgatggcgacgccg

SEQ ID NO: 735 - DNA, 20 bp, Sus scrofa
  source 1..20: mol_type = unassigned DNA
agtctctgcgacgcgatcca

SEQ ID NO: 736 - DNA, 20 bp, Sus scrofa
  source 1..20: mol_type = unassigned DNA
gtaggtgcctaatgaacggt

SEQ ID NO: 737 - DNA, 20 bp, Sus scrofa
  source 1..20: mol_type = unassigned DNA
tggctacatcaacggcgacg

SEQ ID NO: 738 - DNA, 20 bp, Sus scrofa
  source 1..20: mol_type = unassigned DNA
gagtctctgcgacgcgatcc

SEQ ID NO: 739 - DNA, 20 bp, Sus scrofa
  source 1..20: mol_type = unassigned DNA
ggggcccacggttgggtcta

SEQ ID NO: 740 - DNA, 20 bp, Sus scrofa
  source 1..20: mol_type = unassigned DNA
acctccgccgtcgccgtcgg

SEQ ID NO: 741 - DNA, 20 bp, Sus scrofa
  source 1..20: mol_type = unassigned DNA
ttggcagaggatgcgaggcg

SEQ ID NO: 742 - DNA, 20 bp, Sus scrofa
  source 1..20: mol_type = unassigned DNA
cccgggccctgagcgcgcct

SEQ ID NO: 743 - DNA, 20 bp, Sus scrofa
  source 1..20: mol_type = unassigned DNA
cggcacgcttgcggcgagtg

SEQ ID NO: 744 - DNA, 20 bp, Bos taurus
  source 1..20: mol_type = unassigned DNA
cctgccagtatctcaaaccg

SEQ ID NO: 745 - DNA, 23 bp, Homo sapiens
  source 1..23: mol_type = unassigned DNA
cacatcgatgtcctccccattcc

SEQ ID NO: 746 - DNA, 20 bp, Homo sapiens
  source 1..20: mol_type = unassigned DNA
atggggaggacatcgatgtc

SEQ ID NO: 747 - RNA, 20 nt, synthetic construct
  misc_feature 1..20: note = source = /note="Description of Artificial Sequence: Synthetic oligonucleotide"
  source 1..20: mol_type = other RNA
cacatcgatgtcctccccat

SEQ ID NO: 748 - DNA, 24 bp, synthetic construct
  misc_feature 1..24: note = source = /note="Description of Artificial Sequence: Synthetic oligonucleotide"
  source 1..24: mol_type = other DNA
caccgacatcgatgtcctccccat

SEQ ID NO: 749 - DNA, 24 bp, synthetic construct
  misc_feature 1..24: note = source = /note="Description of Artificial Sequence: Synthetic oligonucleotide"
  source 1..24: mol_type = other DNA
aaacatggggaggacatcgatgtc

SEQ ID NO: 750 - DNA, 26 bp, synthetic construct
  misc_feature 1..26: note = source = /note="Description of Artificial Sequence: Synthetic oligonucleotide"
  source 1..26: mol_type = other DNA
gagggcctatttcccatgattccttc

SEQ ID NO: 751 - DNA, 125 bp, synthetic construct
  misc_feature 1..125: note = source = /note="Description of Artificial Sequence: Synthetic polynucleotide"
  source 1..125: mol_type = other DNA
aaaaaaagcaccgactcggtgccactttttcaagttgataacggactagccttattttaacttgctatttctagctctaaaacatggggaggacatcgatgtcggtgtttcgtcctttccacaag

SEQ ID NO: 752 - DNA, 23 bp, Homo sapiens
  source 1..23: mol_type = unassigned DNA
cacataggtgtcctccccatagg

SEQ ID NO: 753 - DNA, 23 bp, Homo sapiens
  source 1..23: mol_type = unassigned DNA
gaaatcaaggtcctccccatagg

SEQ ID NO: 754 - DNA, 23 bp, Homo sapiens
  source 1..23: mol_type = unassigned DNA
aacttccatctcctccccatggg

SEQ ID NO: 755 - DNA, 23 bp, Homo sapiens
  source 1..23: mol_type = unassigned DNA
gccttctctgtcctccccatggg

SEQ ID NO: 756 - DNA, 23 bp, Homo sapiens
  source 1..23: mol_type = unassigned DNA
gagacccatttcctccccattag

SEQ ID NO: 757 - DNA, 23 bp, Homo sapiens
  source 1..23: mol_type = unassigned DNA
aaaaacaatgtcctccccattag

SEQ ID NO: 758 - DNA, 23 bp, Homo sapiens
  source 1..23: mol_type = unassigned DNA
gccctcgctgccctccccatcag

SEQ ID NO: 759 - DNA, 23 bp, Homo sapiens
  source 1..23: mol_type = unassigned DNA
cacggctgtgtcctccccattgg

SEQ ID NO: 760 - DNA, 23 bp, Homo sapiens
  source 1..23: mol_type = unassigned DNA
tgcttcactgtcctccccatagg

SEQ ID NO: 761 - DNA, 23 bp, Homo sapiens
  source 1..23: mol_type = unassigned DNA
gtcaacgttgtcctcctcattgg

SEQ ID NO: 762 - DNA, 23 bp, synthetic construct
  misc_feature 1..23: note = source = /note="Description of Artificial Sequence: Synthetic primer"
  source 1..23: mol_type = other DNA
gagggcctatttcccatgattcc

SEQ ID NO: 763 - DNA, 23 bp, synthetic construct
  misc_feature 1..23: note = source = /note="Description of Artificial Sequence: Synthetic oligonucleotide"
  source 1..23: mol_type = other DNA
gagggcctatttcccatgattcc

SEQ ID NO: 764 - DNA, 22 bp, synthetic construct
  misc_feature 1..22: note = source = /note="Description of Artificial Sequence: Synthetic oligonucleotide"
  source 1..22: mol_type = other DNA
cttgtggaaaggacgaaacacc

SEQ ID NO: 765 - DNA, 45 bp, synthetic construct
  modified_base 4..23: mod_base = OTHER; note = a, c, t, g, unknown or other
  misc_feature 1..45: note = source = /note="Description of Artificial Sequence: Synthetic oligonucleotide"
  source 1..45: mol_type = other DNA
aacnnnnnnnnnnnnnnnnnnnnggtgtttcgtcctttccacaag

SEQ ID NO: 766-767 - skipped (2 entries)

SEQ ID NO: 768 - DNA, 54 bp, synthetic construct
  misc_feature 1..54: note = source = /note="Description of Artificial Sequence: Synthetic oligonucleotide"
  source 1..54: mol_type = other DNA
aacaccgggtcttcgagaagacctgttttagagctagaaatagcaagttaaaat

SEQ ID NO: 769 - RNA, 20 nt, synthetic construct
  misc_feature 1..20: note = source = /note="Description of Artificial Sequence: Synthetic oligonucleotide"
  source 1..20: mol_type = other RNA
gagtccgagcagaagaagaa

SEQ ID NO: 770 - RNA, 20 nt, synthetic construct
  misc_feature 1..20: note = source = /note="Description of Artificial Sequence: Synthetic oligonucleotide"
  source 1..20: mol_type = other RNA
gtcacctccaatgactaggg

SEQ ID NO: 771 - RNA, 20 nt, synthetic construct
  misc_feature 1..20: note = source = /note="Description of Artificial Sequence: Synthetic oligonucleotide"
  source 1..20: mol_type = other RNA
gtcacctccaatgactagaa

SEQ ID NO: 772 - RNA, 20 nt, synthetic construct
  misc_feature 1..20: note = source = /note="Description of Artificial Sequence: Synthetic oligonucleotide"
  source 1..20: mol_type = other RNA
gtcacctccaatgactgagg

SEQ ID NO: 773 - RNA, 20 nt, synthetic construct
  misc_feature 1..20: note = source = /note="Description of Artificial Sequence: Synthetic oligonucleotide"
  source 1..20: mol_type = other RNA
gtcacctccaatgatcaggg

SEQ ID NO: 774 - RNA, 20 nt, synthetic construct
  misc_feature 1..20: note = source = /note="Description of Artificial Sequence: Synthetic oligonucleotide"
  source 1..20: mol_type = other RNA
gtcacctccaatagctaggg

SEQ ID NO: 775 - RNA, 20 nt, synthetic construct
  misc_feature 1..20: note = source = /note="Description of Artificial Sequence: Synthetic oligonucleotide"
  source 1..20: mol_type = other RNA
gtcacctccagcgactaggg

SEQ ID NO: 776 - RNA, 20 nt, synthetic construct
  misc_feature 1..20: note = source = /note="Description of Artificial Sequence: Synthetic oligonucleotide"
  source 1..20: mol_type = other RNA
gtcacctctgatgactaggg

SEQ ID NO: 777 - RNA, 20 nt, synthetic construct
  misc_feature 1..20: note = source = /note="Description of Artificial Sequence: Synthetic oligonucleotide"
  source 1..20: mol_type = other RNA
gtcaccctcaatgactaggg

SEQ ID NO: 778 - RNA, 20 nt, synthetic construct
  misc_feature 1..20: note = source = /note="Description of Artificial Sequence: Synthetic oligonucleotide"
  source 1..20: mol_type = other RNA
gtcatttccaatgactaggg

SEQ ID NO: 779 - RNA, 20 nt, synthetic construct
  misc_feature 1..20: note = source = /note="Description of Artificial Sequence: Synthetic oligonucleotide"
  source 1..20: mol_type = other RNA
gttgcctccaatgactaggg

SEQ ID NO: 780 - RNA, 20 nt, synthetic construct
  misc_feature 1..20: note = source = /note="Description of Artificial Sequence: Synthetic oligonucleotide"
  source 1..20: mol_type = other RNA
gtcacctccaatgactgaag

SEQ ID NO: 781 - RNA, 20 nt, synthetic construct
  misc_feature 1..20: note = source = /note="Description of Artificial Sequence: Synthetic oligonucleotide"
  source 1..20: mol_type = other RNA
gtcacctccaatggtcaggg

SEQ ID NO: 782 - RNA, 20 nt, synthetic construct
  misc_feature 1..20: note = source = /note="Description of Artificial Sequence: Synthetic oligonucleotide"
  source 1..20: mol_type = other RNA
gtcacctccagcaactaggg

SEQ ID NO: 783 - RNA, 20 nt, synthetic construct
  misc_feature 1..20: note = source = /note="Description of Artificial Sequence: Synthetic oligonucleotide"
  source 1..20: mol_type = other RNA
gtcaccttcgatgactaggg

SEQ ID NO: 784 - RNA, 20 nt, synthetic construct
  misc_feature 1..20: note = source = /note="Description of Artificial Sequence: Synthetic oligonucleotide"
  source 1..20: mol_type = other RNA
gtcattcccaatgactaggg

SEQ ID NO: 785 - RNA, 20 nt, synthetic construct
  misc_feature 1..20: note = source = /note="Description of Artificial Sequence: Synthetic oligonucleotide"
  source 1..20: mol_type = other RNA
gctgcctccaatgactaggg

SEQ ID NO: 786 - RNA, 20 nt, synthetic construct
  misc_feature 1..20: note = source = /note="Description of Artificial Sequence: Synthetic oligonucleotide"
  source 1..20: mol_type = other RNA
gtcacctccaatgaccgaaa

SEQ ID NO: 787 - RNA, 20 nt, synthetic construct
  misc_feature 1..20: note = source = /note="Description of Artificial Sequence: Synthetic oligonucleotide"
  source 1..20: mol_type = other RNA
gtcacctccaatagtcgggg

SEQ ID NO: 788 - RNA, 20 nt, synthetic construct
  misc_feature 1..20: note = source = /note="Description of Artificial Sequence: Synthetic oligonucleotide"
  source 1..20: mol_type = other RNA
gtcacctccggcagctaggg

SEQ ID NO: 789 - RNA, 20 nt, synthetic construct
  misc_feature 1..20: note = source = /note="Description of Artificial Sequence: Synthetic oligonucleotide"
  source 1..20: mol_type = other RNA
gtcacccttggtgactaggg

SEQ ID NO: 790 - RNA, 20 nt, synthetic construct
  misc_feature 1..20: note = source = /note="Description of Artificial Sequence: Synthetic oligonucleotide"
  source 1..20: mol_type = other RNA
gtcgttctcaatgactaggg

SEQ ID NO: 791 - RNA, 20 nt, synthetic construct
  misc_feature 1..20: note = source = /note="Description of Artificial Sequence: Synthetic oligonucleotide"
  source 1..20: mol_type = other RNA
gacatcgatgtcctccccat

SEQ ID NO: 792 - RNA, 20 nt, synthetic construct
  misc_feature 1..20: note = source = /note="Description of Artificial Sequence: Synthetic oligonucleotide"
  source 1..20: mol_type = other RNA
gacatcgatgtcctccccgc

SEQ ID NO: 793 - RNA, 20 nt, synthetic construct
  misc_feature 1..20: note = source = /note="Description of Artificial Sequence: Synthetic oligonucleotide"
  source 1..20: mol_type = other RNA
gacatcgatgtcctccttat

SEQ ID NO: 794 - RNA, 20 nt, synthetic construct
  misc_feature 1..20: note = source = /note="Description of Artificial Sequence: Synthetic oligonucleotide"
  source 1..20: mol_type = other RNA
gacatcgatgtcctttccat

SEQ ID NO: 795 - RNA, 20 nt, synthetic construct
  misc_feature 1..20: note = source = /note="Description of Artificial Sequence: Synthetic oligonucleotide"
  source 1..20: mol_type = other RNA
gacatcgatgtctcccccat

SEQ ID NO: 796 - RNA, 20 nt, synthetic construct
  misc_feature 1..20: note = source = /note="Description of Artificial Sequence: Synthetic oligonucleotide"
  source 1..20: mol_type = other RNA
gacatcgatgctctccccat

SEQ ID NO: 797 - RNA, 20 nt, synthetic construct
  misc_feature 1..20: note = source = /note="Description of Artificial Sequence: Synthetic oligonucleotide"
  source 1..20: mol_type = other RNA
gacatcgacatcctccccat

SEQ ID NO: 798 - RNA, 20 nt, synthetic construct
  misc_feature 1..20: note = source = /note="Description of Artificial Sequence: Synthetic oligonucleotide"
  source 1..20: mol_type = other RNA
gacatcagtgtcctccccat

SEQ ID NO: 799 - RNA, 20 nt, synthetic construct
  misc_feature 1..20: note = source = /note="Description of Artificial Sequence: Synthetic oligonucleotide"
  source 1..20: mol_type = other RNA
gacactgatgtcctccccat

SEQ ID NO: 800 - RNA, 20 nt, synthetic construct
  misc_feature 1..20: note = source = /note="Description of Artificial Sequence: Synthetic oligonucleotide"
  source 1..20: mol_type = other RNA
gatgtcgatgtcctccccat

SEQ ID NO: 801 - RNA, 20 nt, synthetic construct
  misc_feature 1..20: note = source = /note="Description of Artificial Sequence: Synthetic oligonucleotide"
  source 1..20: mol_type = other RNA
gacatcgatgtcctccttgt

SEQ ID NO: 802 - RNA, 20 nt, synthetic construct
  misc_feature 1..20: note = source = /note="Description of Artificial Sequence: Synthetic oligonucleotide"
  source 1..20: mol_type = other RNA
gacatcgatgtcccttccat

SEQ ID NO: 803 - RNA, 20 nt, synthetic construct
  misc_feature 1..20: note = source = /note="Description of Artificial Sequence: Synthetic oligonucleotide"
  source 1..20: mol_type = other RNA
gacatcgatgctttccccat

SEQ ID NO: 804 - RNA, 20 nt, synthetic construct
  misc_feature 1..20: note = source = /note="Description of Artificial Sequence: Synthetic oligonucleotide"
  source 1..20: mol_type = other RNA
gacatcggcatcctccccat

SEQ ID NO: 805 - RNA, 20 nt, synthetic construct
  misc_feature 1..20: note = source = /note="Description of Artificial Sequence: Synthetic oligonucleotide"
  source 1..20: mol_type = other RNA
gacactaatgtcctccccat

SEQ ID NO: 806 - RNA, 20 nt, synthetic construct
  misc_feature 1..20: note = source = /note="Description of Artificial Sequence: Synthetic oligonucleotide"
  source 1..20: mol_type = other RNA
ggtgtcgatgtcctccccat

SEQ ID NO: 807 - RNA, 20 nt, synthetic construct
  misc_feature 1..20: note = source = /note="Description of Artificial Sequence: Synthetic oligonucleotide"
  source 1..20: mol_type = other RNA
gacatcgatgtcctctttgc

SEQ ID NO: 808 - RNA, 20 nt, synthetic construct
  misc_feature 1..20: note = source = /note="Description of Artificial Sequence: Synthetic oligonucleotide"
  source 1..20: mol_type = other RNA
gacatcgatgtctctttcat

SEQ ID NO: 809 - RNA, 20 nt, synthetic construct
  misc_feature 1..20: note = source = /note="Description of Artificial Sequence: Synthetic oligonucleotide"
  source 1..20: mol_type = other RNA
gacatcgatacttcccccat

SEQ ID NO: 810 - RNA, 20 nt, synthetic construct
  misc_feature 1..20: note = source = /note="Description of Artificial Sequence: Synthetic oligonucleotide"
  source 1..20: mol_type = other RNA
gacatcagcaccctccccat

SEQ ID NO: 811 - RNA, 20 nt, synthetic construct
  misc_feature 1..20: note = source = /note="Description of Artificial Sequence: Synthetic oligonucleotide"
  source 1..20: mol_type = other RNA
gacgctagtgtcctccccat

SEQ ID NO: 812 - RNA, 20 nt, synthetic construct
  misc_feature 1..20: note = source = /note="Description of Artificial Sequence: Synthetic oligonucleotide"
  source 1..20: mol_type = other RNA
gagtccgagcagaagaagaa

SEQ ID NO: 813 - RNA, 20 nt, synthetic construct
  misc_feature 1..20: note = source = /note="Description of Artificial Sequence: Synthetic oligonucleotide"
  source 1..20: mol_type = other RNA
gagtccgagcagaagaaggg

SEQ ID NO: 814 - RNA, 20 nt, synthetic construct
  misc_feature 1..20: note = source = /note="Description of Artificial Sequence: Synthetic oligonucleotide"
  source 1..20: mol_type = other RNA
gagtccgagcagaagagaaa

SEQ ID NO: 815 - RNA, 20 nt, synthetic construct
  misc_feature 1..20: note = source = /note="Description of Artificial Sequence: Synthetic oligonucleotide"
  source 1..20: mol_type = other RNA
gagtccgagcagaaagagaa

SEQ ID NO: 816 - RNA, 20 nt, synthetic construct
  misc_feature 1..20: note = source = /note="Description of Artificial Sequence: Synthetic oligonucleotide"
  source 1..20: mol_type = other RNA
gagtccgagcaggggaagaa

SEQ ID NO: 817 - RNA, 20 nt, synthetic construct
  misc_feature 1..20: note = source = /note="Description of Artificial Sequence: Synthetic oligonucleotide"
  source 1..20: mol_type = other RNA
gagtccgagcgaaagaagaa

SEQ ID NO: 818 - RNA, 20 nt, synthetic construct
  misc_feature 1..20: note = source = /note="Description of Artificial Sequence: Synthetic oligonucleotide"
  source 1..20: mol_type = other RNA
gagtccgaatagaagaagaa

SEQ ID NO: 819 - RNA, 20 nt, synthetic construct
  misc_feature 1..20: note = source = /note="Description of Artificial Sequence: Synthetic oligonucleotide"
  source 1..20: mol_type = other RNA
gagtccaggcagaagaagaa

SEQ ID NO: 820 - RNA, 20 nt, synthetic construct
  misc_feature 1..20: note = source = /note="Description of Artificial Sequence: Synthetic oligonucleotide"
  source 1..20: mol_type = other RNA
gagtctgagcagaagaagaa

SEQ ID NO: 821 - RNA, 20 nt, synthetic construct
  misc_feature 1..20: note = source = /note="Description of Artificial Sequence: Synthetic oligonucleotide"
  source 1..20: mol_type = other RNA
gaacccgagcagaagaagaa

SEQ ID NO: 822 - RNA, 20 nt, synthetic construct
  misc_feature 1..20: note = source = /note="Description of Artificial Sequence: Synthetic oligonucleotide"
  source 1..20: mol_type = other RNA
gagtccgagcagaagagaga

SEQ ID NO: 823 - RNA, 20 nt, synthetic construct
  misc_feature 1..20: note = source = /note="Description of Artificial Sequence: Synthetic oligonucleotide"
  source 1..20: mol_type = other RNA
gagtccgagcagagagagaa

SEQ ID NO: 824 - RNA, 20 nt, synthetic construct
  misc_feature 1..20: note = source = /note="Description of Artificial Sequence: Synthetic oligonucleotide"
  source 1..20: mol_type = other RNA
gagtccgagcgagagaagaa

SEQ ID NO: 825 - RNA, 20 nt, synthetic construct
  misc_feature 1..20: note = source = /note="Description of Artificial Sequence: Synthetic oligonucleotide"
  source 1..20: mol_type = other RNA
gagtccggatagaagaagaa

SEQ ID NO: 826 - RNA, 20 nt, synthetic construct
  misc_feature 1..20: note = source = /note="Description of Artificial Sequence: Synthetic oligonucleotide"
  source 1..20: mol_type = other RNA
gagtctaagcagaagaagaa

SEQ ID NO: 827 - RNA, 20 nt, synthetic construct
  misc_feature 1..20: note = source = /note="Description of Artificial Sequence: Synthetic oligonucleotide"
  source 1..20: mol_type = other RNA
ggacccgagcagaagaagaa

SEQ ID NO: 828 - RNA, 20 nt, synthetic construct
  misc_feature 1..20: note = source = /note="Description of Artificial Sequence: Synthetic oligonucleotide"
  source 1..20: mol_type = other RNA
gagtccgagcagaagggagg

SEQ ID NO: 829 - RNA, 20 nt, synthetic construct
  misc_feature 1..20: note = source = /note="Description of Artificial Sequence: Synthetic oligonucleotide"
  source 1..20: mol_type = other RNA
gagtccgagcagggagggaa

SEQ ID NO: 830 - RNA, 20 nt, synthetic construct
  misc_feature 1..20: note = source = /note="Description of Artificial Sequence: Synthetic oligonucleotide"
  source 1..20: mol_type = other RNA
gagtccgagtgagggaagaa

SEQ ID NO: 831 - RNA, 20 nt, synthetic construct
  misc_feature 1..20: note = source = /note="Description of Artificial Sequence: Synthetic oligonucleotide"
  source 1..20: mol_type = other RNA
gagtccagatggaagaagaa

SEQ ID NO: 832 - RNA, 20 nt, synthetic construct
  misc_feature 1..20: note = source = /note="Description of Artificial Sequence: Synthetic oligonucleotide"
  source 1..20: mol_type = other RNA
gagcctaggcagaagaagaa

SEQ ID NO: 833 - RNA, 20 nt, synthetic construct
  misc_feature 1..20: note = source = /note="Description of Artificial Sequence: Synthetic oligonucleotide"
  source 1..20: mol_type = other RNA
gcgccaccggttgatgtgat

SEQ ID NO: 834 - RNA, 20 nt, synthetic construct
  misc_feature 1..20: note = source = /note="Description of Artificial Sequence: Synthetic oligonucleotide"
  source 1..20: mol_type = other RNA
gcgccaccggttgatgtggc

SEQ ID NO: 835 - RNA, 20 nt, synthetic construct
  misc_feature 1..20: note = source = /note="Description of Artificial Sequence: Synthetic oligonucleotide"
  source 1..20: mol_type = other RNA
gcgccaccggttgatgcaat

SEQ ID NO: 836 - RNA, 20 nt, synthetic construct
  misc_feature 1..20: note = source = /note="Description of Artificial Sequence: Synthetic oligonucleotide"
  source 1..20: mol_type = other RNA
gcgccaccggttgacatgat

SEQ ID NO: 837 - RNA, 20 nt, synthetic construct
  misc_feature 1..20: note = source = /note="Description of Artificial Sequence: Synthetic oligonucleotide"
  source 1..20: mol_type = other RNA
gcgccaccggttagtgtgat

SEQ ID NO: 838 - RNA, 20 nt, synthetic construct
  misc_feature 1..20: note = source = /note="Description of Artificial Sequence: Synthetic oligonucleotide"
  source 1..20: mol_type = other RNA
gcgccaccggccgatgtgat

SEQ ID NO: 839 - RNA, 20 nt, synthetic construct
  misc_feature 1..20: note = source = /note="Description of Artificial Sequence: Synthetic oligonucleotide"
  source 1..20: mol_type = other RNA
gcgccaccaattgatgtgat

SEQ ID NO: 840 - RNA, 20 nt, synthetic construct
  misc_feature 1..20: note = source = /note="Description of Artificial Sequence: Synthetic oligonucleotide"
  source 1..20: mol_type = other RNA
gcgccattggttgatgtgat

SEQ ID NO: 841 - RNA, 20 nt, synthetic construct
  misc_feature 1..20: note = source = /note="Description of Artificial Sequence: Synthetic oligonucleotide"
  source 1..20: mol_type = other RNA
gcgctgccggttgatgtgat

SEQ ID NO: 842 - RNA, 20 nt, synthetic construct
  misc_feature 1..20: note = source = /note="Description of Artificial Sequence: Synthetic oligonucleotide"
  source 1..20: mol_type = other RNA
gcatcaccggttgatgtgat

SEQ ID NO: 843 - RNA, 20 nt, synthetic construct
  misc_feature 1..20: note = source = /note="Description of Artificial Sequence: Synthetic oligonucleotide"
  source 1..20: mol_type = other RNA
gcgccaccggttgatgcagt

SEQ ID NO: 844 - RNA, 20 nt, synthetic construct
  misc_feature 1..20: note = source = /note="Description of Artificial Sequence: Synthetic oligonucleotide"
  source 1..20: mol_type = other RNA
gcgccaccggttggcatgat

SEQ ID NO: 845 - RNA, 20 nt, synthetic construct
  misc_feature 1..20: note = source = /note="Description of Artificial Sequence: Synthetic oligonucleotide"
  source 1..20: mol_type = other RNA
gcgccaccggccaatgtgat

SEQ ID NO: 846 - RNA, 20 nt, synthetic construct
  misc_feature 1..20: note = source = /note="Description of Artificial Sequence: Synthetic oligonucleotide"
  source 1..20: mol_type = other RNA
gcgccactaattgatgtgat

SEQ ID NO: 847 - RNA, 20 nt, synthetic construct
  misc_feature 1..20: note = source = /note="Description of Artificial Sequence: Synthetic oligonucleotide"
  source 1..20: mol_type = other RNA
gcgctgtcggttgatgtgat

SEQ ID NO: 848 - RNA, 20 nt, synthetic construct
  misc_feature 1..20: note = source = /note="Description of Artificial Sequence: Synthetic oligonucleotide"
  source 1..20: mol_type = other RNA
gtatcaccggttgatgtgat

SEQ ID NO: 849 - RNA, 20 nt, synthetic construct
  misc_feature 1..20: note = source = /note="Description of Artificial Sequence: Synthetic oligonucleotide"
  source 1..20: mol_type = other RNA
gcgccaccggttgatacagc

SEQ ID NO: 850 - RNA, 20 nt, synthetic construct
  misc_feature 1..20: note = source = /note="Description of Artificial Sequence: Synthetic oligonucleotide"
  source 1..20: mol_type = other RNA
gcgccaccggttagcacgat

SEQ ID NO: 851 - RNA, 20 nt, synthetic construct
  misc_feature 1..20: note = source = /note="Description of Artificial Sequence: Synthetic oligonucleotide"
  source 1..20: mol_type = other RNA
gcgccaccgaccagtgtgat

SEQ ID NO: 852 - RNA, 20 nt, synthetic construct
  misc_feature 1..20: note = source = /note="Description of Artificial Sequence: Synthetic oligonucleotide"
  source 1..20: mol_type = other RNA
gcgccattaactgatgtgat

SEQ ID NO: 853 - RNA, 20 nt, synthetic construct
  misc_feature 1..20: note = source = /note="Description of Artificial Sequence: Synthetic oligonucleotide"
  source 1..20: mol_type = other RNA
gcgttgttggttgatgtgat

SEQ ID NO: 854 - RNA, 20 nt, synthetic construct
  misc_feature 1..20: note = source = /note="Description of Artificial Sequence: Synthetic oligonucleotide"
  source 1..20: mol_type = other RNA
gtcacctccaatgactaggg

SEQ ID NO: 855 - RNA, 20 nt, synthetic construct
  misc_feature 1..20: note = source = /note="Description of Artificial Sequence: Synthetic oligonucleotide"
  source 1..20: mol_type = other RNA
gtcacctccaatgactaaga

SEQ ID NO: 856 - RNA, 20 nt, synthetic construct
  misc_feature 1..20: note = source = /note="Description of Artificial Sequence: Synthetic oligonucleotide"
  source 1..20: mol_type = other RNA
gtcacctccaatgattagga

SEQ ID NO: 857 - RNA, 20 nt, synthetic construct
  misc_feature 1..20: note = source = /note="Description of Artificial Sequence: Synthetic oligonucleotide"
  source 1..20: mol_type = other RNA
gtcacctccagtgactagga

SEQ ID NO: 858 - RNA, 20 nt, synthetic construct
  misc_feature 1..20: note = source = /note="Description of Artificial Sequence: Synthetic oligonucleotide"
  source 1..20: mol_type = other RNA
gtcacttccaatgactagga

SEQ ID NO: 859 - RNA, 20 nt, synthetic construct
  misc_feature 1..20: note = source = /note="Description of Artificial Sequence: Synthetic oligonucleotide"
  source 1..20: mol_type = other RNA
atcacctccaatgactagga

SEQ ID NO: 860 - RNA, 20 nt, synthetic construct
  misc_feature 1..20: note = source = /note="Description of Artificial Sequence: Synthetic oligonucleotide"
  source 1..20: mol_type = other RNA
gtcacctccaatgaccaagg

SEQ ID NO: 861 - RNA, 20 nt, synthetic construct
  misc_feature 1..20: note = source = /note="Description of Artificial Sequence: Synthetic oligonucleotide"
  source 1..20: mol_type = other RNA
gtcacctccaataactaagg

SEQ ID NO: 862 - RNA, 20 nt, synthetic construct
  misc_feature 1..20: note = source = /note="Description of Artificial Sequence: Synthetic oligonucleotide"
  source 1..20: mol_type = other RNA
gtcacctctaatgactaagg

SEQ ID NO: 863 - RNA, 20 nt, synthetic construct
  misc_feature 1..20: note = source = /note="Description of Artificial Sequence: Synthetic oligonucleotide"
  source 1..20: mol_type = other RNA
gtcgcctccaatgactaagg

SEQ ID NO: 864 - RNA, 20 nt, synthetic construct
  misc_feature 1..20: note = source = /note="Description of Artificial Sequence: Synthetic oligonucleotide"
  source 1..20: mol_type = other RNA
gtcacctccaatggccaggg

SEQ ID NO: 865 - RNA, 20 nt, synthetic construct
  misc_feature 1..20: note = source = /note="Description of Artificial Sequence: Synthetic oligonucleotide"
  source 1..20: mol_type = other RNA
gtcacctccagtgaccaggg

SEQ ID NO: 866 - RNA, 20 nt, synthetic construct
  misc_feature 1..20: note = source = /note="Description of Artificial Sequence: Synthetic oligonucleotide"
  source 1..20: mol_type = other RNA
gtcacccccaatgaccaggg

SEQ ID NO: 867 - RNA, 20 nt, synthetic construct
  misc_feature 1..20: note = source = /note="Description of Artificial Sequence: Synthetic oligonucleotide"
  source 1..20: mol_type = other RNA
gccacctccaatgaccaggg

SEQ ID NO: 868 - RNA, 20 nt, synthetic construct
  misc_feature 1..20: note = source = /note="Description of Artificial Sequence: Synthetic oligonucleotide"
  source 1..20: mol_type = other RNA
gacatcgatgtcctccccat

SEQ ID NO: 869 - RNA, 20 nt, synthetic construct
  misc_feature 1..20: note = source = /note="Description of Artificial Sequence: Synthetic oligonucleotide"
  source 1..20: mol_type = other RNA
gacatcgatgtcctccctag

SEQ ID NO: 870 - RNA, 20 nt, synthetic construct
  misc_feature 1..20: note = source = /note="Description of Artificial Sequence: Synthetic oligonucleotide"
  source 1..20: mol_type = other RNA
gacatcgatgtccttcccag

SEQ ID NO: 871 - RNA, 20 nt, synthetic construct
  misc_feature 1..20: note = source = /note="Description of Artificial Sequence: Synthetic oligonucleotide"
  source 1..20: mol_type = other RNA
gacatcgatgccctccccag

SEQ ID NO: 872 - RNA, 20 nt, synthetic construct
  misc_feature 1..20: note = source = /note="Description of Artificial Sequence: Synthetic oligonucleotide"
  source 1..20: mol_type = other RNA
gacattgatgtcctccccag

SEQ ID NO: 873 - RNA, 20 nt, synthetic construct
  misc_feature 1..20: note = source = /note="Description of Artificial Sequence: Synthetic oligonucleotide"
  source 1..20: mol_type = other RNA
aacatcgatgtcctccccag

SEQ ID NO: 874 - RNA, 20 nt, synthetic construct
  misc_feature 1..20: note = source = /note="Description of Artificial Sequence: Synthetic oligonucleotide"
  source 1..20: mol_type = other RNA
gacatcgatgtcctctctat

SEQ ID NO: 875 - RNA, 20 nt, synthetic construct
  misc_feature 1..20: note = source = /note="Description of Artificial Sequence: Synthetic oligonucleotide"
  source 1..20: mol_type = other RNA
gacatcgatgtcttccctat

SEQ ID NO: 876 - RNA, 20 nt, synthetic construct
  misc_feature 1..20: note = source = /note="Description of Artificial Sequence: Synthetic oligonucleotide"
  source 1..20: mol_type = other RNA
gacatcgacgtcctccctat

SEQ ID NO: 877 - RNA, 20 nt, synthetic construct
  misc_feature 1..20: note = source = /note="Description of Artificial Sequence: Synthetic oligonucleotide"
  source 1..20: mol_type = other RNA
gacgtcgatgtcctccctat

SEQ ID NO: 878 - RNA, 20 nt, synthetic construct
  misc_feature 1..20: note = source = /note="Description of Artificial Sequence: Synthetic oligonucleotide"
  source 1..20: mol_type = other RNA
gacatcgatgtcccctccat

SEQ ID NO: 879 - RNA, 20 nt, synthetic construct
  misc_feature 1..20: note = source = /note="Description of Artificial Sequence: Synthetic oligonucleotide"
  source 1..20: mol_type = other RNA
gacatcgatgccctctccat

SEQ ID NO: 880 - RNA, 20 nt, synthetic construct
  misc_feature 1..20: note = source = /note="Description of Artificial Sequence: Synthetic oligonucleotide"
  source 1..20: mol_type = other RNA
gacatcaatgtcctctccat

SEQ ID NO: 881 - RNA, 20 nt, synthetic construct
  misc_feature 1..20: note = source = /note="Description of Artificial Sequence: Synthetic oligonucleotide"
  source 1..20: mol_type = other RNA
ggcatcgatgtcctctccat

SEQ ID NO: 882 - RNA, 20 nt, synthetic construct
  misc_feature 1..20: note = source = /note="Description of Artificial Sequence: Synthetic oligonucleotide"
  source 1..20: mol_type = other RNA
gagtccgagcagaagaagaa

SEQ ID NO: 883 - RNA, 20 nt, synthetic construct
  misc_feature 1..20: note = source = /note="Description of Artificial Sequence: Synthetic oligonucleotide"
  source 1..20: mol_type = other RNA
gagtccgagcagaagaaaag

SEQ ID NO: 884 - RNA, 20 nt, synthetic construct
  misc_feature 1..20: note = source = /note="Description of Artificial Sequence: Synthetic oligonucleotide"
  source 1..20: mol_type = other RNA
gagtccgagcagaaaaagag

SEQ ID NO: 885 - RNA, 20 nt, synthetic construct
  misc_feature 1..20: note = source = /note="Description of Artificial Sequence: Synthetic oligonucleotide"
  source 1..20: mol_type = other RNA
gagtccgagcggaagaagag

SEQ ID NO: 886 - RNA, 20 nt, synthetic construct
  misc_feature 1..20: note = source = /note="Description of Artificial Sequence: Synthetic oligonucleotide"
  source 1..20: mol_type = other RNA
gagtctgagcagaagaagag

SEQ ID NO: 887 - RNA, 20 nt, synthetic construct
  misc_feature 1..20: note = source = /note="Description of Artificial Sequence: Synthetic oligonucleotide"
  source 1..20: mol_type = other RNA
aagtccgagcagaagaagag

SEQ ID NO: 888 - RNA, 20 nt, synthetic construct
  misc_feature 1..20: note = source = /note="Description of Artificial Sequence: Synthetic oligonucleotide"
  source 1..20: mol_type = other RNA
gagtccgagcagaagcaaaa

SEQ ID NO: 889 - RNA, 20 nt, synthetic construct
  misc_feature 1..20: note = source = /note="Description of Artificial Sequence: Synthetic oligonucleotide"
  source 1..20: mol_type = other RNA
gagtccgagcaggagaaaaa

SEQ ID NO: 890 - RNA, 20 nt, synthetic construct
  misc_feature 1..20: note = source = /note="Description of Artificial Sequence: Synthetic oligonucleotide"
  source 1..20: mol_type = other RNA
gagtccgaacagaagaaaaa

SEQ ID NO: 891 - RNA, 20 nt, synthetic construct
  misc_feature 1..20: note = source = /note="Description of Artificial Sequence: Synthetic oligonucleotide"
  source 1..20: mol_type = other RNA
gagcccgagcagaagaaaaa

SEQ ID NO: 892 - RNA, 20 nt, synthetic construct
  misc_feature 1..20: note = source = /note="Description of Artificial Sequence: Synthetic oligonucleotide"
  source 1..20: mol_type = other RNA
gagtccgagcagagggagaa

SEQ ID NO: 893 - RNA, 20 nt, synthetic construct
  misc_feature 1..20: note = source = /note="Description of Artificial Sequence: Synthetic oligonucleotide"
  source 1..20: mol_type = other RNA
gagtccgagcggaaggagaa

SEQ ID NO: 894 - RNA, 20 nt, synthetic construct
  misc_feature 1..20: note = source = /note="Description of Artificial Sequence: Synthetic oligonucleotide"
  source 1..20: mol_type = other RNA
gagtccaagcagaaggagaa

SEQ ID NO: 895 - RNA, 20 nt, synthetic construct
  misc_feature 1..20: note = source = /note="Description of Artificial Sequence: Synthetic oligonucleotide"
  source 1..20: mol_type = other RNA
gggtccgagcagaaggagaa

SEQ ID NO: 896 - RNA, 20 nt, synthetic construct
  misc_feature 1..20: note = source = /note="Description of Artificial Sequence: Synthetic oligonucleotide"
  source 1..20: mol_type = other RNA
gcgccaccggttgatgtgat

SEQ ID NO: 897 - RNA, 20 nt, synthetic construct
  misc_feature 1..20: note = source = /note="Description of Artificial Sequence: Synthetic oligonucleotide"
  source 1..20: mol_type = other RNA
gcgccaccggttgatgtaac

SEQ ID NO: 898 - RNA, 20 nt, synthetic construct
  misc_feature 1..20: note = source = /note="Description of Artificial Sequence: Synthetic oligonucleotide"
  source 1..20: mol_type = other RNA
gcgccaccggttgatgtgac

SEQ ID NO: 899 - RNA, 20 nt, synthetic construct
  misc_feature 1..20: note = source = /note="Description of Artificial Sequence: Synthetic oligonucleotide"
  source 1..20: mol_type = other RNA
gcgccaccggctgatgtgac

SEQ ID NO: 900 - RNA, 20 nt, synthetic construct
  misc_feature 1..20: note = source = /note="Description of Artificial Sequence: Synthetic oligonucleotide"
  source 1..20: mol_type = other RNA
gcgccgccggttgatgtgac

SEQ ID NO: 901 - RNA, 20 nt, synthetic construct
  misc_feature 1..20: note = source = /note="Description of Artificial Sequence: Synthetic oligonucleotide"
  source 1..20: mol_type = other RNA
acgccaccggttgatgtgac

SEQ ID NO: 902 - RNA, 20 nt, synthetic construct
  misc_feature 1..20: note = source = /note="Description of Artificial Sequence: Synthetic oligonucleotide"
  source 1..20: mol_type = other RNA
gcgccaccggttgatataat

SEQ ID NO: 903 - RNA, 20 nt, synthetic construct
  misc_feature 1..20: note = source = /note="Description of Artificial Sequence: Synthetic oligonucleotide"
  source 1..20: mol_type = other RNA
gcgccaccggttaatgtaat

SEQ ID NO: 904 - RNA, 20 nt, synthetic construct
  misc_feature 1..20: note = source = /note="Description of Artificial Sequence: Synthetic oligonucleotide"
  source 1..20: mol_type = other RNA
gcgccaccagttgatgtaat

SEQ ID NO: 905 - RNA, 20 nt, synthetic construct
  misc_feature 1..20: note = source = /note="Description of Artificial Sequence: Synthetic oligonucleotide"
  source 1..20: mol_type = other RNA
gcgtcaccggttgatgtaat

SEQ ID NO: 906 - RNA, 20 nt, synthetic construct
  misc_feature 1..20: note = source = /note="Description of Artificial Sequence: Synthetic oligonucleotide"
  source 1..20: mol_type = other RNA
gcgccaccggttggtatgat

SEQ ID NO: 907 - RNA, 20 nt, synthetic construct
  misc_feature 1..20: note = source = /note="Description of Artificial Sequence: Synthetic oligonucleotide"
  source 1..20: mol_type = other RNA
gcgccaccggctgatatgat

SEQ ID NO: 908 - RNA, 20 nt, synthetic construct
  misc_feature 1..20: note = source = /note="Description of Artificial Sequence: Synthetic oligonucleotide"
  source 1..20: mol_type = other RNA
gcgccatcggttgatatgat

SEQ ID NO: 909 - RNA, 20 nt, synthetic construct
  misc_feature 1..20: note = source = /note="Description of Artificial Sequence: Synthetic oligonucleotide"
  source 1..20: mol_type = other RNA
gtgccaccggttgatatgat

SEQ ID NO: 910 - RNA, 20 nt, synthetic construct
  misc_feature 1..20: note = source = /note="Description of Artificial Sequence: Synthetic oligonucleotide"
  source 1..20: mol_type = other RNA
gtcacctccaatgactaggg

SEQ ID NO: 911 - RNA, 20 nt, synthetic construct
  misc_feature 1..20: note = source = /note="Description of Artificial Sequence: Synthetic oligonucleotide"
  source 1..20: mol_type = other RNA
gtcacctccaatgaccaaga

SEQ ID NO: 912 - RNA, 20 nt, synthetic construct
  misc_feature 1..20: note = source = /note="Description of Artificial Sequence: Synthetic oligonucleotide"
  source 1..20: mol_type = other RNA
gtcacctccaatggctggga

SEQ ID NO: 913 - RNA, 20 nt, synthetic construct
  misc_feature 1..20: note = source = /note="Description of Artificial Sequence: Synthetic oligonucleotide"
  source 1..20: mol_type = other RNA
gtcacctccaacgaccagga

SEQ ID NO: 914 - RNA, 20 nt, synthetic construct
  misc_feature 1..20: note = source = /note="Description of Artificial Sequence: Synthetic oligonucleotide"
  source 1..20: mol_type = other RNA
gtcacctccgatgattagga

SEQ ID NO: 915 - RNA, 20 nt, synthetic construct
  misc_feature 1..20: note = source = /note="Description of Artificial Sequence: Synthetic oligonucleotide"
  source 1..20: mol_type = other RNA
gtcacctccaatggccaagg

SEQ ID NO: 916 - RNA, 20 nt, synthetic construct
  misc_feature 1..20: note = source = /note="Description of Artificial Sequence: Synthetic oligonucleotide"
  source 1..20: mol_type = other RNA
gtcacctccaacgattaagg

SEQ ID NO: 917 - RNA, 20 nt, synthetic construct
  misc_feature 1..20: note = source = /note="Description of Artificial Sequence: Synthetic oligonucleotide"
  source 1..20: mol_type = other RNA
gtcacctccgatggctaagg

SEQ ID NO: 918 - RNA, 20 nt, synthetic construct
  misc_feature 1..20: note = source = /note="Description of Artificial Sequence: Synthetic oligonucleotide"
  source 1..20: mol_type = other RNA
gtcaccttcaataactaagg

SEQ ID NO: 919 - RNA, 20 nt, synthetic construct
  misc_feature 1..20: note = source = /note="Description of Artificial Sequence: Synthetic oligonucleotide"
  source 1..20: mol_type = other RNA
gtcacctccaatggccaaga

SEQ ID NO: 920 - RNA, 20 nt, synthetic construct
  misc_feature 1..20: note = source = /note="Description of Artificial Sequence: Synthetic oligonucleotide"
  source 1..20: mol_type = other RNA
gtcacctccagtggctggga

SEQ ID NO: 921 - RNA, 20 nt, synthetic construct
  misc_feature 1..20: note = source = /note="Description of Artificial Sequence: Synthetic oligonucleotide"
  source 1..20: mol_type = other RNA
gtcaccttcaacgaccagga

SEQ ID NO: 922 - RNA, 20 nt, synthetic construct
  misc_feature 1..20: note = source = /note="Description of Artificial Sequence: Synthetic oligonucleotide"
  source 1..20: mol_type = other RNA
gtcatctccgatgattagga

SEQ ID NO: 923 - RNA, 20 nt, synthetic construct
  misc_feature 1..20: note = source = /note="Description of Artificial Sequence: Synthetic oligonucleotide"
  source 1..20: mol_type = other RNA
gccaccttcaatggctagga

SEQ ID NO: 924 - RNA, 20 nt, synthetic construct
  misc_feature 1..20: note = source = /note="Description of Artificial Sequence: Synthetic oligonucleotide"
  source 1..20: mol_type = other RNA
gacatcgatgtcctccccat

SEQ ID NO: 925 - RNA, 20 nt, synthetic construct
  misc_feature 1..20: note = source = /note="Description of Artificial Sequence: Synthetic oligonucleotide"
  source 1..20: mol_type = other RNA
gacatcgatgtcctctctag

SEQ ID NO: 926 - RNA, 20 nt, synthetic construct
  misc_feature 1..20: note = source = /note="Description of Artificial Sequence: Synthetic oligonucleotide"
  source 1..20: mol_type = other RNA
gacatcgatgtccccctcag

SEQ ID NO: 927 - RNA, 20 nt, synthetic construct
  misc_feature 1..20: note = source = /note="Description of Artificial Sequence: Synthetic oligonucleotide"
  source 1..20: mol_type = other RNA
gacatcgatgttctctccag

SEQ ID NO: 928 - RNA, 20 nt, synthetic construct
  misc_feature 1..20: note = source = /note="Description of Artificial Sequence: Synthetic oligonucleotide"
  source 1..20: mol_type = other RNA
gacatcgatatccttcccag

SEQ ID NO: 929 - RNA, 20 nt, synthetic construct
  misc_feature 1..20: note = source = /note="Description of Artificial Sequence: Synthetic oligonucleotide"
  source 1..20: mol_type = other RNA
gacatcgatgtcccctctat

SEQ ID NO: 930 - RNA, 20 nt, synthetic construct
  misc_feature 1..20: note = source = /note="Description of Artificial Sequence: Synthetic oligonucleotide"
  source 1..20: mol_type = other RNA
gacatcgatgttcttcctat

SEQ ID NO: 931 - RNA, 20 nt, synthetic construct
  misc_feature 1..20: note = source = /note="Description of Artificial Sequence: Synthetic oligonucleotide"
  source 1..20: mol_type = other RNA
gacatcgatatcccccctat

SEQ ID NO: 932 - RNA, 20 nt, synthetic construct
  misc_feature 1..20: note = source = /note="Description of Artificial Sequence: Synthetic oligonucleotide"
  source 1..20: mol_type = other RNA
gacatcggtgtcatccctat

SEQ ID NO: 933 - RNA, 20 nt, synthetic construct
  misc_feature 1..20: note = source = /note="Description of Artificial Sequence: Synthetic oligonucleotide"
  source 1..20: mol_type = other RNA
gacatcgatgtcccctctag

SEQ ID NO: 934 - RNA, 20 nt, synthetic construct
  misc_feature 1..20: note = source = /note="Description of Artificial Sequence: Synthetic oligonucleotide"
  source 1..20: mol_type = other RNA
gacatcgatgcccccctcag

SEQ ID NO: 935 - RNA, 20 nt, synthetic construct
  misc_feature 1..20: note = source = /note="Description of Artificial Sequence: Synthetic oligonucleotide"
  source 1..20: mol_type = other RNA
gacatcggtgttctctccag

SEQ ID NO: 936 - RNA, 20 nt, synthetic construct
  misc_feature 1..20: note = source = /note="Description of Artificial Sequence: Synthetic oligonucleotide"
  source 1..20: mol_type = other RNA
gacaccgatatccttcccag

SEQ ID NO: 937 - RNA, 20 nt, synthetic construct
  misc_feature 1..20: note = source = /note="Description of Artificial Sequence: Synthetic oligonucleotide"
  source 1..20: mol_type = other RNA
ggcatcggtgtcccccccag

SEQ ID NO: 938 - RNA, 20 nt, synthetic construct
  misc_feature 1..20: note = source = /note="Description of Artificial Sequence: Synthetic oligonucleotide"
  source 1..20: mol_type = other RNA
gagtccgagcagaagaagaa

SEQ ID NO: 939 - RNA, 20 nt, synthetic construct
  misc_feature 1..20: note = source = /note="Description of Artificial Sequence: Synthetic oligonucleotide"
  source 1..20: mol_type = other RNA
gagtccgagcagaaggaaag

SEQ ID NO: 940 - RNA, 20 nt, synthetic construct
  misc_feature 1..20: note = source = /note="Description of Artificial Sequence: Synthetic oligonucleotide"
  source 1..20: mol_type = other RNA
gagtccgagcagaggaggag

SEQ ID NO: 941 - RNA, 20 nt, synthetic construct
  misc_feature 1..20: note = source = /note="Description of Artificial Sequence: Synthetic oligonucleotide"
  source 1..20: mol_type = other RNA
gagtccgagcaaaaggagag

SEQ ID NO: 942 - RNA, 20 nt, synthetic construct
  misc_feature 1..20: note = source = /note="Description of Artificial Sequence: Synthetic oligonucleotide"
  source 1..20: mol_type = other RNA
gagtccgagtagaaaaagag

SEQ ID NO: 943 - RNA, 20 nt, synthetic construct
  misc_feature 1..20: note = source = /note="Description of Artificial Sequence: Synthetic oligonucleotide"
  source 1..20: mol_type = other RNA
gagtccgagcagagggaaaa

SEQ ID NO: 944 - RNA, 20 nt, synthetic construct
  misc_feature 1..20: note = source = /note="Description of Artificial Sequence: Synthetic oligonucleotide"
  source 1..20: mol_type = other RNA
gagtccgagcaaaaaaaaaa

SEQ ID NO: 945 - RNA, 20 nt, synthetic construct
  misc_feature 1..20: note = source = /note="Description of Artificial Sequence: Synthetic oligonucleotide"
  source 1..20: mol_type = other RNA
gagtccgagtagaggaaaaa

SEQ ID NO: 946 - RNA, 20 nt, synthetic construct
  misc_feature 1..20: note = source = /note="Description of Artificial Sequence: Synthetic oligonucleotide"
  source 1..20: mol_type = other RNA
gagtccgggcaggagaaaaa

SEQ ID NO: 947 - RNA, 20 nt, synthetic construct
  misc_feature 1..20: note = source = /note="Description of Artificial Sequence: Synthetic oligonucleotide"
  source 1..20: mol_type = other RNA
gagtccgagcagagggaaag

SEQ ID NO: 948 - RNA, 20 nt, synthetic construct
  misc_feature 1..20: note = source = /note="Description of Artificial Sequence: Synthetic oligonucleotide"
  source 1..20: mol_type = other RNA
gagtccgagcggaggaggag

SEQ ID NO: 949 - RNA, 20 nt, synthetic construct
  misc_feature 1..20: note = source = /note="Description of Artificial Sequence: Synthetic oligonucleotide"
  source 1..20: mol_type = other RNA
gagtccgggcaaaaggagag

SEQ ID NO: 950 - RNA, 20 nt, synthetic construct
  misc_feature 1..20: note = source = /note="Description of Artificial Sequence: Synthetic oligonucleotide"
  source 1..20: mol_type = other RNA
gagttcgagtagaaaaagag

SEQ ID NO: 951 - RNA, 20 nt, synthetic construct
  misc_feature 1..20: note = source = /note="Description of Artificial Sequence: Synthetic oligonucleotide"
  source 1..20: mol_type = other RNA
gggtccgggcagaggaagag

SEQ ID NO: 952 - RNA, 20 nt, synthetic construct
  misc_feature 1..20: note = source = /note="Description of Artificial Sequence: Synthetic oligonucleotide"
  source 1..20: mol_type = other RNA
gcgccaccggttgatgtgat

SEQ ID NO: 953 - RNA, 20 nt, synthetic construct
  misc_feature 1..20: note = source = /note="Description of Artificial Sequence: Synthetic oligonucleotide"
  source 1..20: mol_type = other RNA
gcgccaccggttgatataac

SEQ ID NO: 954 - RNA, 20 nt, synthetic construct
  misc_feature 1..20: note = source = /note="Description of Artificial Sequence: Synthetic oligonucleotide"
  source 1..20: mol_type = other RNA
gcgccaccggttggtgcgac

SEQ ID NO: 955 - RNA, 20 nt, synthetic construct
  misc_feature 1..20: note = source = /note="Description of Artificial Sequence: Synthetic oligonucleotide"
  source 1..20: mol_type = other RNA
gcgccaccggtcgatatgac

SEQ ID NO: 956 - RNA, 20 nt, synthetic construct
  misc_feature 1..20: note = source = /note="Description of Artificial Sequence: Synthetic oligonucleotide"
  source 1..20: mol_type = other RNA
gcgccaccgattgacgtgac

SEQ ID NO: 957 - RNA, 20 nt, synthetic construct
  misc_feature 1..20: note = source = /note="Description of Artificial Sequence: Synthetic oligonucleotide"
  source 1..20: mol_type = other RNA
gcgccaccggttggtataat

SEQ ID NO: 958 - RNA, 20 nt, synthetic construct
  misc_feature 1..20: note = source = /note="Description of Artificial Sequence: Synthetic oligonucleotide"
  source 1..20: mol_type = other RNA
gcgccaccggtcgacgtaat

SEQ ID NO: 959 - RNA, 20 nt, synthetic construct
  misc_feature 1..20: note = source = /note="Description of Artificial Sequence: Synthetic oligonucleotide"
  source 1..20: mol_type = other RNA
gcgccaccgattggtgtaat

SEQ ID NO: 960 - RNA, 20 nt, synthetic construct
  misc_feature 1..20: note = source = /note="Description of Artificial Sequence: Synthetic oligonucleotide"
  source 1..20: mol_type = other RNA
gcgccactggttaatgtaat

SEQ ID NO: 961 - RNA, 20 nt, synthetic construct
  misc_feature 1..20: note = source = /note="Description of Artificial Sequence: Synthetic oligonucleotide"
  source 1..20: mol_type = other RNA
gcgccaccggttggtataac

SEQ ID NO: 962 - RNA, 20 nt, synthetic construct
  misc_feature 1..20: note = source = /note="Description of Artificial Sequence: Synthetic oligonucleotide"
  source 1..20: mol_type = other RNA
gcgccaccggctggtgcgac

SEQ ID NO: 963 - RNA, 20 nt, synthetic construct
  misc_feature 1..20: note = source = /note="Description of Artificial Sequence: Synthetic oligonucleotide"
  source 1..20: mol_type = other RNA
gcgccactggtcgatatgac

SEQ ID NO: 964 - RNA, 20 nt, synthetic construct
  misc_feature 1..20: note = source = /note="Description of Artificial Sequence: Synthetic oligonucleotide"
  source 1..20: mol_type = other RNA
gcgctaccgattgacgtgac

SEQ ID NO: 965 - RNA, 20 nt, synthetic construct
  misc_feature 1..20: note = source = /note="Description of Artificial Sequence: Synthetic oligonucleotide"
  source 1..20: mol_type = other RNA
gtgccactggttggtgtgac

SEQ ID NO: 966 - RNA, 20 nt, synthetic construct
  misc_feature 1..20: note = source = /note="Description of Artificial Sequence: Synthetic oligonucleotide"
  source 1..20: mol_type = other RNA
gtcacctccaatgactaggg

SEQ ID NO: 967 - DNA, 23 bp, synthetic construct
  misc_feature 1..23: note = source = /note="Description of Artificial Sequence: Synthetic oligonucleotide"
  misc_feature 1..23: note = source = /note="Description of Combined DNA/RNA Molecule: Synthetic oligonucleotide"
  source 1..23: mol_type = other DNA
  modified_base 2: mod_base = OTHER; note = uracil
  modified_base 7: mod_base = OTHER; note = uracil
  modified_base 11: mod_base = OTHER; note = uracil
  modified_base 15: mod_base = OTHER; note = uracil
gtcacctccaatgactagggtgg

SEQ ID NO: 968 - DNA, 23 bp, synthetic construct
  misc_feature 1..23: note = source = /note="Description of Artificial Sequence: Synthetic oligonucleotide"
  misc_feature 1..23: note = source = /note="Description of Combined DNA/RNA Molecule: Synthetic oligonucleotide"
  source 1..23: mol_type = other DNA
  modified_base 2: mod_base = OTHER; note = uracil
  modified_base 7: mod_base = OTHER; note = uracil
  modified_base 12: mod_base = OTHER; note = uracil
  modified_base 16: mod_base = OTHER; note = uracil
gtcaactccaatgattaggacag

SEQ ID NO: 969 - DNA, 23 bp, synthetic construct
  misc_feature 1..23: note = source = /note="Description of Artificial Sequence: Synthetic oligonucleotide"
  misc_feature 1..23: note = source = /note="Description of Combined DNA/RNA Molecule: Synthetic oligonucleotide"
  source 1..23: mol_type = other DNA
  modified_base 2: mod_base = OTHER; note = uracil
  modified_base 7: mod_base = OTHER; note = uracil
  modified_base 12: mod_base = OTHER; note = uracil
  modified_base 16: mod_base = OTHER; note = uracil
gtcacctccacttcctagggcag

SEQ ID NO: 970 - DNA, 23 bp, synthetic construct
  misc_feature 1..23: note = source = /note="Description of Artificial Sequence: Synthetic oligonucleotide"
  misc_feature 1..23: note = source = /note="Description of Combined DNA/RNA Molecule: Synthetic oligonucleotide"
  source 1..23: mol_type = other DNA
  modified_base 2: mod_base = OTHER; note = uracil
  modified_base 7: mod_base = OTHER; note = uracil
  modified_base 16: mod_base = OTHER; note = uracil
gtcacttccaaggactagagaag

SEQ ID NO: 971 - DNA, 23 bp, synthetic construct
  misc_feature 1..23: note = source = /note="Description of Artificial Sequence: Synthetic oligonucleotide"
  misc_feature 1..23: note = source = /note="Description of Combined DNA/RNA Molecule: Synthetic oligonucleotide"
  source 1..23: mol_type = other DNA
  modified_base 2: mod_base = OTHER; note = uracil
  modified_base 7: mod_base = OTHER; note = uracil
  modified_base 16: mod_base = OTHER; note = uracil
gtcacctccagggtctagggcag

SEQ ID NO: 972 - DNA, 23 bp, synthetic construct
  misc_feature 1..23: note = source = /note="Description of Artificial Sequence: Synthetic oligonucleotide"
  misc_feature 1..23: note = source = /note="Description of Combined DNA/RNA Molecule: Synthetic oligonucleotide"
  source 1..23: mol_type = other DNA
  modified_base 2: mod_base = OTHER; note = uracil
  modified_base 7: mod_base = OTHER; note = uracil
  modified_base 12: mod_base = OTHER; note = uracil
  modified_base 16: mod_base = OTHER; note = uracil
gtcaactccaatgacttgggagg

SEQ ID NO: 973 - DNA, 23 bp, synthetic construct
  misc_feature 1..23: note = source = /note="Description of Artificial Sequence: Synthetic oligonucleotide"
  misc_feature 1..23: note = source = /note="Description of Combined DNA/RNA Molecule: Synthetic oligonucleotide"
  source 1..23: mol_type = other DNA
  modified_base 2: mod_base = OTHER; note = uracil
  modified_base 7: mod_base = OTHER; note = uracil
  modified_base 12: mod_base = OTHER; note = uracil
  modified_base 16: mod_base = OTHER; note = uracil
gtcaccttaaatgacttgggaag

SEQ ID NO: 974 - DNA, 23 bp, synthetic construct
  misc_feature 1..23: note = source = /note="Description of Artificial Sequence: Synthetic oligonucleotide"
  misc_feature 1..23: note = source = /note="Description of Combined DNA/RNA Molecule: Synthetic oligonucleotide"
  source 1..23: mol_type = other DNA
  modified_base 2: mod_base = OTHER; note = uracil
  modified_base 7: mod_base = OTHER; note = uracil
  modified_base 16: mod_base = OTHER; note = uracil
ttcacctccaaaaactagggaag

SEQ ID NO: 975 - DNA, 23 bp, synthetic construct
  misc_feature 1..23: note = source = /note="Description of Artificial Sequence: Synthetic oligonucleotide"
  misc_feature 1..23: note = source = /note="Description of Combined DNA/RNA Molecule: Synthetic oligonucleotide"
  source 1..23: mol_type = other DNA
  modified_base 7: mod_base = OTHER; note = uracil
  modified_base 12: mod_base = OTHER; note = uracil
  modified_base 16: mod_base = OTHER; note = uracil
gctacctccagtgactagggaag

SEQ ID NO: 976 - DNA, 12 bp, Homo sapiens
  source 1..12: mol_type = unassigned DNA
tgactagggtgg

SEQ ID NO: 977 - DNA, 11 bp, Homo sapiens
  source 1..11: mol_type = unassigned DNA
tgactgggtgg

SEQ ID NO: 978 - DNA, 14 bp, Homo sapiens
  source 1..14: mol_type = unassigned DNA
tgactatagggtgg

SEQ ID NO: 979 - DNA, 12 bp, Homo sapiens
  source 1..12: mol_type = unassigned DNA
tgactagggaag

SEQ ID NO: 980 - DNA, 11 bp, Homo sapiens
  source 1..11: mol_type = unassigned DNA
tgactgggaag

SEQ ID NO: 981 - DNA, 14 bp, Homo sapiens
  source 1..14: mol_type = unassigned DNA
tgactatagggaag

SEQ ID NO: 982 - DNA, 14 bp, Homo sapiens
  source 1..14: mol_type = unassigned DNA
tgactggagggaag

SEQ ID NO: 983 - DNA, 13 bp, Homo sapiens
  source 1..13: mol_type = unassigned DNA
tgactacgggaag

SEQ ID NO: 984 - RNA, 20 nt, synthetic construct
  misc_feature 1..20: note = source = /note="Description of Artificial Sequence: Synthetic oligonucleotide"
  source 1..20: mol_type = other RNA
gagtccgagcagaagaagaa

SEQ ID NO: 985 - RNA, 23 nt, synthetic construct
  misc_feature 1..23: note = source = /note="Description of Artificial Sequence: Synthetic oligonucleotide"
  source 1..23: mol_type = other RNA
gagtccgagcagaagaagaaggg

SEQ ID NO: 986 - RNA, 23 nt, synthetic construct
  misc_feature 1..23: note = source = /note="Description of Artificial Sequence: Synthetic oligonucleotide"
  source 1..23: mol_type = other RNA
gaggccgagcagaagaaagacgg

SEQ ID NO: 987 - RNA, 23 nt, synthetic construct
  misc_feature 1..23: note = source = /note="Description of Artificial Sequence: Synthetic oligonucleotide"
  source 1..23: mol_type = other RNA
gagtcccagcagaggaagcagag

SEQ ID NO: 988 - DNA, 23 bp, synthetic construct
  misc_feature 1..23: note = source = /note="Description of Artificial Sequence: Synthetic oligonucleotide"
  misc_feature 1..23: note = source = /note="Description of Combined DNA/RNA Molecule: Synthetic oligonucleotide"
  source 1..23: mol_type = other DNA
  modified_base 4: mod_base = OTHER; note = uracil
gagtccaagcagaggaaggatag

SEQ ID NO: 989 - DNA, 23 bp, synthetic construct
  misc_feature 1..23: note = source = /note="Description of Artificial Sequence: Synthetic oligonucleotide"
  misc_feature 1..23: note = source = /note="Description of Combined DNA/RNA Molecule: Synthetic oligonucleotide"
  source 1..23: mol_type = other DNA
  modified_base 4: mod_base = OTHER; note = uracil
gagtcagagcagaactagaaggg

SEQ ID NO: 990 - RNA, 23 nt, synthetic construct
  misc_feature 1..23: note = source = /note="Description of Artificial Sequence: Synthetic oligonucleotide"
  source 1..23: mol_type = other RNA
gagtcccaggagaagaagagagg

SEQ ID NO: 991 - DNA, 23 bp, synthetic construct
  misc_feature 1..23: note = source = /note="Description of Artificial Sequence: Synthetic oligonucleotide"
  misc_feature 1..23: note = source = /note="Description of Combined DNA/RNA Molecule: Synthetic oligonucleotide"
  source 1..23: mol_type = other DNA
  modified_base 4: mod_base = OTHER; note = uracil
gagtccaagcagtagaggaaggg

SEQ ID NO: 992 - DNA, 23 bp, synthetic construct
  misc_feature 1..23: note = source = /note="Description of Artificial Sequence: Synthetic oligonucleotide"
  misc_feature 1..23: note = source = /note="Description of Combined DNA/RNA Molecule: Synthetic oligonucleotide"
  source 1..23: mol_type = other DNA
  modified_base 4: mod_base = OTHER; note = uracil
gagtccgagaaaatgaagaagag

SEQ ID NO: 993 - RNA, 23 nt, synthetic construct
  misc_feature 1..23: note = source = /note="Description of Artificial Sequence: Synthetic oligonucleotide"
  source 1..23: mol_type = other RNA
gagtcccagaagaagaaaaaaag

SEQ ID NO: 994 - RNA, 23 nt, synthetic construct
  misc_feature 1..23: note = source = /note="Description of Artificial Sequence: Synthetic oligonucleotide"
  source 1..23: mol_type = other RNA
gagtcccaggagaagaaaaacag

SEQ ID NO: 995 - RNA, 23 nt, synthetic construct
  misc_feature 1..23: note = source = /note="Description of Artificial Sequence: Synthetic oligonucleotide"
  source 1..23: mol_type = other RNA
gagtcagaacagaagaacaacag

SEQ ID NO: 996 - DNA, 23 bp, synthetic construct
  misc_feature 1..23: note = source = /note="Description of Artificial Sequence: Synthetic oligonucleotide"
  misc_feature 1..23: note = source = /note="Description of Combined DNA/RNA Molecule: Synthetic oligonucleotide"
  source 1..23: mol_type = other DNA
  modified_base 4: mod_base = OTHER; note = uracil
gagtccaagaagaataagaatag

SEQ ID NO: 997 - RNA, 23 nt, synthetic construct
  misc_feature 1..23: note = source = /note="Description of Artificial Sequence: Synthetic oligonucleotide"
  source 1..23: mol_type = other RNA
gaatccaagcagaagaagagaag

SEQ ID NO: 998 - RNA, 23 nt, synthetic construct
  misc_feature 1..23: note = source = /note="Description of Artificial Sequence: Synthetic oligonucleotide"
  source 1..23: mol_type = other RNA
gagtcagaccaggagaagaagag

SEQ ID NO: 999 - RNA, 23 nt, synthetic construct
  misc_feature 1..23: note = source = /note="Description of Artificial Sequence: Synthetic oligonucleotide"
  source 1..23: mol_type = other RNA
aagtccgagaagaagcagaaaag

SEQ ID NO: 1000 - DNA, 23 bp, synthetic construct
  misc_feature 1..23: note = source = /note="Description of Artificial Sequence: Synthetic oligonucleotide"
  misc_feature 1..23: note = source = /note="Description of Combined DNA/RNA Molecule: Synthetic oligonucleotide"
  source 1..23: mol_type = other DNA
  modified_base 4: mod_base = OTHER; note = uracil
gagtctgggcaggagaagaagag

SEQ ID NO: 1001 - DNA, 23 bp, synthetic construct
  misc_feature 1..23: note = source = /note="Description of Artificial Sequence: Synthetic oligonucleotide"
  misc_feature 1..23: note = source = /note="Description of Combined DNA/RNA Molecule: Synthetic oligonucleotide"
  source 1..23: mol_type = other DNA
  modified_base 4: mod_base = OTHER; note = uracil
gagtctgaacggaagaagaaaag

SEQ ID NO: 1002 - DNA, 23 bp, synthetic construct
  misc_feature 1..23: note = source = /note="Description of Artificial Sequence: Synthetic oligonucleotide"
  misc_feature 1..23: note = source = /note="Description of Combined DNA/RNA Molecule: Synthetic oligonucleotide"
  source 1..23: mol_type = other DNA
  modified_base 4: mod_base = OTHER; note = uracil
aagtctgagcagaagaagcacag

SEQ ID NO: 1003 - RNA, 23 nt, synthetic construct
  misc_feature 1..23: note = source = /note="Description of Artificial Sequence: Synthetic oligonucleotide"
  source 1..23: mol_type = other RNA
aagtccgaggagaggaagaaagg

SEQ ID NO: 1004 - RNA, 23 nt, synthetic construct
  misc_feature 1..23: note = source = /note="Description of Artificial Sequence: Synthetic oligonucleotide"
  source 1..23: mol_type = other RNA
gaggcccagcagaggaagaagag

SEQ ID NO: 1005 - DNA, 23 bp, synthetic construct
  misc_feature 1..23: note = source = /note="Description of Artificial Sequence: Synthetic oligonucleotide"
  misc_feature 1..23: note = source = /note="Description of Combined DNA/RNA Molecule: Synthetic oligonucleotide"
  source 1..23: mol_type = other DNA
  modified_base 4: mod_base = OTHER; note = uracil
gagttccagaagaagaagaagag

SEQ ID NO: 1006 - DNA, 23 bp, synthetic construct
  misc_feature 1..23: note = source = /note="Description of Artificial Sequence: Synthetic oligonucleotide"
  misc_feature 1..23: note = source = /note="Description of Combined DNA/RNA Molecule: Synthetic oligonucleotide"
  source 1..23: mol_type = other DNA
  modified_base 4: mod_base = OTHER; note = uracil
gagtactagaagaagaagaaaag

SEQ ID NO: 1007 - DNA, 23 bp, synthetic construct
  misc_feature 1..23: note = source = /note="Description of Artificial Sequence: Synthetic oligonucleotide"
  misc_feature 1..23: note = source = /note="Description of Combined DNA/RNA Molecule: Synthetic oligonucleotide"
  source 1..23: mol_type = other DNA
  modified_base 4: mod_base = OTHER; note = uracil
gactcctagcaaaagaagaatgg

SEQ ID NO: 1008 - DNA, 23 bp, synthetic construct
  misc_feature 1..23: note = source = /note="Description of Artificial Sequence: Synthetic oligonucleotide"
  misc_feature 1..23: note = source = /note="Description of Combined DNA/RNA Molecule: Synthetic oligonucleotide"
  source 1..23: mol_type = other DNA
  modified_base 4: mod_base = OTHER; note = uracil
gagtttgagtagaagaagaagag

SEQ ID NO: 1009 - RNA, 23 nt, synthetic construct
  misc_feature 1..23: note = source = /note="Description of Artificial Sequence: Synthetic oligonucleotide"
  source 1..23: mol_type = other RNA
gagtaagagaagaagaagaaggg

SEQ ID NO: 1010 - RNA, 23 nt, synthetic construct
  misc_feature 1..23: note = source = /note="Description of Artificial Sequence: Synthetic oligonucleotide"
  source 1..23: mol_type = other RNA
gagtaggaggagaagaagaaagg

SEQ ID NO: 1011 - DNA, 23 bp, synthetic construct
  misc_feature 1..23: note = source = /note="Description of Artificial Sequence: Synthetic oligonucleotide"
  misc_feature 1..23: note = source = /note="Description of Combined DNA/RNA Molecule: Synthetic oligonucleotide"
  source 1..23: mol_type = other DNA
  modified_base 4: mod_base = OTHER; note = uracil
gagtcctagcaggagaagaagag

SEQ ID NO: 1012 - DNA, 23 bp, synthetic construct
  misc_feature 1..23: note = source = /note="Description of Artificial Sequence: Synthetic oligonucleotide"
  misc_feature 1..23: note = source = /note="Description of Combined DNA/RNA Molecule: Synthetic oligonucleotide"
  source 1..23: mol_type = other DNA
  modified_base 4: mod_base = OTHER; note = uracil
gattcctaccagaagaagaatgg

SEQ ID NO: 1013 - RNA, 23 nt, synthetic construct
  misc_feature 1..23: note = source = /note="Description of Artificial Sequence: Synthetic oligonucleotide"
  source 1..23: mol_type = other RNA
gagtcccagcaaaagaagaaaag

SEQ ID NO: 1014 - RNA, 23 nt, synthetic construct
  misc_feature 1..23: note = source = /note="Description of Artificial Sequence: Synthetic oligonucleotide"
  source 1..23: mol_type = other RNA
gagagcaagcagaagaagaaggg

SEQ ID NO: 1015 - RNA, 23 nt, synthetic construct
  misc_feature 1..23: note = source = /note="Description of Artificial Sequence: Synthetic oligonucleotide"
  source 1..23: mol_type = other RNA
aagtcagaggagaagaagaaaag

SEQ ID NO: 1016 - DNA, 23 bp, synthetic construct
  misc_feature 1..23: note = source = /note="Description of Artificial Sequence: Synthetic oligonucleotide"
  misc_feature 1..23: note = source = /note="Description of Combined DNA/RNA Molecule: Synthetic oligonucleotide"
  source 1..23: mol_type = other DNA
  modified_base 4: mod_base = OTHER; note = uracil
gagtctaagcagaagaagaagag

SEQ ID NO: 1017 - DNA, 23 bp, synthetic construct
  misc_feature 1..23: note = source = /note="Description of Artificial Sequence: Synthetic oligonucleotide"
  misc_feature 1..23: note = source = /note="Description of Combined DNA/RNA Molecule: Synthetic oligonucleotide"
  source 1..23: mol_type = other DNA
  modified_base 4: mod_base = OTHER; note = uracil
acgtctgagcagaagaagaatgg

SEQ ID NO: 1018 - DNA, 12 bp, Homo sapiens
  source 1..12: mol_type = unassigned DNA
gaagaagaaggg

SEQ ID NO: 1019 - DNA, 13 bp, Homo sapiens
  source 1..13: mol_type = unassigned DNA
gaagaaggaaggg

SEQ ID NO: 1020 - DNA, 13 bp, Homo sapiens
  source 1..13: mol_type = unassigned DNA
gaagaaagaaggg

SEQ ID NO: 1021 - DNA, 15 bp, Homo sapiens
  source 1..15: mol_type = unassigned DNA
gaagaattagaaggg

SEQ ID NO: 1022 - DNA, 14 bp, Homo sapiens
  source 1..14: mol_type = unassigned DNA
gaagaacagaaggg

SEQ ID NO: 1023 - DNA, 11 bp, Homo sapiens
  source 1..11: mol_type = unassigned DNA
gaagagaaggg

SEQ ID NO: 1024 - DNA, 11 bp, Homo sapiens
  source 1..11: mol_type = unassigned DNA
gaagaaaaggg

SEQ ID NO: 1025 - DNA, 12 bp, Homo sapiens
  source 1..12: mol_type = unassigned DNA
gaagaaagacgg

SEQ ID NO: 1026 - DNA, 11 bp, Homo sapiens
  source 1..11: mol_type = unassigned DNA
gaagaagacgg

SEQ ID NO: 1027 - DNA, 13 bp, Homo sapiens
  source 1..13: mol_type = unassigned DNA
gaagaaaagacgg

SEQ ID NO: 1028 - DNA, 13 bp, Homo sapiens
  source 1..13: mol_type = unassigned DNA
gaagaatagacgg

SEQ ID NO: 1029 - DNA, 13 bp, Homo sapiens
  source 1..13: mol_type = unassigned DNA
gaagaacagacgg

SEQ ID NO: 1030 - DNA, 14 bp, Homo sapiens
  source 1..14: mol_type = unassigned DNA
gaagaataagacgg

SEQ ID NO: 1031 - DNA, 12 bp, Homo sapiens
  source 1..12: mol_type = unassigned DNA
ggagaagaagag

SEQ ID NO: 1032 - DNA, 13 bp, Homo sapiens
  source 1..13: mol_type = unassigned DNA
ggagaaagaagag

SEQ ID NO: 1033 - DNA, 11 bp, Homo sapiens
  source 1..11: mol_type = unassigned DNA
ggagagaagag

SEQ ID NO: 1034 - DNA, 11 bp, Homo sapiens
  source 1..11: mol_type = unassigned DNA
ggagaaaagag

SEQ ID NO: 1035 - DNA, 14 bp, Homo sapiens
  source 1..14: mol_type = unassigned DNA
ggagaatagaagag

SEQ ID NO: 1036 - DNA, 12 bp, Homo sapiens
  source 1..12: mol_type = unassigned DNA
gaagaagaagag

SEQ ID NO: 1037 - DNA, 13 bp, Homo sapiens
  source 1..13: mol_type = unassigned DNA
gaagaaagaagag

SEQ ID NO: 1038 - DNA, 11 bp, Homo sapiens
  source 1..11: mol_type = unassigned DNA
gaagagaagag

SEQ ID NO: 1039 - DNA, 11 bp, Homo sapiens
  source 1..11: mol_type = unassigned DNA
gaagaaaagag

SEQ ID NO: 1040 - DNA, 384 bp, Homo sapiens
  source 1..384: mol_type = unassigned DNA
cccagtggctgctctgggggcctcctgagtttctcatctgtgcccctccctccctggcccaggtgaaggtgtggttccagaaccggaggacaaagtacaaacggcagaagctggaggaggaagggcctgagtccgagcagaagaagaagggctcccatcacatcaaccggtggcgcattgccacgaagcaggccaatggggaggacatcgatgtcacctccaatgactagggtgggcaaccacaaacccacgagggggcagagtgctgcttgctgctggccaggcccctgcgtgggcccaagctggactctggccactccctggccaggctttggggaggcctggagtcatggccccacagggcttgaagcccggggccgccat

SEQ ID NO: 1041 - DNA, 23 bp, Homo sapiens
  source 1..23: mol_type = unassigned DNA
gtcacctccaatgactagggtgg

SEQ ID NO: 1042 - DNA, 23 bp, Homo sapiens
  source 1..23: mol_type = unassigned DNA
gacatcgatgtcctccccattgg

SEQ ID NO: 1043 - DNA, 23 bp, Homo sapiens
  source 1..23: mol_type = unassigned DNA
gagtccgagcagaagaagaaggg

SEQ ID NO: 1044 - DNA, 23 bp, Homo sapiens
  source 1..23: mol_type = unassigned DNA
gcgccaccggttgatgtgatggg

SEQ ID NO: 1045 - DNA, 23 bp, Homo sapiens
  source 1..23: mol_type = unassigned DNA
ggggcacagatgagaaactcagg

SEQ ID NO: 1046 - DNA, 23 bp, Homo sapiens
  source 1..23: mol_type = unassigned DNA
gtacaaacggcagaagctggagg

SEQ ID NO: 1047 - DNA, 23 bp, Homo sapiens
  source 1..23: mol_type = unassigned DNA
ggcagaagctggaggaggaaggg

SEQ ID NO: 1048 - DNA, 23 bp, Homo sapiens
  source 1..23: mol_type = unassigned DNA
ggagcccttcttcttctgctcgg

SEQ ID NO: 1049 - DNA, 23 bp, Homo sapiens
  source 1..23: mol_type = unassigned DNA
gggcaaccacaaacccacgaggg

SEQ ID NO: 1050 - DNA, 23 bp, Homo sapiens
  source 1..23: mol_type = unassigned DNA
gctcccatcacatcaaccggtgg

SEQ ID NO: 1051 - DNA, 23 bp, Homo sapiens
  source 1..23: mol_type = unassigned DNA
gtggcgcattgccacgaagcagg

SEQ ID NO: 1052 - DNA, 23 bp, Homo sapiens
  source 1..23: mol_type = unassigned DNA
ggcagagtgctgcttgctgctgg

SEQ ID NO: 1053 - DNA, 23 bp, Homo sapiens
  source 1..23: mol_type = unassigned DNA
gcccctgcgtgggcccaagctgg

SEQ ID NO: 1054 - DNA, 23 bp, Homo sapiens
  source 1..23: mol_type = unassigned DNA
gagtggccagagtccagcttggg

SEQ ID NO: 1055 - DNA, 23 bp, Homo sapiens
  source 1..23: mol_type = unassigned DNA
ggcctccccaaagcctggccagg

SEQ ID NO: 1056 - RNA, 20 nt, synthetic construct
  misc_feature 1..20: note = source = /note="Description of Artificial Sequence: Synthetic oligonucleotide"
  source 1..20: mol_type = other RNA
gacatcgatgtcctccccat

SEQ ID NO: 1057 - DNA, 23 bp, synthetic construct
  misc_feature 1..23: note = source = /note="Description of Artificial Sequence: Synthetic oligonucleotide"
  misc_feature 1..23: note = source = /note="Description of Combined DNA/RNA Molecule: Synthetic oligonucleotide"
  source 1..23: mol_type = other DNA
  modified_base 5: mod_base = OTHER; note = uracil
  modified_base 9: mod_base = OTHER; note = uracil
  modified_base 11: mod_base = OTHER; note = uracil
  modified_base 14: mod_base = OTHER; note = uracil
  modified_base 20: mod_base = OTHER; note = uracil
gacatcgatgtcctccccattgg

SEQ ID NO: 1058 - DNA, 23 bp, synthetic construct
  misc_feature 1..23: note = source = /note="Description of Artificial Sequence: Synthetic oligonucleotide"
  misc_feature 1..23: note = source = /note="Description of Combined DNA/RNA Molecule: Synthetic oligonucleotide"
  source 1..23: mol_type = other DNA
  modified_base 5: mod_base = OTHER; note = uracil
  modified_base 9: mod_base = OTHER; note = uracil
  modified_base 14: mod_base = OTHER; note = uracil
gacatcgatagcctccccactgg

SEQ ID NO: 1059 - RNA, 23 nt, synthetic construct
  misc_feature 1..23: note = source = /note="Description of Artificial Sequence: Synthetic oligonucleotide"
  source 1..23: mol_type = other RNA
gacaccgatgtcatctccatcag

SEQ ID NO: 1060 - RNA, 23 nt, synthetic construct
  misc_feature 1..23: note = source = /note="Description of Artificial Sequence: Synthetic oligonucleotide"
  source 1..23: mol_type = other RNA
gacatgaatgacctccccatcag

SEQ ID NO: 1061 - RNA, 23 nt, synthetic construct
  misc_feature 1..23: note = source = /note="Description of Artificial Sequence: Synthetic oligonucleotide"
  source 1..23: mol_type = other RNA
gaaatcaaggtcctccccatagg

SEQ ID NO: 1062 - RNA, 23 nt, synthetic construct
  misc_feature 1..23: note = source = /note="Description of Artificial Sequence: Synthetic oligonucleotide"
  source 1..23: mol_type = other RNA
cacataggtgtcctccccatagg

SEQ ID NO: 1063 - RNA, 20 nt, synthetic construct
  misc_feature 1..20: note = source = /note="Description of Artificial Sequence: Synthetic oligonucleotide"
  source 1..20: mol_type = other RNA
gcgccaccggttgatgtgat

SEQ ID NO: 1064 - DNA, 23 bp, synthetic construct
  misc_feature 1..23: note = source = /note="Description of Artificial Sequence: Synthetic oligonucleotide"
  misc_feature 1..23: note = source = /note="Description of Combined DNA/RNA Molecule: Synthetic oligonucleotide"
  source 1..23: mol_type = other DNA
  modified_base 11..12: mod_base = OTHER; note = uracil
  modified_base 15: mod_base = OTHER; note = uracil
  modified_base 17: mod_base = OTHER; note = uracil
  modified_base 20: mod_base = OTHER; note = uracil
gcgccaccggttgatgtgattgg

SEQ ID NO: 1065 - DNA, 23 bp, synthetic construct
  misc_feature 1..23: note = source = /note="Description of Artificial Sequence: Synthetic oligonucleotide"
  misc_feature 1..23: note = source = /note="Description of Combined DNA/RNA Molecule: Synthetic oligonucleotide"
  source 1..23: mol_type = other DNA
  modified_base 11..12: mod_base = OTHER; note = uracil
  modified_base 15: mod_base = OTHER; note = uracil
  modified_base 17: mod_base = OTHER; note = uracil
gggccatgggttgatgtgacgag

SEQ ID NO: 1066 - DNA, 27 bp, synthetic construct
  misc_feature 1..27: note = source = /note="Description of Artificial Sequence: Synthetic oligonucleotide"
  source 1..27: mol_type = other DNA
gcccgggtggaactggtagccatgaat

SEQ ID NO: 1067 - DNA, 26 bp, synthetic construct
  misc_feature 1..26: note = source = /note="Description of Artificial Sequence: Synthetic oligonucleotide"
  source 1..26: mol_type = other DNA
gttgaagatgaagcccagagcggagt

SEQ ID NO: 1068 - DNA, 27 bp, synthetic construct
  misc_feature 1..27: note = source = /note="Description of Artificial Sequence: Synthetic oligonucleotide"
  source 1..27: mol_type = other DNA
gcttccgacgaggtggccatcaaggat

SEQ ID NO: 1069 - DNA, 27 bp, synthetic construct
  misc_feature 1..27: note = source = /note="Description of Artificial Sequence: Synthetic oligonucleotide"
  source 1..27: mol_type = other DNA
gcaccatctctccgtggtaccccgggt

SEQ ID NO: 1070 - DNA, 26 bp, synthetic construct
  misc_feature 1..26: note = source = /note="Description of Artificial Sequence: Synthetic oligonucleotide"
  source 1..26: mol_type = other DNA
ggtggaactggtagccatgaatgaga

SEQ ID NO: 1071 - DNA, 27 bp, synthetic construct
  misc_feature 1..27: note = source = /note="Description of Artificial Sequence: Synthetic oligonucleotide"
  source 1..27: mol_type = other DNA
gccatgaatgagaccgacccaaagagc

SEQ ID NO: 1072 - DNA, 27 bp, synthetic construct
  misc_feature 1..27: note = source = /note="Description of Artificial Sequence: Synthetic oligonucleotide"
  source 1..27: mol_type = other DNA
gcatcctcgtgggcacttccgacgagg

SEQ ID NO: 1073 - DNA, 27 bp, synthetic construct
  misc_feature 1..27: note = source = /note="Description of Artificial Sequence: Synthetic oligonucleotide"
  source 1..27: mol_type = other DNA
gcagagcggagtgctgttctcccaagt

SEQ ID NO: 1074 - DNA, 26 bp, synthetic construct
  misc_feature 1..26: note = source = /note="Description of Artificial Sequence: Synthetic oligonucleotide"
  source 1..26: mol_type = other DNA
ggtcggtctcattcatggctaccagt

SEQ ID NO: 1075 - DNA, 26 bp, synthetic construct
  misc_feature 1..26: note = source = /note="Description of Artificial Sequence: Synthetic oligonucleotide"
  source 1..26: mol_type = other DNA
gcaataaaaggtgctattgctatagt

SEQ ID NO: 1076 - DNA, 20 bp, Sus scrofa
  source 1..20: mol_type = unassigned DNA
gggagtctttcgctagggtg